European Patent Specification EP 3 787 668 B1, published October 25, 2023. Title: Probiotic bacterial strains producing antimicrobial proteins and compositions comprising these for use in the treatment of diarrhoeal and other microbial diseases. Applicant: Crigasseni AG. The sequence listing filed with the application follows.

SEQUENCE LISTING (163 sequences)

SEQ ID NO: 1 - DNA, 1677 bp, Lactobacillus gasseri CCOS 960
atgcttgctcaagcagcggtcgaatcagcttggggtcaatcaggtttggcacaatcgcctaataataacttattcggtattaagggctcttacaatgggcaatcagtaaatatgaatactggtgagtacggcagcaatggttattacactactaacgctggatttagaaagtatccatcatatactgaatcatttgaagataatggctctttattacgtaaccaaatgggtaactattactctggtacgtgggtagaaaattcaaagaactacgctcaagcaactcaaaatggtttacaaggcaagtatgcaacagcgccaaactatgctcagacacttaatagtgttattgcagctaatggatttgataagtacgatcccgttacccaagttgttaacgaaaatcgtacagtcgcacaaaccacaccaattatgagtgccccagttgatgctagcgttggtactcaagttggtactgcaagaactggtcaaaacgtaaatgttactaagtacatcacttataacaatggtgttaagcgtgcatatattggtactggctggattaacgcacttgcatttagtccaattactactaatacaactactaagcaaaatactgccgctaatactaataatcaagcaagtcaagcagttaagacgccagtcgcacaaactcaacaagttaagagtcaagcacctgcagctccagtaaaagctgcaactgtaaaagtaaagagtgccgctgaagttaaaactccagttcaaactaccactttaaacgttaaaactgaaaataaagcagcacaacctgtaaagcaattagctgtttcattagctgttgcacctaagaaggttgaagttaagaagaacgttgtgaaagctgaaccagctaagacaactccagtaaaaactgaaactactaaaactgaaaacaaagaagttaagactgcaactccagtagttaaaactactgatacagttaaaaaagttgaaactccagcagttaaaccagttgaatctgtaaagaaggaatcaactccagttgttaagactactccagttactgtaactaaagaagctgcaaagaccaccgaagctccagtagttaaacctaagaaggttgaagttaaggaaattaagactactccagtaactactagtgctaaaactgttgtaaagcctgttcaaagttaccaaagtgcagtaactactgctgcaaacaataactatggtactcaatggattagtactaatactgctcctaaggctgcatctactgttttaattaaggttactaagactgttgatgttttatcagcaccagatggtcaaaaattagaccaacaagttgaagctggctcagaatttgttgttgttgcttctaagtactacaatggcaacttatattacgaaattagtaatggtaaatggattatggcaaaatatactactcaagaagcacaaattactgcaaaatctggtgtattaactattaattctaagccagactatggtgtaccagtatggcgtgttccaggtcaagatcaaattgctggtaagttcttgaaagacggctcaagctggagatacttccgtgtagcaaacgttcaaggacaaacttggtatgaccttggcggaaatcaatgggtatctgccaagtctgtactagttcgttaa

SEQ ID NO: 2 - DNA, 627 bp, Lactobacillus gasseri CCOS 960
atgccgcgtagacgccgtcaaaaaaatattcaatatgtaattgcaagagcctttgctatttgctttactttggtagtaattttatcaggctttttgtactggcgtcacgaggtcgcggttaatgaacaattaaggcaagcgcagttagaaaaggaacgcgctcttcaaagtaaagaaaggtttattaaagtagtagctccaattgctcaaagagcagataagccttatggtttatttccaagtgttaccattgcgcaagcatgcttagaaagtaattttggtcaaagtgagctttcaaaaaaatattataatttgttcggtgtcaagggaaccgatcctaatactagccgagagctgacgacttcggaatttgttaatgatcactgggaaactgtaactggtcgttttcaaatttataattcttatgaagaatctattcaggcacatacgcggttatttgtgaatggaactagctggaataaagatcaatatcagcatgttttagctgcaaaagattatgcaagtcaagcgcaagctttagagacggatggttatgcgactgatccaggttatgctaaaaagctaattgatttaattaaagagttcaatttaacgcaatatgattaa

SEQ ID NO: 3 - DNA, 1542 bp, Lactobacillus gasseri CCOS 960
atggttattacactactaacgctggatttagagaagtatccatcatatactgaatcatttgaagataatggctctttattacgtaaccaaatgggtaactattactctggtacgtgggtagaaaattcaaagaactacgctcaagcaactcaaaatggtttacaaggcaagtatgcaacagcgccaaactatgctcagacacttaatagtgttattgcagctaatggatttgataagtacgatcccgttacccaagttgttaacgaaaatcgtacagtcgcacaaaccacaccaattatgagtgccccagttgatgctagcgttggtactcaagttggtactgcaagaactggtcaaaacgtaaatgttactaagtacatcacttataacaatggtgttaagcgtgcatatattggtactggctggattaacgcacttgcatttagtccaattactactaatacaactactaagcaaaatactgccgctaatactaataatcaagcaagtcaagcagttaagacgccagtcgcacaaactcaacaagttaagagtcaagcacctgcagctccagtaaaagctgcaactgtaaaagtaaagagtgccgctgaagttaaaactccagttcaaactaccactttaaacgttaaaactgaaaataaagcagcacaacctgtaaagcaattagctgtttcattagctgttgcacctaagaaggttgaagttaagaagaacgttgtgaaagctgaaccagctaagacaactccagtaaaaactgaaactactaaaactgaaaacaaagaagttaagactgcaactccagtagttaaaactactgatacagttaaaaaagttgaaactccagcagttaaaccagttgaatctgtaaagaaggaatcaactccagttgttaagactactccagttactgtaactaaagaagctgcaaagaccaccgaagctccagtagttaaacctaagaaggttgaagttaaggaaattaagactactccagtaactactagtgctaaaactgttgtaaagcctgttcaaagttaccaaagtgcagtaactactgctgcaaacaataactatggtactcaatggattagtactaatactgctcctaaggctgcatctactgttttaattaaggttactaagactgttgatgttttatcagcaccagatggtcaaaaattagaccaacaagttgaagctggctcagaatttgttgttgttgcttctaagtactacaatggcaacttatattacgaaattagtaatggtaaatggattatggcaaaatatactactcaagaagcacaaattactgcaaaatctggtgtattaactattaattctaagccagactatggtgtaccagtatggcgtgttccaggtcaagatcaaattgctggtaagttcttgaaagacggctcaagctggagatacttccgtgtagcaaacgttcaaggacaaacttggtatgaccttggcggaaatcaatgggtatctgccaagtctgtactagttcgttaa

SEQ ID NO: 4 - DNA, 315 bp, Lactobacillus gasseri CCOS 960
atgaaaaaaagaacattcactggtattgctaccgcggcacttatcacaactgccggtatatcagttaccaacaaccttaaaccagaaaatccattaaaaactggtgaaggtactgttcaagctgcaacatatcaacaagaatttttaaacaaagctattccagctgctacaactgcatcatctaagtatggtacttatacttcagttatgcttgctcaagcagcggtcgaatcagcttgggtcaatcaggtttggcacaatcgcctaataataacttattcggtattaagggctcttacaatgggcaatcagtaa

SEQ ID NO: 5 - DNA, 2319 bp, Lactobacillus plantarum CCOS 893
ttgctaagtaccgctttgctgccgatgttgagtggtaaagctgatacggcaagtacaaatcaaaaaccggcagctgcgactaagggaaacagcgctgcttcagctgcaagccaacaagtgaccttaagtgctggcagtcagacggaaacgacagcggccggtgcgactgaccaatcagttgccagtgacggtgccaagactgacgatcaagctgaatcgaccagcacgacgacggctactaccagtgcgacaagtcgtgtcacagtgcgggcagccagtcaagtcgctaaagctgacagtacagaactgcaaagtcagtcctccgccagtgaagctgccaaggataacgcggctgctagtgctacggcggactccacaactagtgctgttgatcaacttgataaaacggccaaagctagtgcagccacgagccaagccagtcacagtacgactaatgagacggctaaagccagcgcggccgcaagtcaggatagtcatgtcactacggaccaatccagcgtgactgtgacgagtgaagtagccaaatcagccgcatcgtcagccgcacctaagcaagcgactgagcaggcggtagccgcgaaaatctcaccaaagattgagacggctgtggcggctgatgcggtccagtcatcagcgatgatggcacggtccacgcgggcaatgactagtcaggaaatcttcctgagtcagattaaagcgggggcaatctctggttggaacaagtatcaagtcttgccatcagtcacggccgcacaggcaattctggaaagtggttggggacaatcacaacttgcaactcagggaaacaacttattcggtatcaagggaagttatcatgggcaatcaatctacttcccaacccaggaatggaatggctcacaatacattacgattcaagacgcttttcggaagtacccgaattggtcagctagtgttgaagatcatggcgcctttttggttgtcaatccgcgttacagcaatttaattggggttaccgattatcggcgcgttgccagtctcttgcaacaagacggctacgcaaccgcgccaacgtacgcgagttcgctgatcagcatcattgaatataacaagctacacgagtgggatcaagaagcgctcagtggtcaggcaagtggcggaaatgataataaccaagttcagcctgatcaagacgtcaccccaaccagtggtacacataagtttactaagacaacgacaattcacaatgcgccggacgccacgagtgccgtagtgggtacttacaacgctggtgaaacagtcaattacaatggtaagttaacggtcggtaatgcaacttggttacgctatcagtcctattctggcgtatcacggtatgtgatgattagtcaaacaacaactaatgataataataaccaggcgacagttacgccagctagtgggtcgtataagtttaccgcaaagaccaacattcgatcagctgcaagcaaaacggctcaagtggtcggcacttataatgctggtgagacggtttactataatggcaagattaccacgggtgggacaacttggttacggtatttatcctattcaggcgctcagcattacgtggctatgagtggtgatgaggttggttctgtggctaaaccggacgtggttgcaaccagtgggtcgtatcgtttcacgaaaacgacagcaatcaagagttcacctgcaactagtgcgacaacggttgggtcttataatgctggcgatacggtctattacaatggtaaggtgacgacaaatggtcagacttggttacgttacatgtcttactcaggtgcccagcattatgtgcaaattagtggtgagagtacgtcgaccaatgttgataaaccgcaagtaacgcctcaaagtggtagttatcgctttacgcaaacaacggcgattaagaatacaccggccggaaatgccccaagtgtcggtacctatagtgctggtgatacagtctactacaacgctaaggtaacggctaacggccagacttggttacggtatttgtcttattcgggcgcccaacattacgtagcgattagtggtaatgccgctaccggaaatacgacgtctaagccggtaacaaacagtcaaggggcgttccgcttcgtaacgacgactaatattcgtacggcgccaagtacgcgcgcaagcgttgtcggtgaatataacccaggtgaaacggtttattacaatgggacggttcaagctgagggttacacgtggctccgatatctgagtcgctccggtgcaacgcactatgttgctaagcttgaaggctag

SEQ ID NO: 6 - DNA, 639 bp, Lactobacillus plantarum CCOS 893
atggcgggtaagcggcgaaaatcgcgccggaagcaacggacaaagacacaattatttgtgaagaagggccgccttcagtgggtcaatatcttattagtgttggcggcgatggtggggatggtttggtatattcagcataattgggcggttaagtcgcgggttacggcgacagcacctacaacaacgcatgcggcatttattaaaaagctagtaccagctgcgcaacagcttgatcagcaataccacgtgctggctagtatcacgctaagtcaggcgattttggaatcggattggggacaaagtaccaatgcgacagagaataataatttatttggggttaagtccacgtcgggacggctcatgacgacgcaggagtattatgacggggcctatcatacggtcaaacggcgcttcgccgtttatgatagctggcacgcttcgctggtcgatcatgccaagaaattggcgtacggaacgacttgggattctcagcactacgctgcggtgattaaggcaactgattatcagacagctgcgcaagcattgcagacggctggatatgcgactgatccaagttatgcacaaaaattaattaatattattcaaaaatatgacttacaacggtatgatagaaagtaa

SEQ ID NO: 7 - DNA, 1266 bp, Lactobacillus plantarum CCOS 893
atgagcagtgttttaggaattacattagcaaagcctgtacaagggaaagctgatcaaacatcaagtcctagtaccactaaagttaaagccgcaacttcaggtgctacctcagaagtatcatcaattagtacaattacggctaacagtgctactaacgtgtcttcagcaacccatcaattttcaacagcaactactactagccagcaggccagttcagccactagtaatatttccacaactacagcaagcaaacaaatatctaaatccactactggtaagctaaattcaaatgagacagcaactacaagtaatagcgcggctacctccgtagacagtacggcaccatatataccagcaaaatccaatgtcagtttcaccgacaacatcaagtcaactattgcaaatactccgacaacggtagcagcaccagctattcctagtcatagcacgcaatttattgatgattcagcccctatcacatccccgacacccgttacaactaattctatccatgttcgaccatttacagtacatagttcattttcgtttaaaccaggtcaatttttacgcttcacacttcctaatgttgctttacttcgcgatgacgttgaacaaggtgttccaaattacgtaaaaaactttttcattgcaattaaacctggtgcaatgattgggtggtcacaatatcatattctaccatccatttctggagcacaagcattactcgaaagtggttggggaaaatccacattatcagttcaaggtcataatttatttggaatcaaaggctcatatcatggtcattctattgaaatgccaacaacagaatatttaaatggcgaagacgtaacgattgaggctacctttcgaaaatacccagactgggcaactagtattgttgatcatggcgcattccttaatcaaaattctcgttaccgtaatttgcttggagtaaaaaattattcgaccgttgcatgggatttgcaaaacgatggctacgcaacggcacctaactatgccacttcattaattaatgccattcaagattacgatctgcaggaatgggatcaagaagcctttacgggcaatactggttcgacaactacaaccaccggtaaccacaggtccggcacttatacctttattcagaattcgaatatccggacagaaccatccttatctgcacctatcattggtgtttattatcctggggacgtggttaattacacaggtcagattaaagccgaaggatatacttggttataa

SEQ ID NO: 8 - DNA, 777 bp, Lactobacillus plantarum CCOS 893
atggtcgttccagttgatatttggaaccaacgtggcgatgcttctgaccaagttaccttaaaatggccggataatcgtaaacctaaagcggcatttacggttaaccgcaccctggcagctcccggtaacacgatcaagtttacaaatgcctcatccaaaaacgcaaccagctataaatgggaatttgacggtgccacaaagacgaccagcaccgccaaaaaccccacggtcacttaccgtaaggctggcacttataacgtcacattaaccgctaaaaataaggatggccaacggcacgttacaatgaaaaagctcattacgattacaccgaaagctcaaggcgctttaaccttactatccaagaacgccaagaccagtgcctccggatacacgaatagtagtgaagcacctaaaatggcggtggatgggaaactcgatactaaatggtgtgcaaccggtaaggcaccgcataccttgaggctggatttaggccgtcaaacgactgtgagtgcggttaaattagcgcatgccaaagctggtggcgaaggtgctgatatgaacacccgcgcttggaccattcaggtcagcactgatggcaaacgctacacggacgttgcccggacctacaataacacgcaagccactagtctcaatactttcgcggctacttcggcgcgctacgtccggttagtagtcgataaaccaacccaagttgctgacaccgccgttcggatttacgaaatggacgtgctaggattgacgcaaacactcaaataa

SEQ ID NO: 9 - DNA, 285 bp, Lactobacillus plantarum CCOS 893
atgcgtaaggacaccgctagcacaatcaaactctacaccacggacctagacgtcactgccgatacccaggttagtttaaccgctaaggcatctggtaaatctacagctaaactagtggtgaccttaaaggacggccgcactaagaccatcgcgggtgaccggacactcagcaagcactggacgaccgttagctatgacgttagtcagttaacaaaaaaacaatcaaaggccttagcctcaaaatcagtgccgccgagactgatgctagctacagcgttcaattag

SEQ ID NO: 10 - DNA, 1227 bp, Lactobacillus crispatus CCOS 961
atgaagaagagacttttgaccagttttgctgctgccgcaatgcttacttctgtagctgtgccagcagtaaatactacgatgatgaatcaagcctcaagccaacgagtttctgccgctaccgctgatcaaactgcatttttaaacaaggctgccaagcaggcagttaaagcagctaaaaaatatggaactttgccatcagtgatgattgcccaggcaataactgagtcaggctggggaaagtcaggattagccgtgaatgctaataacctttttgggatgaaggctgatgattcttggacaggtgagacttatactgccaagactagagaagaagataaaaacggtaagagctactatattactgctaagtttagaaaatacccatcttttgaacaatcatttgaagataatgggagtaagttgagaaatggtgtttcttgggatccgttgcgttataagggcacttggattgaaaatgcatcaacttatgcagctgcaaccaaggctttgaccggtacgtatgctacagactctaagtatgataaggcattaaatagtcatattactagttctaatttgactaagtatgatccagtaaccgttaatactactagaacttatactgctggcaaggatagttcaacttataattggccaactgctccatctgttgccagtgttattggctctgttaaagctggtgaaaaagtagtagttaccaagactattactttccatgatggttcaagcagaatgtatattgatggtcgcggttgggttaatggctcagttttggacaagagcagttccgcaactaaggaaccagtaactcaggcacctaagaatgtgccagctgtttctaagaacttgatgcataatgcctatgtttatgaccaaaatggtaagaagctaaagggcaagatgtacaagaccagtgatgaaaacggtggtaagtggatcaatacttatggtaccaagaccatcaagggtaagacctactaccgtgtcggtgaaaatgaatacattgcagctggtaatattgatggtagcctcagattcttgaagaagaatgcttatgtttacaatcaatatggcaatcgcgataacaatttgaagcacaagaagaatagccaaattgctacttacggcagtgctataactatcaatggtaagaaatactataaggtaggtattcgtcaatacgttaagaaatcgaacttcatgtaa

SEQ ID NO: 11 - DNA, 648 bp, Lactobacillus crispatus CCOS 961
atggcaagaaaacgtaaatcaagagtaccaaaaagtgtcaaaaccgttgtgcgtgtattcgtaattctatttattctgatggttgcttttgtcggctttagatattataggcgttacgcgattcaatcagagcagattcaacaagcacagctgcaaaaagaacaggaagcagcaaaactattaaaacagaaaaaagactttatcaaaaaaattggtccgattgcgcgcgaagtggacaagtcgtatgacttattgccaagcatcacgattgctcaagcctgcctagaaagtaattatggacaaagtgatttgtcgcaaaaatacaacaatctttttggtgttaaaggatccaacccgaacacttcggcagtgatgacaactaaggaatatgtaaagaataagtgggttaccgtgaaggcgcgtttccaaatatatgactcatatgaggcttctattcgggctcacgctagattattccagaatgggacaacgtggaaccacgatcagtataagcatgttctagcatccaaagattataagacacaagctaaagccttggttaccgacggctatgcgactgatccggactatgccgataagctgattaatttgattgaacagtttgatcttgaaaaatatgataagtaa

SEQ ID NO: 12 - DNA, 315 bp, Lactobacillus gasseri CCOS 960
atgaaaaatgaattaaaacaagtgttgaatgactttatctcacttgctaagactcattatgatagaaaaggcaacgaatacttattagaacaacttgaagttgctttagataagttagaacataatgttcaagatgaagtagatgaagcccgtgcaacttatcaaaatataaatactatttgtcttactaaccatcttcacttggaaacagatgaagaagcattacttgaaaagattaaagaattttcaatgagtaaaggctggcttggtggcttaaacagttggaatacaactaatacttggcctggaagataa

SEQ ID NO: 13 - DNA, 141 bp, Lactobacillus gasseri CCOS 960
gtggggaatgctgtaataggagctgctacgggagctactcgcggagtaagttggtgcagaggattcggaccatggggaatgactgcctgtggcttaggaggtgctgcaattggaggatatctgggatataagagtaattaa

SEQ ID NO: 14 - DNA, 228 bp, Lactobacillus gasseri CCOS 960
atgaaaaattttaatacattatcatttgaaacattggctaacatagttggtgggagaaataattgggctgctaatataggtggagtaggtggagcgacagtcgctggatgggctcttggaaatgcagtttgcggtcctgcttgtggctttgttggagcacactatgttccaatagcatgggctggcgtaacggcagctactggtggattcggaaagataagaaagtag

SEQ ID NO: 15 - DNA, 996 bp, Lactobacillus gasseri CCOS 960
atgattggaaaagaaactcaaatacgtttagtaaataaattagaaaatatacaccacgttgttgttcaagcttcagcactcgatggaagtaatgtatttgtcctacaattacttcatagacagagcgatgttattgtttatcaaactccaaatgatagcgaaactgtgacctttaatgaggatcatccaattttatacttgaaaggacccaattcagctggtacagcgggtggacatactcaaacttgggtacaaagtggagaagacaataaatggttcgttggaactaaacctaaaaagcatggtaatacttattggacaacgcaaattgcgcgagtaacagttcctggctatcaaactcaaatttttaccagtaatacggagttgccaagactttcttatcttaatcgcgcaggttcaggctatggcgatggaagtgtagcttatcctggcaaagatttagttagagtagaagcagctgtttcaccgaataaacaatatttcttaattgcaagtattgacatcaatcacacaggtcattttgctatctataatcttgatgaagttaataaaaaactagatcaagcagaagaaaaagctgaagatgttaatattcagagcttgaattgtttaggtgcatttaatatcccatattttaatgatcaaaagattatttcgattcaaggctatggaattgatgataataaggacatttatatttccagtcagcccagcccgcatacaacgttcttaggatttccaaaacaaggcaaaccacgtgaaattgttaaaattccctggggaatatccgatctaagtaaatggtcagtggtaaatttagacaacagtttaaaattagatgcactaaacttttgcactgaatttgaaggaattcaagtaactggtgattgtctttacttaaccgttgcctatcaccaacgaaacagtgatttgactactttgatgaatcgaatatatcaggttgaaaaattttag

SEQ ID NO: 16 - DNA, 1461 bp, Lactobacillus crispatus CCOS 961
atgataacaggtattaagcggttaagacagacaaaaagatgggctggattagccgcttttttattaggaattttagctgttttatcagttatatattttattgtaattttaattgcagcaatgggagctgctacagatgatgaatgtgatacaggaggagaacaaggaggagtagtagaaggacgaattagtgtcattgaatcacctaagtatggacagaccgctatgatgcatatagcggatgctgtgcatgagaaaactgggattagtgctagattactttttgctcaaatgggacaggaaacaggtaatggtgatagttcagttgctaaacatgatcataactttggtggtatgacttattcagaaggaagcactatcggtaccaaaggtgaaagccgtggtagtgaaggtggtaattacgttcactacaagaacttaagtgattttgcgaccgagtgggctgtgacggttcagaatggttttaaaaaagctggattaggaaaagatgctacagttgctcaatatgctcatgcaatgaaaaaagcaggatactataccgcagctgaaagtgattaccaagcaggtatggaagctcaagctaaaaaatatgatgccttgaaaggcaataaatcactagctaaaggtgatgggtctagtggctcagataattcagctgaggaagattgtaagccaataagcggcaaatgggggtggccattcaagtcaattcctaaaaaaggaccaggtaatacaatctcaggtgagcaattatttggtaagtcatctacaagaacaggtggctttcatgatggtgttgactttggtactgttccatatggtggacaagatattttggcaattcatggtggaaccgttaagaaaattgcatttcaaggacatactcaagatggtctaggaatgtacgtttgggtagaaggctccgacggttggaatgtcatttatcaggaattcggctttgatgaagcagatttgaaatacgtcaaggtagaggtaggcgacaaagtttcagtaggagataaaataggtcacttagcaagtaatgcacatggtattactcacgttcacattggtgcaactgaaaaagattttgctaccgcagagctctctgcgtacaaagatgatggtacttggaaagacccaattaaattaattaaagatggtttgaacaatgatgcagaatctgaagaagatgatggcttatcaaaaactgaatctgaagcacgtgactggattgttcagagagaatctggaggtagatgggacgcagttaacccagctaacccaagtgtttatggacgttatcaattaaagagagaatatcttaatggtgattacagtcataagaatcaaacaagggtagcaaataaatatgtaaaaggcagatatggttcatggcgtaatgcacaaaaattctggatgaaacatacctggtattaa

SEQ ID NO: 17 - DNA, 981 bp, Lactobacillus crispatus CCOS 961
atggttaaaagtattacacctcatttgttttatcgcttgaatgggatgcaccatgttgtagcccaagttggtgtagtaaatggtgatcatgtttttgccttgcaacttcttcacagtgcacatgatgtgttggtttatagaaaacatgaaggtttaactaagaacatcgattatactgatccacacttagtaatgatgggctttggccacacgcaaacctgggtagcagctaatgacaaggatgaatatttcgtaggtgctaaaccaaattcaggcaactggactactcaaattgcacgagtaaagtacccaagacttttaccagaaagatatacttcaaatacacaacttccacgtttgtcacacttgaatcacgtaaccgacgttccttatgatggtcatgatcacttgcacagagtagaagcttcagtttcaccaaatggcaagtacttcatgattgcttcaatttgggatgatggttcaggtcactttggtttgtttgacttaaatgaagtaaaccaaaagttgaatgaaaatggcactaagaacacgccaattactgatttgcattgccttagtgcttttcacattgataactttgatcatccaagcgtggcaccaagtgaagaagctccacaaatgattgattctgttcagggctacgccattgatgatgacaagaatatttatatttctaaccaattgtcacccaagattgatcatgcgaatggtgaagttactacttggtcacgtaagatcgttaagtttccatggggtgaaactaatccagagaactggcaagtagcaatgattgatggtattgatttgcctgatcgctacagtgaagtagaaagtattcatgttcaggcgccagatgacatttatctaactgtggcttaccaccaaaaatatgtcaaagatggcgagtttaagttaagaactttggagaatcaaattttccacattagtgatttaggctaa

SEQ ID NO: 18 - DNA, 936 bp, Lactobacillus crispatus CCOS 961
atgttagatgcaacaaatattagaattttagatagattcgatatgaatacaggttacagagctgtagttcaaaaaggtaatgtaggatcaaagtatgtttatggtttacagttaagaaataaccagacagaaacacatgtattgcgtggcttccgtggcaacgtgacaacccctgtgcttactttagtaggtgcagcagctggacacacccaaacttgggaatattcaggtagatctggtaaatggttcgttggtactaaaaacaagaataaatgggcttctcaaattgctcgagcagatattagatacaaatcatatgcttcatcaaatactgaattcccacgtttagcatacttgaaccgcgcaggtaatcctgaagatcaatgctctggtgatgaaatggaacgcgctgaagtagcagtttcaccagattatagtatgcttttaattgctactattgagaataatggaacaggccacttttcaatttatgacctaaatgtcattaataatgcattagatgaggctggaaataatggtttcgtaaatatgggaaattatcaatgtgaaactagttttacagtatatggtttgtatggatctgttttaaactctgtacaaggttatgatcttgataattctggtaatatttatattactagtcaaaaatcaccaagtttaagtaatggttcatggtcatactatcacaaggaaattgtaaaaattccgttttatgcacgtaatgatcaatctcaatgggaaaatgtaaacttaagtgcatttggtggattagatatttcaggtgaacatagtgaagttgaaagtatccaaattattgatgaaaatcacggttacttaactgttgcataccatgctaatgttaacggtaaaaataaaactgtttcaaataaggtttatgaattagcttgggactaa

SEQ ID NO: 19 - DNA, 252 bp, Lactobacillus crispatus CCOS 961
atgaacaaatttgaaactttaacttatgaagaactgtcagctgttttcggtggtaacggtggtaaagcaagacgccgtagaaaaatcacaaattgtgctaaagctattggaatgggagcgttgaaggatggactaaaatatggcattgcaggcactgcatttggtactccaattggtacagtaggtggagctatatttggtgctaatgtgggtattattagcggatcagtttcttgtgtatcacatttgtaa

SEQ ID NO: 20 - DNA, 198 bp, Lactobacillus crispatus CCOS 961
atgaagaattttaaggtagtaaataatattgagctaaatagagttgttggtggtaaaattattcgattaactccatatatgttgtataatactaagacacataaaactatcccagattacggtgcaatttggggtaaagcgggtcaaaccgtagccaatggatggttacaatatggaccatggggcagtagaggttaa

SEQ ID NO: 21 - DNA, 219 bp, Lactobacillus crispatus CCOS 961
atggtaaagtttcaagaactaaaagaaaatcaattaagtcaagttttaggcggtacacatcacaagcgcggaggcggaaagtaccattactatggtaatggtgtatattgcaaccgatattattgtcatgataatttagcacaaatgtgggatagcgttggtcgtattatgtatactggatggcagaaggatggaccatttgcgcatcctttggtgtaa

SEQ ID NO: 22 - DNA, 675 bp, Lactobacillus crispatus CCOS 961
atgaaaaaaactgaaagtaagtttgcacttttagctgctttaattgctattttagcttttgcctctattcccttatggcaaaacaatctgaatagtttacgaccacaaactcacacggttaagaaaaagaagactgctaaaaagaaaaaagtcgttcatcttacttggggttacccttttaagaagctctatgaaaagaaaatcaaatttaaatctggacaaaagtttggtgaaactgacgtcattcgtcgagtctatcctagcaagagttattttcatgatggctatgacttcggatttagtgaagttggacattcttccgtatatgctgtgcatgcaggaactgtccatcgtgttaaatacgccccaggtttaggactttatatttggattatttccgatgatggctatgttgaagtttaccaggaaggcttcctcagtattactgatatttatgttaaaaaaggtcaaaaagtcaagttgggacaaaaaattggtaaactgaccggctctcacattcatttaggagttactaagacagataaagattacattgataaaaagcatgacaatacgccatgcaaatactattggaaagataatggcacttggttaaatccaatgaaaatcattgaagataatctaagggcagcaggtaaagatccagtccaataa

SEQ ID NO: 23 - DNA, 624 bp, Lactobacillus crispatus CCOS 961
atgaaatttcgtaaattaataatttctttgttaggtactgcattattaacttcaagcgttggtttatcaaccaccactgcttctgctgatacgcttgatgactcacaaaatacaactgaagttcaacccaagaacctcaagtgggcttatccgtttaaagccaacaagaaaaatggtgttcgtccaatgtataatgcacaaacttttggcataactaactatatgcgttctactacaccaccttcctactttcatgatggttgggattttggtttttcagaagttgggcattctaacgtatatgcaattcatcaaggtactgttaaaaaggttgcttatggcaacggccttggctggttcatctgggttattagtcctgataattacgttgaagtttaccaagaagggtttaataagaaaaaagacatttatgttaagactggtcaaaagattaaattagatcaaaagatcggtaagctaactggctcacacttacaccttggcgttactcaaacaaataaagattacataaacaaatatggttttccatgtaagaattggaacgttaacaacggaacttggctcaatccaatcgaggttatcaaaagcaacttaaagaaatag

SEQ ID NO: 24 - DNA, 1293 bp, Bifidobacterium bifidum CCOS 571
atgaggatgcagcagatcaaacacggcggcaggaggccgcgccccagttcagcccccaccatcatcgcggccatgctctgcgtggtggcccttgtggcggcaggcacggcatggtggatgctgcgcccccagcaaaaagacacgctcgaacatctcgcgcagccacagtcctcctcttcgacgctgaaccgcgacaaggcccccacaccgaaaccgcagaaatctcaggagcggcagaaggcagccggtgactcccccgcggccaaggcgagccgcgccatcgccacgatgagtctcgatgaacgggccgggcagctcatcatggcaccgatgttcgcaggcggcaatccggccgatctcagcgccctcatcagcacacgccatgtcggttccgtggtgctcatcggcaactggaacaacggcacagccgcagccaagaccgccgctgacgcgctgcaaagctatgctccgagcggcaaccagctgatcgtctccaccgatcaggaaggcggccaggtgcagcatctcaagggcagtggattcgacacgatgccgtccgcggtggcgcagggccagatgagcgctgacacgctgcgctcctccgcaaagacctggggcggccagctcaagcaagccggcatcaacgtcgacctggccccggtattggggacggtgcaggtcaagcgttcctcgaacgctccgattggcgcgctgaaccgcgatttcggtttggattccaacggaaacgcgcagcacggcatcgcgttcgtcgaaggcatgcgcgacgcgggcgtcggcgcgaccgtcaagcactaccccggtttgggcgcggtgaccggcaataccgatttcacgaccgaaggcatcctcgacaccacgaccacgcttgatggcgaggagataggcgcgttcaacaccacgatcaagcaggcgaagccggctatggtgatgatgtcgctggcgacctaccagcgcatcgactcgtcggcgcccgccgcgttctccagcaagatcatcgacggcacgctgcgcggcagcgtcggctatgacggcgtggtgatctcagactccctttcggccgcggcggtcagcggcatagcgaccaaggacctgggcgtgcgtctggtggacgccggcggcgatttggcgtgcataggcgatacgtcatatgtgacgccgattcttgacggtatcatcgcccgtgcgcagtccgacccggccttcgcgaagaaggtgacggcctccgcaacgcgcgtaatgaccctgaaataccagatgggactggcgaagtga

SEQ ID NO: 25 - DNA, 5808 bp, Bifidobacterium bifidum CCOS 571
atggcagttcgcagacttggtggccgcatcgtggctttcgccgccacagtggccttgtcaataccgttagggttgttaacaaattcagcgtgggcggtcgaggacgccacccgatccgactccaccacgcagatgagctccacgccggaggtggtctactccagcgccgtggattccaagcagaatcgcacctcggatttcgacgccaactggaagttcatgctgtccgattccgtgcaggcgcaggatccggcgttcgacgattcggcctggcagcaggtcgacctgccgcatgactacagcatcacgcagaagtactcgcagagtaatgaggccgaaagcgcataccttcccggcggcaccggctggtaccgcaagtccttcaccatcgaccgggacctcgccggcaagcgcatcgccatcaacttcgacggcgtgtacatgaacgccaccgtctggttcaacggcgtcaagctcggcacccatccgtacggctactcgccgttctccttcgacctgaccggcaacgccaagttcggtggggagaacaccatcgtcgtcaaggtcgagaacaggctgccgtccagccgctggtactccggctccggcatctaccgcgacgtcaccctcaccgtcaccgacggcgtgcacgtcggcaataacggcgtggccatcaagaccccgagcctcgccacccaaaacggcggcaacgtgacgatgaacctcaccaccaaggtcgccaacgacaccaaggccgcggcgaacatcaccctcaagcagaccgtgttccccaagggaggcaagaccgacgccgccatcggcaccgtcaccaccgcatccaagtccatcgcggccggtgccagcgcggacgtgacctccacgatcaccgccgcctcgcccaagctgtggagcatcaagaacccgaacctgtacaccgtgcgcaccgaagtgctcaacggcggcaaggtgctcgacacttacgacaccgaatacggcttccgctggaccggcttcgatgcgaccagcggtttctcgctcaacggcgagaaagtcaagctcaagggcgtctcaatgcatcatgaccagggatcgctcggtgcggtcgccaaccgccgcgccatcgagcgccaggtcgagattctccagaagatgggcgtcaactcgatccgcaccacgcacaaccccgcagccaaggcgctgattgacgtctgcaacgagaagggcgtcctcgtggtcgaagaggtcttcgacatgtggaaccggtcgaagaacggcaacaccgaggattacggcaagtggttcggccaggccatcgccggtgacaacgccgtcctgggtggcgacaaggacgagacctgggccaagttcgacctgaccagcaccatcaaccgtgacaggaacgccccgtccgtcatcatgtggtcgctcggcaacgagatgatggaaggcatcagcggcagcgtctcgggcttcccggctacctccgccaagctggtcgcatggacgaaggccgcggacagcacccgcccgatgacctacggcgacaacaagatcaaggccaactggaacgagtcgaacaccatgggcgacaacctgaccgccaacggcggcgtggtcggcaccaactactccgacggcgcgaactacgacaagatccgcacgacccacccctcatgggccatctacggttccgagacggcgtccgccatcaacagccgaggcatctacaaccgcaccaccggcggcgcccagtcaagcgacaagcagctgaccagctatgacaattccgcagtcggctggggtgccgtcgccagctccgcctggtacgacgtggtccagcgcgatttcgtcgccggcacatacgtgtggaccggcttcgactatctcggcgaacccaccccgtggaacggcaccggctccggcgccgtgggctcctggccgtcgccgaagaactcgtacttcggcatcgtcgacaccgcaggattcccgaaggacacctattacttctatcagagccagtggaacgacgacgtgcacacgctgcacatcctccccgcatggaacgagaacgtcgtcgccaagggctccggcaacaacgtgccggtcgtcgtctacaccgacgcggccaaggtcaagctgtacttcacaccgaagggcagcaccgaaaagcgactgatcggagagaagtccttcaccaagaagaccaccgcggccggatacacctatcaggtctacgagggcgccgacaaggactccaccgcccacaagaacatgtacctgacctggaacgtgccgtgggccgagggcaccatctccgccgaagcatacgacgagaacaacaggctgatccccgaggggtccaccgagggcaacgcgtcggtgaccaccaccggcaaggccgcgaagcttaaagccgatgccgaccgcaagacgatcaccgcggacggcaaggacctgtcgtacatcgaggtcgacgtgaccgacgccaacggccatatcgtccccgatgccgccaaccgcgtcaccttcgacgtcaagggcgccggcaaactggtcggcgtcgacaacggcagctcgccggatcacgactcctatcaggccgacaaccgcaaggcgttcagcggcaaggtgctcgccatcgtccagtccaccaaggaggcgggcgagatcaccgtcaccgccaaggccgacggtctgcaatcatccacagtgaagatcgccaccaccgccgtccccggcaccagcaccgagaagacggtccgcagcttctactactcgcgcaactactacgtcaagaccggcaacaagccgattttgccgagtgatgtcgaggtgcgctactccgacggcacgtcggaccgtcagaacgtcacatgggacgcagtcagcgacgaccagatcgccaaggccggttcgttcagcgtggccggcacggtcgccgggcagaagatctccgtgcgcgtgacgatgatcgacgagatcggtgcgctgctcaactattcggccagcacaccggtcggcacgcccgccgtgctgcctggctcgcgtccggccgtgctgcccgacggcaccgtgaccagcgcgaacttcgccgtcgactggaccaagcccgctgacaccgtgtacaacacggccggcaccgtcaaggtccccggcaccgccaccgtcttcggcaaggagttcaaggtcaccgcgacgatccgcgtgcagcggtcgcaggtcaccatcggcagcagcgtctccggcaatgcgctgcgcctgactcagaacatccccgccgacaagcagtccgacacgctggacgccatcaaggacggctccacgaccgtcgacgccaataccggcggcggcgcgaacccgtcagcatggaccaactgggcgtactcgaaggccggccacaacaccgccgagatcaccttcgagtacgcgaccgagcagcagctcggccagattgtcatgtacttcttccgcgacagcaacgcggtgaggttccccgacgccggcaagacgaagatccagatctccgcggacggcaagaactggacggatctcgctgccacggagaccatcgcggcccaggagtcgtccgaccgagtcaagccgtacacctatgacttcgctccggtgggagccacgttcgtcaaggtcacggtcaccaacgccgacaccacaacccccagcggcgtggtctgcgccggcctgaccgagatcgagctgaagaccgcgaccagcaagttcgtcacgaacacgtccgccgcgctctcgtcgctgacggtgaacggcacgaaggtctccgactccgtgctcgccgccggctcctacaacacgcccgcgatcatcgcggacgtcaaagccgagggcgaaggcaacgccagcgtcaccgtgctgcccgcgcacgacaacgtgatccgcgtgatcaccgagtccgaggaccacgtcacgcgcaagaccttcactatcaacctgggcacggagcaggaattccccgcagactccgatgaacgcgactacccggccgccgacatgacggtcaccgcgggtagcgaacagacgtccggcaccgcgaccgaaggcccgaagaaattcgcggtcgacggcaacaccagcacgtactggcattccaactggacgcccaccaccgtgaacgacctgtggatcgccttcgagctccagaaacccaccaagctcgacgcgctgcgctacctgccgcgccccgcgggcagcaagaacggctccgtcaccgaatacaaggttcaggtcagcgatgacggcaccaactggaccgacgcgggctccggcacatggaccaccgattacggctggaagctcgccgagttcaatcagccggtgaccaccaagcacgtgcggctcaaggccgtccacacctatgcggattccggcaacgacaagttcatgtccgcctccgaaatccgcctgcgcaaggccgtcgacaccaccgacatcagcggcgcgaccgtgaccgtgcccgccaagctgaccgtcgaccgggtggacgccgaccatcccgccaccttcgccacgaaggacgtgacggtgacgttgggcgacgccacgctgcgctacggcgtggactacctgctcgactacgcgggcaacaccgccgtcggcaaggccacggtgaccgtgcgcggcatcgacaagtactccggcaccgtcgccaagacgttcaccatcgaactgaagaacgccccggcgccggaaccgacgctgacctcggtgagcgtcaagaccaagccttccaagctgacctacgtggtcggcgacgcgttcgacccggcaggactggtgctgcagctcaactatgacgacgacagcaccggcaccgtgacctggaacacgcagacggccggcgacttcacgttcaagcctgcgctcgacgcgaagctcaaggtcaccgacaagaccgtcaccgtcacctaccagggcaagtccgcggtcatcgacatcaccgtctcgcagcccgccccgaccgtcagcaagacggatctggacaaggccatcaaggcgatcgaggccaagaacccggattcatccaagtacacggccgactcgtggaagaccttcgcggacgccatggcgcatgccaaggccgtcatcgcggatgattccgccacccagcaggacatcgataacgcgctcaaggcgctgaccgacgcctacgccgggctgaccgagaagacgcccgaacccgcccccgtcagcaagtccgagctggacaagaagatcaaggcgatcgaggccgagaagctggacgggtcgaagtacacggccgagtcgtggaaggcgttcgagaccgccctggcgcatgccaaggccgtcatcgccagcgattccgccacccagcaggatgtggacgcggcccttggcgccctgacctccgctcgtgacggactgaccgagaagggcgaggtcaagcccgacccgaagcctgaaccgggcaccgtcgacaaggcggcgctggataaggcggtcaagaaggtcgaggccgagaagctggacgggtcgaagtacacggccgactcgtggaaggcgttcgagaccgccctggcgcatgccaaggccgtcatcggcaacgccaactccacgcagttcgacatcgacaacgcgctgtcgatgctcaacgacgcccgcgccgcgctcaaggagaagcccggccgcatcatcgccatcatcgatggcagcgcactgagcaagaccggcgcatccgtcgccgtcatcgcctccgtcgcggccgcgatgctggcggtcggtgccggcgtcatggcgttgcgccgcaagcgctcctga

SEQ ID NO: 26 - DNA, 465 bp, Bifidobacterium bifidum CCOS 571
atgcattcgcgaccgatgttcccgattccggagacgcaggtcggcgacggctgggtcggcgacgtcgactacacgaagcaggccacgaagcaggacagcaatttcctcgtcgactgggtgcgcgtgtaccaatccgaggggcagccggtgacgcgtttcgacgacctggacggcgccgagagcggcgcgtaccggagcgcccccgcctcacggaccgaggggctgaccgcagtgagcaacggcgacgccgcctggcggaacaagaacaacttctactacggcggacagccgcggtatgagaccagccgttcccatgccgtgcccctgatgcagggccgattcgccctgcgcttgcggggcccacaaacactctgccgaatccggacgaatgcttttacccgcagcgagcgacccgttgcaggcaaggttgtgccgccgaatcggcgaaatcgcgcggcgccgtga

SEQ ID NO: 27 - DNA, 558 bp, Bifidobacterium bifidum CCOS 571
atgatttcggcgagccgagagatacactccatcaacctgtaccgcaatgggtatgagaacgcgctgaacacgttcaagcgcatcaaggtcgaagtgtcctccaacgaggacttctccgacgcgaacgtgctgttcggcaccgccgacgtcgaggaaaccgccgcgaccaagctcgccgcgcagaccatcaacctgaccacgcccgtcaccgcgcggtacgtgcgcatctggcagaagggccattgcatccagaacacgaactcctcatggaagggatacggcaacggcgtgggcttgcgcgaaatcgaggtcatcgccaagctcaaggacggcgagaccctgccggacgcgcaggagacgcgcaacatcgcgctcggcaagttgccgtatgtgtacggcctcgacccgaccaacatcgcggcgatcagcgacggcaagcaggacgacaactacgccgtgcacaacagcaccggcgagcggtggctgcagttcgaatacaagaaccgctaccgtatccacgagggctcaagccgggcacctatccgctggtccgcatag

SEQ ID NO: 28 - DNA, 327 bp, Bifidobacterium bifidum CCOS 571
atgagacaattattccgccgtatcacgaccatatccgccacatgcgcgttggccgtttcggttgcagccgcagtcgcggtggccgccgaacccaccacaggcaacatacttaccggcaaactgcccacgaccaacagcacgcatctgatcggcgacggcgacaccggattcggcccgaccgacagcaacatcaccaaaatcatcgccggagaagagaacggcagcgcggaaaacaacggatacgccagctgggacgacgtatacctgcaatatgatttcggcgagccgagagatacactccatcaacctgtaccgcaatgggtatga

SEQ ID NO: 29 - DNA, 5796 bp, Bifidobacterium bifidum CCOS 571
atgagaaaacgagtggtttcagtggcccttgcggttgcgctcgctgtcgccccactgggggtggtcagcacagcgtccgccgcgccgctttctgcaagtgatttgcaaactctcgcgctccgttcagcggctagctccaatgacgcgaacgccaacgatgtcgccaccgtcgcggacgatgctgccgtgaacggctggacgattgaccgcaacaccgccaaaggcggcgaaattcttgcagccggcactggcgattatgcgggatggactcatttcaagtccacctccgccaacggcaatgccaccagcagcagtggctatccggctgtcgccattagcggcaagacgattgacctgactcgggctggagagttctccatcaaggtcaagtccccgcaggctggttccgcgaaccgtttcggcttctacctcggctacaaggatccgggcaacgccctgttcctgggctatgacaaggggggctggttctggcagaagtatgtcggaggcaatggcgattggtacaacggcacacgtgtcgctgcccctgccgcgaacgctgaaatcaccgtcaacgtctcctggactgccgccaaggttgccacgctgactattgacggacagaaggcgttcgatgtggattactcctcgatgaccgcgctgaccgacaagctcgccatgaaggccggctcttactccggcaccagcgaagtcactgatgtctacttcaaaaacttcaccgtgggtgaagtcgccaagcacaacgtgaccggcaaggtcgtcgacgccagcggcgccgccatcgccggcgccgaagtcgtcaccggcaagaactccgccaccaccgcggcggacggcaccttcaccctcaccggcctcgccgccggcgactacacgctgaccgtgtccgccgaaggctacgatgacgccaccaagaccgtcaccgtcgccgatggcaatgcctcagtcggcaacatcacgctgaacaagtcggccgaagtcgctactgagacgctctccaccgccgccatggacgtgcgcgtgaagaagaacttcccgtccgtgtacgactacacgatgaagaagctcgacggcaagatcatgtacggccagccgaaggacgtgcgcgtcatcaccattaacggcaccgacgtgacgctgaaggactccgacgtgaccttcaagaaggtcagcgcgaccgaggcccagtacacgctgaacgtcaagagcggcgacaagatcaacgcggtcgtcaccgtgcagatcaaggtcgtcgacaatacgctcaagctcaacgtcaccaagatcgtgaacaaggcggatgacgccaagaccgaggccgaggagaacccggtccagacgattgcgttcccgaaccagagcctcatctccgtgcgctccggtcaggacggcgcccagttcaccggcgcccgcatgtcgtccgacactgccaggcccggtgacaccaacttcgacatcaccgccgacaccacggtcagcaatgcgaacgactacacctacggcttcgtctcgggcaatggcctgagcgccggcctgtggtccaactccgagcacgacggcaccaccgtcggcaacaccgtcgccggcggtgcgaggaacacccgcgtgctcacctccacccagaaggtcggcaaggccacctccttcggtctgggcactgcaccgtggtactaccaccgcgtcgtgaccgacacgaagaagaacacctacaccgtcgaagagaccgacatgccgaagatggccgtcgccatcgccggcgacgagaacgaggacggcacggtcaactgggaagatggcgcgatcgcataccgcgacatcatgaacaacccatacaagtccgaggaagtgcccgagctggtcgcatggcgcatcgccatgaacttcggctcccaggcgcagaacccgttcctgaccacgcttgacaacgtcaagaaggtcgccctcaacaccgacggcctcggccagtccgtgctgctcaagggctacggcaacgaaggccacgactccggccatccggactacggcgacatcaacacccgcgccggcggcgccgcggacatgaacaccctgatggagaagggcaccaagtacggcgcccgcttcggcgtgcacgtcaacgcgtccgaaatgtacccggaagccaaggccttcagcgaggacatggtgcgtcgcaactccagtggcggcctgagctacggctggaactggctggatcagggcatcggcatcgacggcatctacgatctcgcctccggcatgcgcaagtcccgcttcgctgacctcaagagcaaggtcggcgacaacatggacttcatctacctcgacgtgtggggcaacaacacctccggcgccgaggactcgtgggaaacccgcaagatgagccaaatgatcaaccagaacggctggcgtatgaccaccgaatggggcgccggcaacgagtatgacgcaaccttccagcactgggccgccgaccttacctacggtggttccgccatgaagggcgagaattctcaggtcatgcgcttcctgcgcaaccaccagaaggacagctgggtcggcgactacccgtcgtacggccaggccgcgaacgccccgctgctcggcggctacagcatgaaggacttcgaaggctggcagggacgcaacgactacgccgcgtacatcaggaacctgtacacgcacgacgtgtccaccaagttcatccagcacttcaaggtcgtccgctgggtcaacagcccgctcgacgccacctccgtgaaggatgcctccgtcaacaacggcaacgagcagatcacgctgaaggacgaccacggcaacgtcgtcgtcctgtcccgtggctccaacgacaccaacaacaccgcgtaccgcaaccgcaccatcacgctcaacggcatcaccgtggcgtccggcgcggtctccccgggcaacagcaacaccgtcaagggcactgagtcctacctgctgccgtggctgtgggacgtgaacaccggcaagctcgtcaagtcctccgatgagaagctgtaccactggaatacccagggcggcaccaccgagtggaccctgccgaaggattggcagaacctcgcctccgtcaaggtgtaccagctcaccgaccagggcaagaccaacgagaagaccgtcgccgtctccggcggcaagatctcgctgaccgccgaggccgagaccccgtacgtcgtgaccaagggctccgagaagcagatctccgtcaagtggagcgaaggcatgcacgtcgtggacgccggcttcaacggcggccagaacaccctcaaggacaactgggccgtctccggcaccggcaaggccgaggtcgaaggcaccaacaacgccatgctgcgcctgaccggtgacgtgaaggtctcccagaagctcaccgacctgaccgcgggcaagcgttacgcgatctacgtgggcgtggacaaccgcaccaactccccggccaagatcaccgtgaccaacggcaccaaggtcctcgccaccaacgagaccggcaagtcgatcgccaagaactacatcaaggcgtacggccacaacacgtactcgaacactgaaggcggcagcagctacttccagaacatgtacgtgtggttcgtggctccggaaagcggcgacgtcaaggtgacgctctcgcactccggcgcatgcgacaacaccgaccatgtgtacttcgatgacgtgcgcgtgcttgagaacggttacaagggcctgacgctcaacgctgacggcaccctgaagacgctcaccaacgacttcgaggacaatgcccagggcatctggccgttcgtggtctccggctccgaaggcgtcgaggacaaccgtatccacctgtccgagctgcatgacccgttcacgcaggccggctgggatgtcaagaagatggacgacgtgctcgacggcaagtggtccgtcaaggccaacggcctgatccagaagggcacgctgatctaccagacgatcccgcagaacgtcaagctggaaccgggcgagacctacaaggtgtcgttcaagtaccagtccggctccgacgacatctacgccatcgccaccggtgacggcgagtacaacgccagcaccgtcaagctcaccaacctgaagaaggccctgggcgaggacggcacggccgagttcgagatcaccggttccatcaccggcgacagctggttcggcatctactcgacctccaccgctcccgacctgcagaacacgtccgattccgccgccaacttcggtggctacaaggacttcgtcctcgatgacctgaaggtcgagcacgtggcatccgccgagcacaccaaggccgacgccgaggcgaagctcaaggaagtcaaggacacctacgacggcaagagcggcgactactccgccgaagtctggaccacgtacgtgaacacggtggccgagatcgaggcgctcatcgccaaggataagcccgactacaccaccgcctacaacaaggctgtggcgctggccgagtacatgaagaacgcaccgggcgacgactcgaacgatgcgtacgacgtggcgaccgacgcctacaccgtcgaggcgggcagccagcaggcactgtcgggcggcaatgagggcccggcaagcctcgcccaggacggcaatgccggcactcactggcacacctcctggagcgccaacgcagtgtccgccggtaccgcctggtatcagttcaacctgaacgagccgacgaccatcgacggtctgcgttacatggcccgcagtggcggcgcgaacgcgaacggcaagatcaagaagtacaagattacgctgacgctgtccgacggcaccaccaaggacgtcgtcaccaatggcacgttcaccacgaccagcggtgtctggcagaaggtcaagttcgacgcggtcaagaacgtcaccaaggtgcgcatcaccgctctcgaaaccgcgggacagtccgcgggcgaggtgaacacgtacgcctccgctgccgagctgcgtgtcaccacggttcgcgacgtgccgagcaccgaggtcaaggtcaacaagtgcgatctgcagaacctgtacgatgacgcttccgccctgaccgaggccacctacaccgccgacacctggaaggtgctcgtcgccaagcgcgacgccgccaagaaggtgctggacgacgagaacgccaccgcgcacgacgtggctctcgcctaccagaacctgaaggatgccatcgccgccctggaagagcgcgtggacacctccaagctcgccggcctggtcgccgatgccgagaagctcaaggaatccgcgtacaccaaggattcgtgggccgcgttcaagaaggctctggatgccgccaaggccgtcctgaacaatgcgaacgccaccaaggctgacgtcgatgccgcgtacaacgcgctgaacgccgcgatgaaggccctgaagcccgcctcctccaagccgactccgaacccggagacgaccgacaagagcaagttgcaggccaccatcgatcaggccaaggccctggatctgagcggttacacgaagaagtccgcccaggccgtgcgtgacgccctcgccaaggcccagagcgtcctcgccgatgacaacgccacccaggctgacatcgacgccgcgcagaaggccctcgctgacgcgatcgccgcactggagaaggccgatgccaacggcaacgccatctccaagacgggtgcgaacgtcgccgtcatcggcatggccggcatgatgctggtcgccgccgctggcgcggtgttcatcgcccgcaagcgcgccgagtga

SEQ ID NO: 30 - DNA, 2604 bp, Bifidobacterium bifidum CCOS 571
atggtttcgccacatcatcttttgaagattgcgactgcgctgtctgcggttgcgttgacggcttccgttgcggttacgccggcttacgcattgcaggatattgcgattgaggatgctgttgcacagagcggtcccgttactgcagataatggcgttgttgtgcagtctgacgatcagtctgacgatcagacgggcgaccagcagtcgcaagacggcatgcctgacaatccgaatgcgaaacttccggataccgtcagtgacgagatttccgacgatgccaccgtggtttcggaagacctggccgttacccccgaaggtgaggtcaagaatattgaaaccggcgaaaccgtgaccgatgcgacactggtcggtacgcaggatcagcagccggatccgctcgccaaaaccaacggcgaatccttcattccggtaagtgcggaagatgtcaaaaatgctgtagccgacgcgaacgtacagctctccaaattcgaaggcaatgaatacggcgcgcactggggcacttacaacaatacgaaagccttcttcgactaccagaacaacctgttcgtgcagcaagccaaaggcgtgatcgacgtttccgaatggcaaggcgacatcgactgggccaaagcgaaagccgacggcgtggaaggcgtgatcatccgcctcggctacggttggggcaacaatgctgacaggaaagcacaacgtaacatttccgaatgcaagcgacttggtatcccgttcggcatctactggtattcctacgcggacactccgtcgattgccaaagaagaaggtgccggcgtggtcgccaaactcaagcgattcggtgtgcgcgcgagcgacttggcgtaccccgtgtactacgacctggaaaagtggacgtggaaggggcatcagccgcccaccgatccgaacgtgtacagcgatatcgtcaacaattggtacggcgcgctgcagtccgccggatacaagaacctgggcgtctactcgtacaccagctacctgcaaggcccgctgaaacatgccgacatttacgccaaaaccacgtgggtggcgcagtacggcgctcgcatgggattcgactcgttcccgaccaacagtcgcggatggcaatacaccagctccggcaaagtgggcggcatcaggggcaatgtggatatgaatgcgtttgggaataaggagtatgtgaatggcgggagtagtaatgatttacaagcggccattgatgtacgcaaaatgactgcagttaccattccgaatggcaattattacatcaatgttcgttccaaagtcgcgtccagtgttgatgttcctggtggaagtgctgcggattccaccgccattcagttgtattccggcaacagttccaaggctcagcagttcacttttactaggcagtctgatgggagctacgagatcgtcaatgtgaattccggcaaggctttggacgtgcgtaatggtgttgctgagaataacgctgtagtgcaacagtattctcgaaataattcccaggctcagcgatggtttattcgtgattccggagcgggatcttatttgcagtccgctctcggtaattgggttctggatttgagtggcggaaatactgcgaatggtgctgcgattcggctgtatgcgccaaatggcactgcttcacagctgtttgttgtttcgtcaagcgatgccagtatagctactggagtgtcgatgattatcacttcggttgcgaataaaaaacttgtcacggatgtgacgggtgcgtcaacggcgaacggggcgcgagtccagcttgattcaagtaataatacgaacgcccagaaatatcgatttgaatcaatcggcaacggaacttacaagattatcaatgctaattcaggcaaggtgctggatgtggctggcggatccactgctgatggagcggcattgcagcaatatacgagtaacaatactgttgctcagcagtggacagtgcggaattacggcagcggcaggattgcgctggtgtcggtgaacgccaacaaagctgtcgatattccaggtggcaatgccgtgcagcaggctcagctgcagctttattcgccgaatggcactgttgctcagcagtggttggtcgcaaaggcgccgttgacgttgcgcgaacgtttgaacgaaaccgcagccaagcataggcaggatctgccggatggcacctacacgttcggatcgaagcttaatacgtccatgaagatggatgtaagcggcgcttcccgttcaaattatggaaacgtgcagatctgggcgggtaatggaaccaatgctcagaagtggaaagtgacgcatgattccaacggatacgtgaccttgaccagtgtgaactccggcaaagtgttggatgtgaatggcggcgtatctgccaacggaaccaacgtgcaacagtacgattccaatggaacatacgctcagaagtggatagcagtcaaaaactccgatggctcatacacgttccagtcggcgctcgcggaaaacaaagttcttgatgtttcgggtgcttctacctcgaatggtgccaatgtgcaactgtataccgcaaatggcacgaatgctcaaaagtgggtgaaatag

SEQ ID NO: 31 - DNA, 2337 bp, Bifidobacterium bifidum CCOS 571
atgtcattcgatctcattccggaaccgcaatccgtgacattgaaaggggatgccgccgattcggatgatgccggagctccggtacccgtcgcgttgccgctcgtaggccgcatctcggaagatcgcgacatcgatgacatcgccggcgttttcccgacccagcttgccgatgatatcgaagcggcgacgggcctgcgctgggacatcgccagcgatgtcatggtggccggactgcccgcgccaaatgccgcgattgcgcacccggttccgccacacgcttcatgctggaagtcgttcatcacactgagactcgaccccccatccctggagccgcaggaataccgcctgaccatcgcacgctccggcatagacgtcgtcggcggcgatacggaaggcgtgcgcaacggcgtgcagacccttcgccagatcatccgtcagtgcgcgccggcgctgcctcgactcgtcatcgcggacaaaccggcgtacaaggtccgcggctactatctcgacgccacgcgcggccgcgtccccacgctcgactggctgaaaacatgggccgaccggctgtgcctgtacaagtacaaccagcttcagctatacatcgagcacacgttcatgttcgacgatctgagcgagacttggcgcggcaccagcccgctcaagcccgccgacatcatcgcgttcgacgaatactgcgcgcggctcggcatcgagctggtgccgtcggtctcgactttcggacaccagtacatggcgatgcgcacgcgcgagctgcgccatctcggcgagtttcccgaggacgccgaccgtcggtacggtttcgtggagcggcagcgtcaccacacgctcaacatcaccgaaccggagtccctcgcgttctcgttcaagctgatcgatgcttacatgcagctgttccgcacacgcaagttcaacatctgcggcgatgagacgttcgacttgggtcgcggccgttccaagcccgaagccgaacgccgcggcgtggccgcgatgtacgccgacttcgtatcgcagctgtgccgtcacttgtctgagcgcggccgcgatccgatgttctggggcgacatcgctgtggagatgccgcagatcctcggcctgttgccggataacgtcacgctgctcaactggctgtacgcgccgggcatcggcgaagacaaggtacgcctcgtcgcgcaggccggggccccgcagtacgtgtgctcggcggtgtggtgctggaatgcgctgctgccgcgcctcgacgactcgtggaacaacatctcccgactcgcgcgctacggcgtgaagtacggtgcggtcgggtacctggtgaccgactggggtgattacgggcatgtcaacgacccgcgcatggcggtttccggcatgatattcggcgcgcagtgcgcgtggaatccgatggctcatatccagggtgaggccgggtgcggcgacggcgaagaaggctctgctgccggttatgccgatgccgccgccgatgtcgtccgcgagaacaaggccgccgcggacggggattccccggcgccgctcccgtcgagctcggaaagcgacgattacaccggtggcgcggccgacgcgattgcgggcgcgccggccggcggcgatgggtcgtgtgccgagatgtgccgtcgcgtggccgaggtcgaatacggcgaccgttcgggcggcatagtcgaggcactgcgagatgccgcctgtcgtgtggcgttcggctgggatgacatggtctggtactgcgagctggatgaaggcgacggacggatgaatcgcgatgccgcatcggcgatgcatctcggcgtgcatgggttcagcggggaatacgggcgggagtgggaggcccgactgctgggcagtgccgatcttgatgaggctcggcgcacgatgctgcaagggctgtcgccgcatatcgtccgcgcggccgaggcgaacgaggcgctgctgtgcgacgccatgcgactcggcgccgccgccggtcgcgcatcgcgtttgggtgcggctcggcgtgatgtgccggcgatgctggccgccatcgaggggcagcgctggttcaacttggtcggcttgtgccttgcgcggcggcatgacgtcatcacggtcgatgccggcgatatcgcccgcgcgtcggccggattgatcgaaccggacgcaggctcttccgcagggccggaagccgtgcaggatgtctcgattcgagtggcacgtggtctggagcgctggttcgagacctactgcgacttgtggcgttctgtcagcgcggaatcggaattggcccgcatcgcctccatcgtgtggcgctgtgccgacgccctgcgttcataa

SEQ ID NO: 32 - DNA, 915 bp, Bifidobacterium bifidum CCOS 571
atggctgatagattcggagcttttctgcctcacgacacctcgggcgacgttgcccagctgcacggcatcggtctgcaaaaattcggcgacacctggtatgcatatggcgagaacaaggtaaacggcaatttgttccagggcgtgtgctgttatacaaccaccgatttcatcgcatggcgcagccacggcatcgtacttgatgtgcaagaagacggctccgccctcgccgctgaccgtatcggcgagcggccgaaggtgctgcattgccccgccaccggcaaatatgtcatgtatattcatgccgaaacgcccgactacggatacgcgcacatcggcgtcgccgtggccgacgccccaaccggcccgttcgcattccagaccaccatcacgtggcgtggctacctgagccgtgacatcggcgtcttccaggacgaggacggcagcggctacatcatgagcgaggaccgcgaccatggcacgcacatttaccgtctcgccgacgactacctcaccatcgtcgaggacgtcgcctgtgagcgtgccaccgactacccatacggcctggaatcgccgaccatcatcaagaaggacggcctgtactactggttcggctcgcaactgaccagctgggacaccaacgacaacaagtactccaccgccaccgacctgcacggcccgtggagcgagtggaagctgttcgcgccggagggtgcgaagacctacgattcgcaggtcgatatcgtggtgccgctggacgacgacccgtacaacagcgagcacttcctgttcatcggcgaccgctggcaggagcatgacctcggcaactcgccgatcgtacagatgccgatttccatcgccgacggcgtggcgtcgctgacgtggagcgacacctacgagggcaccacccaccgctga

SEQ ID NO: 33 - DNA, 1905 bp, Bifidobacterium bifidum CCOS 571
atgatgcaattcaccatgtccggaaccatgctgcgcttcgatgagacgacgctgcggttctcattcagccgcgacggtgcgacctggagcggctgcgacggcatagagccgcagctgacgcgcgaggatcgttcattctcgttcgccggcgccgctaccgtcacgcatgagcggatcgagaccggcaccggagtcggcgtgcgcagcgtgttcgccgggttcgcgggtgcggattacgcttttgagacgtatatctggatcgagcggtcgagcggcgacgtgctatgcgaatgggtgccactgcgcgagtgtggggccgagccgcgcatcgacagggtgctttggcctgcgccgctgtccttcgaccatgcggacgcgcatgacgtgacgctcatcacccacgagcagggcgtgatgataccgaataactggcctaccgaggtcggcactgatgcggtctccttcggcgggcggttcgagactgcgggcgggtacatgccctggttcgcgcagttgcgcagcgacgggcatgcgtacatcgccatctgcgagacgccatggaacgcaggatatgacatcgaccatccggccggcggaccgtacacgcacgtcggaatgtggttcgagccaagtctcggccgcatggattaccgtcgtgtcgtgcgatatcgtctcctcgaccacgccgaccataccgccgtctgcaagacgtaccgcgcttacgtcaacgaacgcggccggctgcgcacgctggcggagaaggcggcgcgcaacccgtcggtgcgtgacctgctcggccgttcatgggtgcatgtcggcatcaagacgaaggttcagccggactcgtcgttctatgatcccgcgcagcccggcaagaatgattcgctcgtcacgttcgcgcagcgcgaacggcagatgcgcacgctgcacgaaatgggtgccgggcggctgtacctgcatctggacggctgggcgcagcccggctacgacaacggccatcccgactatctgcccgcatgccgcgaggccggcggctggaagggcatgaaatcgctggtcgacgcctgtcatgagcagggagacctgttcggcacgcatgaccaataccgcgactattacttcgccgcgcgcacgttcgacccgcgcaatgcgatccgactggcggacggcacgatgcccgagcacgcgatgtgggccggcgggcgccaaacgtacctgtgcgccgagcttgcgccggattacgtgcgccgcaacttcagtgagatcgccacgcacggcatcgcgctggactgcgcgtatctggacgtgttcacctgcaatgaaggcgacgaatgctcgcatcccgagcaccgcatgacccgccgcggatgctacgagcgccgcgccgaatgcttcgaatacctgctggcgcacggcattctcacctcgtccgaggaggtgtccgactgggcggtgccgagcctggtgttctgccattacgcgccgtacgacttccagatgcgctcccccgacgcgcctcggcacggcatcccggtgccgttgtacaacctcgtctaccatgactgcgtgatccagccgtggatgatggatcgggtggccggtggcgacgactacatgctgtacgcgctgctcaacggcggtgcgccgtacctgatccgtgacgccgcatatgccggcatggacggtgatatgaatgccgcactgcgcgcccgtaccgagaatgacatcgagcggtgtgcggtcgtggccgggctgcaccggcgcgtcggcatgcaggagctcgtgcggcatgaccttgtcggcggcgacccgctggtgcagcgctcggtcttcgccgacggcaccgccgtgacgtgtgatttccacgcgcagacgtatgaggtagcagcgaacggttctcattaa

SEQ ID NO: 34 - DNA, 3417 bp, Bifidobacterium bifidum CCOS 571
atgcgagcgaatggtaattccacgcatgagattctaggcaaaatcgtgacggccatcgcgtcgatcgccatgaccgcggcgttcgcggttccggccatggcggccagcgacagcgacacggcggccgactccggcacgacccaacagtcgggccagtacaagatctacccccagccgcagaacaccgagtatggcgacggcagtctgattctgcgcgacaaggcgaacaccgtcgtggaaccgggaatcgattccgccaccaaggcccgtctgaacgaggccctgaagctcaagggcatcgagaccaccgcggccgacgccgtgcccgaaaccgcgtaccagctcaacgtgctggtcggcatcaacggatccaacggcgtggtcgacaagtacgccaagcagctgatcgccgacggcaccctgaaggtggacgacagcacgttctccaagaacgactcctatgtgcttgccgtccgtcagggcaacgcgaagacgcccgacacgatcctcgtgctcggccgcgacaccgattccgcgttctacggcctgactaccctgtaccagatcttccagcagctgccgggccgcgccgtcagcaacctgaccttcagcgactgggccgacgtcaagtcccgcggcttcatcgagggctattacggcagcccgtggagcaccaaggaccgcgtgaacctgatgacctggggcggctactacaagatgaacacctacgtgtacgcccccaaggacgatccgctgcaccgcaacaactggcgcggcctgtacaccgaagaccagatcgagaacgagatcaagccgcaggccgaggccggcaacaagtcgaaggtgcgtttcgtttacgcgctcgcgccgttccataacgacggcgaggctaggggcaagcacttccgcttcgacaccgaggagcactaccagaaggacctcaaggaactcaaggccaagtacatgcagaccattgacgccggcgtacgccagatcgcactgctcgccgacgactccaccgactggggtgcgcagtacggcaacgacaacacctacgtgcgcgtgctgaaggacctgaccgactggatccacgagctgcagcaggagaagaacgacgacggcaccgcgaagtacgagggcctcaaggacacgatcctctactgcccggccctgtacagctacaccggagccggtgacgcctggtacaaggacatcccatccaacgtgcagatcgtcatgaccggcggccgcaccttcggcgtggccagcaaggacttcgccgacacgttcaccaagaacaccggtcgcgccccgttcatgtggatcaactggccgtgctccgacatgaaccgcaacaccgcctaccagtacctggtcatgggaggccagaacaacttcctcaagcccggcgccacatacggcacctacgacggcatcatgctcaacccgatgcagcagtccgagccgagcaagcagggcatcttcatggccgccgactacagctggaacctgtggcagagcgaaaaggacggacaacagtcctgggaggactccttcagctacatcgaccacaactcgccgatcgcgtccaagggctcccgtggcctgcgtgacctcgccatgaacatgcgcatcctcaacgacggcggcatcgacggcgctcacaaggatgccgagtatgacgccgtcaacaagtggtggatcaacaatgagtccgtcgactacaccggcaagctcgacgtcaagggcgtcctgaccgaactcaagggcaagctggacggcggcaccgccaccgcggccgacttcagccaggcgctcaccgtctacaccacgctgcagcgcgccgcgaagaactaccgcgcgaaccccggcgacaagaacatgtttgaccagatcgaaccgtggatcagctactgggacgacctgaccgcctccgccatcgactacatcaccgccgccaagcaggcgctcgcgggtgacaccgagaccgcgaaggcgacctacgcaaccgcgaaggccgctttcgccaagtccgacacgcatacgatcgccgattactaccagcgcaacaagcccgcccgtggcggcctggtcatcgtgcgcccgaccgtgcaggcgctcgattccttcgtcaaggccaagaccagcggcagcgtcaccccgacgccctccgacgccacggtcagcacgaacggcgtgggtgccgcggcatggcatgagaacgtcgatccgaaggccgtcatcgacggtgacgacagcacgttcttctggatgcagtccgccggctgcgactgtgtcaaggccaacgccgccctcaccgtcacctacgccgaggcccgcaaggccaaggagttccgcttcatccaggcggaaaagggcggtgacacgatcgtcaacggcaagatcgaataccaggatgcagatggcaactggaccaagatcggcgacgtgaacggcaaccagaagcagatcttcacgctggactccgccgcgaccgtcaaggccgtgcgcatcaccaacttggcccagacctccaagtggtggaaggtgtacgacctgtccgccaccaagatcgacgaacccggtacggtgaccaaggacgcgctgaacgccaaggtcgccgaagccgagaaggtcgactccgccgactggaccaagtcgagccgcgaggctctcgccgacgcgattgccgccgccaaggccgtcgctgccgaccaggacgccacgcaggccaaggtcgacgccgccgtcgccgcgctcgaatcggcgatgaagggtgtcgaacggtacacggcgaagaccgccgaccagctgaaggccgagcacgtctccaacgacgatgccacctacaccgaggcgagctacaacaagtaccagtccgcgtacgacgacttcgccgccgcgctggccaacgccgacgatctggcgaaggccgacggcgaggcgctggaagcggcctacaccgccgcgaagtccgcgttgcgctacgaccagtccgcacgcgactacgcgcagctcgcgctgaacgacgccgagccttacgtgggcaaggcctccgagtacaccaaggacagctatgccaagttcaccgtcgcgtatgaggccctgagcaagcagctgaaggccgacccgaacggcgagggcgatcccgccacctacaccgcgctgcgcgctgcactcgacaaggccatcaagggcctggtcaagagcgacggcaccgagctggagcggcctggcgagaagcccggcgagaagcccggcgagaacaagcccggcgagaagccgggtgtcaacaagcccggcgccgacggcaagctgtccaacacgggcgccgacgtcttcggtctcatcgccgcgatgacgatgttggccgcggtgggcgtgacgatggccggcctgcgcaagcggatcggctga

SEQ ID NO: 35 - DNA, 5268 bp, Bifidobacterium bifidum CCOS 571
atgaaccgaagaatatctatgtggttgcgcggtcgtggctctccatggagacctgccgccgccgtgatcgccacggtatccatgatgctggcgacggtcatgggcccccatttcgcggggatgcgggcgcaggccgtcgagcccgtgcagaccaccaccatctcgcacaccaagatcgccggcgacggcaactacttcacgttcgccgacaacgcctgggatccgggcaacgacgtgcatacgtggtccaaggcgccatccgacagcctcccggcggaggacatctggtatacggtccgattcttcggcagcgcaatcgacgtctatgcaggcaagaacaggcccatgggcaaggtgaaatactatattgacggagcggaaaaaggcacgtacagcctgtacaacgcctccaacatcaacgagacgaaaatcgcgtcgttcaccggacttgacgaaggtgagcacgtgttcaaggcggtggccacaggcgagcgggacacgaattccacgaacgcgctgatcgactgcgccaaggtcgtcgtgacccatcagccgtacgtggtcaccggcgtcacactcgacacgacctcgatgacgctgggcgttggcgacagcaagcggatctcgtatacggtggcgcccgattacgcgaccatcgatgacatgacctacacgagcggcgacacgagtgtcgccacagtcggcgcagatggcacggtcaccgcggtcgcgccgggagccaccgccatcaccgtggcctcgactgcggccggcatcagcaagatcgtcgacgtcaccgtcgccaggatggcaccgaacctgaccggcggcatcgtggaccccgatacgcaatacacgcagaagcggttcgacgaggtgaaggccctcacgacgaacaaccgggcgctgaaagcatggaagaacgacaaggtcaacagcgagatctcgctcgccgcggtcggcaccaccgtctcgaacctgacggtcaccgcaaacgacctgacgtcgcagggcggcgacgtcatcgccaaaagcaacgtcacggccacgttcatcaagtccaccaaggcatacaacggcagctatctcggctacggagacccgaaccgcgaggtgcccgccgccaccgagaccaaccgctccgaaagcaacgacatcctctaccaaagcggcccgatcacggtgaaggccaatcaggtgcagaacatctgggtatcgttcgccataccgaaggacgccaaggccggcacctacaccaccacgctgaccgccaccgcagacgggatggaaacgccgctcacattcacctacaccatcgaggtgaaggccgctacgctgcccgatccggcagagtatgagaagaacttcgacgtggaactgtggcagtacccgtattcctccgcggaatactacggcgtcaccccgttctcggacgagcacctgcagatcctcagatcaagcatggaactgtacaagtccatcggcggccacgccatcacaaccaccatcaacgaggacgcatggtccggccagacctacagcgccaacgccatccactacccgtcgatggtgaagtggaccaagagcgggggcgggttcacctacgacttcaccgacttcgacaagtgggtgacgttcaacaagggactcggcatcggcgacaagatcgtgatatacagcatcgcgccctggcacggcaacttcacgtactgggagaacgggacgatgaagtccgagaaatacacggtcggatccgagcgctggaggagcgtgtggaccgacttcctgcgcaagctcatcgagcatctgatggacaagggctggttcgacgagtcgtacatcggcatcgacgagcgcggcttcagcgccgacgcgttcgacctgatcgactcgatacggaatatccacgacgtgccgttgaagaccgccggcgcgatggacggcttcgtcaacaagttcgacctggcgctgcgcgtcaccgacctgaacgtcggcgacaccgcggcggcggcccatcccaccgacttcacccggctgatcgaggcgcgtgaggcaaagggccttcgcaccacgctgtactcctgcaccgagcatgagcccggcaacttctcgctgtccgccccggtcgaaagctactggtcggtggtcaacgcgggcgagcagaccagcggcttcctgcgctgggcgtacgacgcatgggtggccgacccgctcaacgacgccacgcacaacgccttcgagcccggcgacccgttcctgatttatccgagcgagaagagcggagacaaggtgtccaagtcgtccgtgcgcctggagcgcatcgccgagggcgtgcgcgacgtgaacaagatcaggctcatggtcaccgagatcccctcgctgcaggccgatgccgacgcgatgtacgcgaagatcagaacgacggtgacgacctcgcactcgtatctgaccgccgcgcaggtcacgcagcttgccaatgagatgagcggattcaagggtgacctcgacacgctcaccgacaagtacatatccctcaaggcgcaaggcacaagcacggtggaatccgttgccatcgacggcggcgaccaggagatcatgctgggcacggcgaagcagctgaccgcgacactcaagccggcgaacctgctgaacgcgtccgtgacatggcgctcgtccaagaccggcgtcgccacggtatccgccaagggcgtggtgaccgccgccggcgtgggctccaccacgatcaccgccacgtccaaggccgacccgacgaaatcggcgagcatcaccctcaccgtgacgccacaggtcgtggcgcaggggctgcactactactcgttcgacgactcgaacgccaacgactcctggggcacccgcaacggcaccgccgacgccacggcgcaatacgttgacggcaagtccggcaaggcgctcaaggtcacggacggcaaaggcgtgaccctggccggcggcaacgacatcgcgaagacggatccgtggacgatcggctactgggtgcgttccgacgccgaactcaccggccgctcggccgtgatgacgagcgcggacggcaagtactcggccgacctcaagatggacgccgaccgcgaatctggcttccgtgtcggcaccgccagcggcgacgtgctcaccttccggtacgacttccagccgggcacgtggtattacatcgcgtggactcaggacaaggcagccggactgaccatgtacgtcaacggcacgaagatcggcgtgacgaacacgtggacgaagatgcacgatgtcgtcgccccgatcgacgtgatcggcggccccggcttcactggcctgatcgacgaggtgaagatctacaagcgcgtgctctccgacaccgagatcgcggccggcatgctgctgcccggtctcaacctcgccgagcatgagaccgatatgtacatcggcgggacgtacaccatcgtcgccaacctgcagggcggcgacggcgatggtacagtcacgttcgagtcgagcgacccgaccatcgccaaggtcgacgcctccggcaccgttaccggagtgtcccgcggaacggcggtcattaccgtccggggaggtggattcaccgacatggtgaccgtcaacgtgagccgcgaactcaccatcaagaacacgctgccgcagtacaagctcgaccagacgaaggtcacggacgtgcacaagtcactcgacacgtccaaccagtacttcggccagcccgacatgatccgcacgaagagcggccgtctgatcacctcgttcccgcaagggcacggcaagggaccgttgatcatgaagatcagcgacgacgacggcgccacctggacgcgcaagaccgacatccccgcgtcgtgggccggttcgcaggagacgccgaccctgtacgtgctcaacctggccgacggcaccgaacgcatcatgatgatcaccgcctgcccgggctggggtaccgactccgccggcaacaggtacggatggaacacatcgtattccgacgacaacggtgagacctggaccgaataccggcactggcagtccaaccgcacgtacgacaacgccaacaacgacgccatcgtcgccatggcgagtctcgtgcagctcaaggactccgacggcaacgacatccagaaatggatgggcgtctaccacaactacgcgtacgtcaatttcaggacgtacctcaccttcgacgagaacggcgacgagcagtggagcgaatcggagccgtatcttgcgcaatggcgcagcatcgaaagcgcataccagatgtgcgagatcggcatgttccgttctcccgacggcaagcggatcatcggtctggcgcgcagccagtcgcacaacaacccggcgacactgatctactccgatgatgagggtgagacgtggagcaagccgatggatctgcccggctcgctggcgggcgaacggcacaagattgcctacgatccgatttccggccgtctgctggtcacgttccgcgagatcaactacgatctcaacggcaacaaccggttcgacggcggcaacgactggaacgccggcgactgggtggcctgggtcggtacctacgaccagctcattaaccaggaggacggcgaataccgcatcctgctggccgaggactggacgagcaacgcgaagtcgggcgacaccggctacgcgggcgtagcggtgctcgacgacggtacgttcatcatggacacgtacggtcactgggacaaggaattctcgcagaactggcccggcggcgtcaccaccgaccgctgctatatcaagcaggcgaagttcaagctcggcgaggtcgaatacgcgaacggtctcatcgaccgcagcggactgaaggcggcaatcaagcgggcagaggcgctgaatgcggccgactacacggctgactcgtgggcgaagatggatgccgcagtgaaggccgcgaaggccggagacgccgacgattccctgcaacaggcgcaggttgacgcgctcgccgccgccatcgatgcggccatcgacgggttgaaggccaaggatgacggtgacaagcccggaccgggtgatggtggcaagcccggcgcgggtgacggcaagcctgacgacggcggcaagcccgatcccggcaagccgggcaagggcgacgagaccaagcccgataccggcaagaagggcgggctgagcgccaccggtgccggcatcgttccgatcgccgccgcggccctgacgctcatggccggtgcggcgctcgcactggccaagcgctga

SEQ ID NO: 36 - DNA, 4884 bp, Bifidobacterium bifidum CCOS 571
atgcgattgaggagagtgaaagcggccataggcagtgtcctggcagccgtgacactactgagtatgtcgctgaccggcgtcacggcggcgcaagccagcgatgacaatcttgcactgaatcagaccgtaacggccagttcatatgaagtggcgacgactgcgcccgagaaggccgtggacggcgatctcggcacacgctggggcaccgcgcagaacaaggccgcaaacgaatggatcgaggtcggcttgggcggcaccaagaccgtcaagcagatcaacatcgatttcgagcgcaaagatgccgatcagaacatcaccagttttaaagtcgagctgaagcagggcgacacctataccaaggtgtatcagaaggacacccgcgccaagcaacaggagatcatcctgcttgaccaggcacagcaggcgtccgccgtgaaggtgaccgtactgtccgccgacggcggcaccatgaactgggtcaacgtgggcatcaacgagatttccgtgtactccgcacccaaggagaccgtgctcgacacggccgacacgaaccacatgctcggcgccaccatgaccgcctccagcaacgagacggcgacgctcacccccgacaaggcgatcgaccagaaccgcaccggccgcaacaaccgttgggccagcggctacgagaccccgagcaacatctggctgaaggcggaattcccgcggctcaccgcggtcaaggacatccgcatctatttcttcgagcgtgacgtgaatccgaagcctaccaatgtccagagcttcgacctgtcctacaccgactccgaaggcaccgagcacacgctcaagtccggctacgcgatgacggcctccgggaccggttatgtcgctgacgtcgtcatccagctcgatcaggccgtcaacgcccgctcgctcaagctgtcgaacttcgcgatcaaaagctccgaatacaacaacgtgagcgtcgccgaatgggaggcgtattcgaacgatcaggccgagccgggcgccacgctcgacagcgtggtctccgacctcgaatccaaccacctgaccatcgagaccgacaccgacacgctggctctgcccactgtgcccgacggctacaccgtcaagttcaacggcgccgactacgagcagctcatcgccgccgacggcaccgtcaaccacccgctggtcgacaagaccgtgcaggtcgcctacgtcgtcaccgacaccgccaccggcaacaccaagacgacctccgacatcccctacgtcgtcaaaggcaccaaccagcagcaggaaggcaacaacgccaagccgaccatcatccccgaaatcgccgaatggcattcgaccagtgccgccaagctggcggcctccgccgtgacgaaggtcgtctacgacgatgattcgctcaaggccgtggtcgacgagttcgtcgccgactacaaggacttcaccggcatcaagctgaccgccaagaagggcgccgccgaagccggtgcgttcaacttcgtcaagaccgactccacggccgcgatcgcgcagctcggcgacgaaggctacacgatggacatccgggccgaccgcgtggtcgccaagtcgtccagcgtgaccggcaacatgtacgcgatgcagacgatcctgcagatgaccaagcaggacgccagcggcttcgtgatcggttcgatgcgcgactacccgcgcttcaccacccgcggactcctgctcgacgtggcccgcaagcccgtctcgctggagatgatgcgcgagatcacccgcacgatgcgctactacaagatgaacgacttccaggcgcatctgtccgacaactacatcttcctggagaactacggcaagggcgacaacgaggacgaggcgttcaaggcctatgacgcgttccgtctcgaatccagcctgaccaacgacaagggcgaatcgcccacggccgaggactactccatctccaagaagacgttcaagcagttcatccaggacgagcgcgccctcggcatgaacgtcgtgccggagatcgacgtgcccgcgcacgccaactccttcacgaagatctggcccgagctcatggtgaagggacgggtctccccgatcaacagcaaccgaccgctcatcgaccacctcgacgtgtccaagcccgagaccatcgccaagatcaaggagatcttcgacgactacaccaagggcgacgacccgacgttcgacagcgacacgaccgtgcacatcggtgccgacgagttcctctacaactacacggcataccgtaagttcatcaacgagatcgtcccctacatcaaggacacgaacaccgtgcgcatgtggggcggcctgacttggatcaacgaccacaagacggagatcaccaaggacgcgatcgagaacgtcgagatgaacctgtggtccaaggactgggccgacggcctccagatgtacaacatgggctacaagctgatcaacacgatcgacgactacggctacatggtgcccaacggcagctacggacgtgccaacgcgtacggcgacctgctgaacatcagccgcgtcttcgacagcttcgagcccaacaagatccgcagcagcggcggctaccaggccgtgccctccggcgacgaccagatgctcggcgccgcgttcgcgatctggagcgacaacatcgacaagagcgcatcgggtctgaccgaatccgacctgtactggcgcttcttcgacgcgatgccgttctacgccgagaagacctgggccgccaccggcaaggagaagggcaccgccgcgaaactcacggcgctggccgccaagcagggaaccggccctcgcaccaacccgtactaccaggccacttcgaagaacagcgtctacgagagctacgacttcaacgacgggctcgccgacgccagcggcaacggccgcgacctgaccatcggcgacggcagcaaggccgccgtcaaggaccagtcgctcaagctcgccggcggctccagctatgccacatccaagctcgacaagctcggcaacggcaacgagctgacgttcgacgtgacgctccagcaggctgccaagcccggagacatcctcttcgaggccgacgctccgtacggcacgcatgacatccgcgtcatggagaacggcaagctcggcttcacgcgagagctgtacaactactacttcgattacgagctgccggtcggcaagacggtcaccgtgaccatcaaggtggaccagcagaccacgaagctgtatgttgacggcgaattcgtgagcgacgcgaccggcaagtacatcgacaagggcatcgagaagaagaccggcatcaccgccgcgaccttcgcactgccgctgcagcgtatcggctcgaagacctctgcgatcaacggcgtcatcgacaacgtcatcgtcaagaagtccgaggccgagacagaccagtacaacaagtcctgctggaccggcacgaccaattccgagacccaatacaacgacacggaaggtctgctgcggtacgcgttcgacaacaacccgagcaccatctggcattccaactggaagggcgccacggacaagctgaccggttcgaactcgttctacgccgagatcgacatgtgccagaagtacacgatcaaccagttctccttcacgccgcgtaccagccaggacagcggacaggtgaccaaggccgatctgtacgtcaaggccaacgcgaacgacgagtggaagcaggtcgccacggatcaggtgttcgaggccagccgcgccaagaagaccttcatgttcgacgagcaggaagtgcggtacgtcaagttcgtggccaagtcctcgaacgatggctgggtcgcggtctccgagttcggcgtggcgaacaagccgtcctccaccgtgcgcgtattcgtcgcggccgatccggccgaaggcggtacggtgagcgtagccgccgagggcgaaaccggcaccgatacggccgtggacgtcgcatccggtgcctcggtgaccgccaaggcggtcacggcggatggctacaggttcagcggctggttcacgacggccagtgagacggcggtttccaccgatgccacgtacacgttcgcagccgacggcaacacggctctgaccgcgaagttcaccaaggactccacgccggatcccggcccgaagccgaccatcagctcgatcgccgtcaccaagccgaccgtcaccgattacaaggtcggcgacacgttcgacgccactggactggcggtcaccgccacaatgtcggacggcagcacgaagaccctgacggccggcgagtacacgctctcagccacgcaggacggtgccgcggtcgcgcttgacaaggcgttcgccaaggccggaaaggtcacggtcacggtcaccgccaacggcaagaccgccaccttcgacgtgaccgtgacggccaaggatcccgatccggaacccgcgacgctcaagtccatcaaggtcacgtccaagccggacaaggccacgtacaccgtggatgagacgttcgccaagaccggtctcgcggtgacgggcacctggtccgacggcaagacggcgctgctgaaggacggcgaatacaagctgtccgcggtcgacgccgacggcaagaccgtcgacttgaccaagccgttcacggccgcgggcgacgtcaccgtcacagtgacctccggcaagctcaccgactccttcacgatcaccgtcaaggcaaagaccgtgaccccgactcctggcgacaacaagccgggcgagaacaagcccggtgccgacaagccgaagccgaacacgcctgacgaggtcgccaagaccggtgcttcggtcacggcggtcgtcttcagcgccctgttgctgttgtccgcaggctacctgctggtgcgtaagcgcaggatctga

SEQ ID NO: 37 - DNA, 5883 bp, Bifidobacterium bifidum CCOS 571
atgcgcagcaaggcattaggaggcctgcttgccgcggctctgtcgttgagcccggcagtggccatcggcgtgcagacggcgtacgcggcaggcggcgatacggcggcgaccgaatacacgctgtaccccaagccgcattcgatccgttatgacagcggacagtacattcttcgcgacatcaacgtcatctatgacgatgacatcgatgaagccacccaggaccgactggacgaagtggcggcgctcaagaacctgaacgtcaccgaatccgacgccgcagtcagcggcaagaccaacgtctatgtgggcgtgaacggttccgatggcaaggccgagactgccatcgaaagcaagtacagcccggattccgccatcttcgacaagaccgactcatacttcctcaagtccgacaacggcacgatctccgtgctcggcaaagacaccgacgccagcttctacggcctgaccaccctgtaccaggtgctcggccagatcgatagcctgacgatccgcaacttcaccgtcaccgactacgccgacgtggtcagccgcggtttcatcgaaggctactacggcaacccgtggagcactcaggaccgcatcaacctgatgaagtggggcggctactacaagctcaactcgtacttctacgcccccaaggacgatccgaagcacaactcgcagtggcgtacgctgtacacgcaggacgagctcgacaccaagatcaagccgctcgccgatgccggcaacgcctccaagacgcgtttcgtgttcgctctgcacccgttcatgaacaacgcgattcggttcaactccgaggcgaactatcaggccgatctgaaggtgctgcaggacaagttcgcgcagaccatcggggtcggcgtacgccagatcgccatcctggccgatgacgcggcgaacgtgggtggtaacaattacaccaagctgctcaccgatatggtcgcgtggctcaaggaaatgaagaagacctacccggacctcaagaccacgctgccgttcgtcacgcaggaatacatgggcaacggcatgagctacttcgccaacttccccaaggaagtgcagatcgtcatgaccggcggacgcgtctggggcgaggtctcgcagaacttcaccgacacgttcacctcgaacgtcggccgcggcccctacatgtggatcaactggccgtgctccgacaactcgaagagccacctgatcatgggcggctacgacacgttcctgcatccgggcgtcgacccgtcgaagatccagggcatcgtgctcaacccgatgcagcagtccgagccgagcaaggtcggcatcttcggcaacgccacctactcgtggaacatctggcggagcaagagcgaggccgaccaggcatggcaggattcgttctcgttcgtcgaccacaactccgctgtgccgaccgccgcgtcgaacgcgctgcgtgagctgtccaagcacaccatcaaccagaacatggattcgcgcgtcaccgcgctgcaggagtccgtggacctggctcccgcactgaccgccgccaaggcgaagctggctgacggcaccatcaccgcccacgacctgaccgacatcaaggccgcgttcgtcacgctgcagaaggcagccaagacctaccgcgccaagggcgatgcgaagatgctcggcgacatcggcaaggactacaccgggcaggacgccaacgagcagatcgccccgtggatcgactgctgggatgacaccaccaaggccgcgctcgcctacatcgcgggtatcgaggccgcgctgaacggcgacacgtcctcgacgctcaaggagtactccgacgcgcagtccgcgttcgccgcgtccaagaagcacggcttctactacgtgaaccacaccgagtacgccgaagtcggcgtgcagcacatcgtgccgttcatcaaggcgatggactcctacctgtccaacaaggtgcagcaggaggccgacccgaacgtcgtgaccaagacgtacatcagcgacgtgttcaccacgccgacctccggctcgatcgaagacatcttcgacggcaaagacagcacggtcacggtgttccagaacccgaactacctgcacaagggcaactacgtcggcgtgaagttcagcaaggccaccacgctcaagagcatccgcttcgcgttcaacggcggcaagaaccacttctaccactccaagctgcagaccaccacggacggcgagaactggaccgacgtgccggatgcgacgttcgagcgcccgaagggctccgaggagccgatcaaagtcaccggtctgaacatcaccggcgtcaccggcgtgcgactgatcgccaccgccgacaacggcgatgacctgtggctcggcatcaagggcatcgacgtcaacaaggtcgagaaggagactctcgctccgtacacggcgactggcgtgcagctggagaacctcaacgccacctacagcagcaccaaggagcagatgatcgacggcaacccgtccacgatcacctacctcaaggacccgaacggcgacaagatcgcggccggcgcggccgtgatcgtcgatctgggctccagcaagccgatcggcgaggtcacgattaccggtcatgcctccagccccgacgaccgtccgagccagggcgtcgtcgaggtcagcgatgacaaggccacctggaccaagcttggtgacctgagagacgacgtcacctccacggtgagcggcaacgtgaccgggcgctacgtacgcatccgcaacaccgccgccaagaacgtgtggtggcgcgtggccgagatcaccgtgaccccgcccgagaccgccgatccgctcaagtcggtgtacacgaacaagacgcagcacgggtacaccgccacgctgggcgccaatacggcggagctgttcgacaaatcgcacacgatgcttgacggcggccagtacgccggactcgatctgctggcgatccgtgatctgaccgacgtcgagctgaacaccggtaacgcaaaccccagcctgcagatctccgacaacggactcgtctggaccactgtcgagccgggcaacctcacgggcaagaccgcccgctacgtgcgcgtgatcaatggcaccgacggagcggccttctcggtcaacaagctcaaggtcggcttttccacggtcggcaagttcggcaagctggtctcatccgacatccagaagcgcaacgattggggaaccgacacccgcgaaagcggcaacgcgttcgacggcgatatgaccacggtcatcaagttcgccggccagccgcgacagggcaacaccgcggtgttcgatctcggtcagccgatcgacatcacctcgctgcgcatctacacgcaggacacgcagtacgactacatccgcgacaccaaggtgcagatgtccgtcgatggcaagacctgggttgacgcgttcgagattggcgacggcgtgtccgacaccgacaccacgaccgcgttcggcgacataagcgacacgaacaagaagaccgattccaactacccgaacgtcttctactacggcaaggacgacatcgccaacggcaccggcatgcgctacctgcgtctgctgaccaccgccgactacccgcagcgtgcactcgcgttcaacgagttcatggtgaatcagggcgcctacgtctccaccgaggcgaacgcggcgttctccgccaccaaggtcgaggagcgcggccacgcgccgagcaacatgatcgacggcgacctgaccaccacgtacaagccgagtgcggccaatggctccctcacctacaagatcgatgacccgagcgacatcaagtcgttccgcatcgtgcagtcgggtgccgccagcggtgcgaccgtcaccggtacggtgtacgacgcggcgaccggaaccactgccggtgtgacggctcgtgcagccgcccgctccgcctccgaggtgacgttcggaacgctggaacaggcgatcaacgagttcaaggtgccggacggcaagcagctgctcagcgtcaagatcgcgtggggtaacgccatccccgagatctccgagttcatcacgctcgactcggccgacaccgacgccgacatcaccacggccaaggcggcgctcaaggagaagatcgacgcgaccgtcgacacttccgcctggaccgcgaacgccaagaccgcgtatgacgaggccaaggccaccgcccaggctgtgtacggcagcccgctggtcggcaaggcttcgatcgacgccgcagccagcgccgtgcaaagcgccatcgacgccgcgcagaccaaggccgacgccgccgcggtcgccgcgctgcgcaagctcgtggacgcagccgtcaccaacgacggccacttctacacgacagtgacgttcaccgcgtacaccgacgcgctcgacgaggtcaaggaagcgctgaaggacacgaacaacctgtccacagcagacgccgcaagcctcaagaaggccgtcgatgacgctctcgccgcgctgaaggactccacctaccagcgtgagctcgcgacgatcgccgtcgacagcttcgccacgatcgacgaggccgactacaccacgaactcctacgcggctttcaaggccgctaaggaggcgctcgacaccctgatcgccgccgacggcaccaagccggccacgttcaagaccaagaccgccgagtacaccaccgccaagaccgcgctggtgaacgtcgccgccctcaaggcccagatcgcgcacgagagcaactacgtggaggcgaactacaccgccgactcgtggaaggcgtactccgacgcgctcaaggccgcaaaggcggagctggtcaacggcaccaccgattcggtggccgccgcgctgaccgcgctgaccactgccgagaacgcgctggtgcgcaccacgacgccgcccgacaccaccgtgctcgacgagaccatcgccgacatggaaaaggttaacggcagcgagtacaccaccgacagctacaaggccctgaccgacgccatcgccaaggcgaagagcgacaaggccaagggggatgccggcctcaaccagcagaacatcgacgccatgaaggcggcgaaggaggccctggtctccaccgtcgaactcaaggcgaaggtcgccgaagccggcaaggttgactcgtccaagtacaccacggccagctacgaggcgctctccaagctgctcgccgcgaaggacgacaccacctccgacccggtcgtcaagggtctcgacacgctgtacaagtccggcaccgtcaaggagctcgccgagcgcgtcgccgccatcgacgccgcggtcgccaagctggatgcccgcgccaccggtgtcaaggactacgtggacggcatcaagctcaaggacaacgacaagggctactacaccgacgccagctacaaggcctactccgacgcctacaaggcgctgaagaagctggccgccgccggtgaaggcgaagtcgggattgccgagttcaccgaagccaaggaggcgttcgaagccgccgaggccaagcttgcctacaagtccgcggactacggcaagatcgatgacctgctcgccaaggtcccctcggacctgagcggctacaccgccgactcggtggcgaagttcgaggcggccaagaaggccgtgaagcgcggactgaccatcgaccagcagagcaaggtcgacgcgatggccgacgcgctcgaagccgccatcaagggcctgactctcaagtcgcaggcacccggtggcaacaagggcgacggaacccagagcggcactcataagggtgacgacatctccaagaccggcgccgacgtgcaggtgttcgcgatcatcatcgcgctcgccacgtgcgctggcctgggcgccgtggcctacgcccgtcgccgccgcgaggcgtga

SEQ ID NO: 38 - DNA, 5772 bp, Bifidobacterium bifidum CCOS 571
atggcgacactcatgtgcggcctgatcacatccggacgtctcgcgcgcgccgtggaaccggcgatcgccggcgtcacggcgagcggtgccgccgcggacggccatgctgcggccgccgcagtcgacggcgatccggcgacctactggcagtcacccgcagactcgtcgatgcaggactaccgccgcttcctcgacttcgacctgcacggcacatacagcatctcgcagatcgacatcaccaacctcgccggctcgtactaccactacgaggtctatctgtccaaggacggcgccgattacggcaaggtggcctacaagagcgatgacgcccccgcgaccggtgccgccgacacgcatcccatcgatgccaccgaagccgcatacgcgcgcatcagcgtcagctacaactccgccgcccagcaggtcaacctcgccgaagtcgctttccacggcaccaaggtctccgacgagcaggccagccccaaggccatctccgtcaccgacttcgactcaagctcgtggggccgggagtgggcccgcgtagagaccgacgccgactatgccgccgagaagaccgtcaccgaggtcagaaacctcgtcggccgcgtgatcggcgagcggtgggtcgacaagttcgacttccagctgcgcggcaaggccgacggcaaggacgtgttcgaaatctcagacgccggcgacgaccggatctccatccgcggcaacaacggcgtctcgctcgcatccggcctcaattattatctgcgccactggtgcaaggtcgactacaacccgctgttcggctcccagctgtccatgccggagagcctgcctgcagtcggccggaaaatcctcaaatacacgaactacgagtaccggtacgcgctcaacttctgcacctactcgtacacgatggcgttctggaactgggatgattacgagccgttcctcgactgggcggcgatgaacggcgtgaacctcatgctcgacatcgtcggacaggaggaggtgctgcgcgagacgctcacccaatacggctacagcgacgacgaggtgcgcgaatacctgtccgggccgggatactacgcatggttctacatgcagaacctgtactcggtcggaggccccctgcccgccgcatggttcgagcagcgcgtcgagctcggccgcaggatccacgaccgcatgcaggcgtacggcatcacgccggtcatccagggcttcggcggtcaggtgccggtcgacttccaggagaagaacccgacgtcggtggccgcgtcgtccggcacatggtccggtttcgaccgcccgtacatgatcaagacgtatctgaccgacgccgacaaggcggccggcaaggaggactacttccagaaggtcggcgacacgttctacaaagctcaggagaacgtgttcggcaaggtgtcgaactactacgcggtcgatccgttccatgagggcggcacgattccagacggcttcgacatcgtcgacatctaccgcaccgtgcagcgcaagatgctcgaccatgacccggcggccgtgtgggtgatgcagcagtggcagtggggcatcgacgagacgaagctctccgggctcgcggacaagggtcaggcgcttgtgctcgacctgcagagcgacctgcgctcgcaggccagcccgatggagaaccagggcgtgccgtgggtgtggaacatgttgcacaacttcggcggacgcatgggccttgacggagtgccggaggtgatctcccaggacatcacgaaagcctacaactccagcggttacatgcgcggcatcggcatcacgcccgaagccatcgacaattcgccgatcgtctacgagctgctgttcgacatgacctgggagcaggatccggtcgactatcgctcctggacgcaggagtatgccgagcgccggtacggcggaaccgacgggacgatcgagaaggcgtgggacatcctgcttgacaccgcctacaagcacacggacggcgaatactatcagggtgcgggcgaatccatcatcaacgcccgcccgtccgacaacaccatcggctcggcgtccacgtggggccacagcgacatagattacgacaagcggcagttcgagaaggccgcggccctgttcgagcaggcgtatgactcgtacaaggactcggccggcttccgctacgattacgtcgacgtgatgcggcaggtgctggccaacagcttccaggaataccagccgctcgccgggcaggcgtacaagtcgggcgatctggagacgttccggacactgtcgtcccggatgctggacatcatcaaggcgcaggacaagctgctttccagctcggacgacttcctcgtgggcgcatggatcgacgacgcccgcacgatgctcgacggcgcggacgattggaccgccgacctgttcgagctcaacgcgcgtgcgctcgtcaccacgtggggtctgaacaagaacggctcgctcatcgactattccaaccgccagtgggccgggctgaccggcgactactactatcggcggtggaagacgtacgtggacaaccggctgaacaaactggagcacggcaccgacttcaccgacccggactggttcgactacggctggcagtgggcgaaccgcaaaagcgacgaggacgggtatggtttcgcgaccgaagccgcggatgacgtcgaccagaaagcgctcggcaagatcatcctcgaccagtattcggtcaccgcgatggacgacgtcaccgacggtggcaccgcggtcgaacgcacgaacctggcgctgggacatgacgtgaccgacgaggacaccggcaccgtcgtccctgacgtgaccgacggcaacaccgacaccggctggacgcagacgggcaagaccgacgccacgctggtggtcgacctcgacggcacgtattcgatcaccggcgccggcatcaccctgcagcagatcgcggccgacttcccgctgcgctacgagatcgatgtctggaacggctcgggatgggtcgagataggccgcagcgaagccgatgccgtcagctccaagaacgaggtcgccgccgacatactcggctccaaggtgcgttggaagttgcattcgacgaacgggcgggacctgaccggcatctacgagctgtccgtctggggagccgcgcagccgcagcccgagtacacgaatctggcgcttggcggcgccgcaagcgccggccccagcgagcggcccgcgtcgaacggcaacgacggcgacgacggtacgctgtgggtcggcaacgggtcagacccgaactggtatcggatcgacctggcgtcggcgcagcgtgtggaccgcgtgcggctcgtgttcgagacggccggccgcctgttccagttcagggtcgtcgcggggctcgctgacggtaccgagcggacactgatcgacgagacgcagaaccagggcgccctcgatcaggtgtatgcggcgaatcttggcgaggaggtcgaacacgtcaccgtggagttcacggggtcggtcggcggcaccgcatggccggcgctcgccgaactcgaactgctgcaggaggccggcgacaccatcgaaggcgtgaacatcgccacctcggccgccatcacgtcgtcgcccaccaaggacgcgcccgagaacgccggcgcgctggtggacggcaaggcgaccgcatgggtgtcccgcgacggcgccacgccggcatggttccagctcgactacgccaaggcccgtgaggtcgacagcatacggctcaagttcgaggaaggccagcccgaccgcagcatgcagttcacgttgaaggtgatcgacgcgaacggcgacgaacatacggtcgccgaacgaaccgaagccgacctgagcaaacagcagggcatcgtgatggacgtgccggtcggcatgagcatcacacgcatccgcatggacatcgccgacgcccgcatcccctccagcggctcgcccgcatggccgctggtgtccgagatcgaggtctacgcgacgcccggcaacgtggctcgcgacgccaagacgacggcctcggacggctcgacgctcacggccgccgacctcgccaagctgacggacggagaccgcgacagcgcggccaccttgacggccacggccgacaagaccctgacattcacgctcgcgaaggccgcggacatcaacatgctcggcctgctggcctccggtaacagcgagccggtgcggttcaaggccgaataccgcgtggtgccgcaggacggcggcggtgcgggcgatggtgcagccgaccagtggaagacgctgaccgactattccggcaatgcgcagatgaagccggagatcgtggcccgccttgcacggcccgtctacaccgacgcggtacgcatcaccgtgctcaacgagaaccccgtcgccatcaacgagttgtacctgtatcaggcggatgcaggggcgtctctggaaagctacctctcgtccgtcgagaccgtgctcggcaagctcaccgtcggcgaatacgccggcaacgtcacccgggcggcgaagaccaagctcgaagtcgtgctggagcgggcgcgggcggcgctggacgccggactgacctcgcgcgaggccggccggtggacgacaaccgtcgaagacgcggtgtccgagttctaccgcaccggctacgtgtcgctcgaccgcaacgcgctgtatgtggcgatcgatgacgccgcggcgctgatcgcgtctctggacgcgcatggcctgcccgcgtcgtcggccgcattggccgaggcgagggcaagcgccaagcaggtctccgacgcctacggcacggtgacgcaacaggatctcgatgacgccgcggctgcgttgcggcggtcggccgacacggcgctcgcgcagcttgacgcgcaggagcgctatcaggtcgtgctggatgcggcggtcaagacgctggaggacgcgcagacggcgggcagcgtcggcgaatacgaggggcagcatccgcaaagcgccgcggacgctctgcgccaggccatcgacgacgccaaggccgcacacggtgcagccgccggagacgccgataaggtggacgccgcggcggacgcgctgcgccaggcgacgaccgcgttcaacgagtcaatcgtgcacatcgatgcggccgcgttggatgcggcgaagcgggcggcgaccggtctggtcgaatcgcagtacgacagggctgcgtgggcgacgatgcgtgaggctcttgcggccgccggagacaccgacatggcgcacatctcccaggccgacgtggacacccttgcggcacggctgaatgatgccatcgccgcgctgtccgacgcgcgtctggaccgtggcccgctgtctgacgccatcgcgtcggctcaggctctcaaggaaggcgattacactgccgaatcgtggaaggcgttcgccgaggcgttggccgccgcgcaggaggagtgcggacggcgatccaccacgcagggcgatctggacaaggccgtaaaggccctgactcaggctcgcgacgggctggagcgcaagcagcccggcggcggtgaggaaccaggaggtggcgaggatcccgagcagcctggcagcggcgggcagaccgagcgtcccggtggcgtcaagcccggcgccggcggcaacgccgatacctccaaacctggcacggcgggcacggaaaccctctcgaagacgggcgcccagacgctgctgctcgcagtgacggcgtgcatcatgcttgccgcgggattctccatcacgacggcgcgctcccgtcgccggtga

SEQ ID NO: 39 - DNA, 3339 bp, Bifidobacterium bifidum CCOS 571
atggagaaaagctccaatagacgtttcggtgtgcgtaccgttgcggccattgtagccggcctgatggtcggtggcatgtgcaccgcgatgacggccagcgccgccgacgatagtgcagccgggtacagtgccacggctcccgtgaatctcacccgcccggccaccgtcccgagcatggacggctggaccgacggcaccggcgcatggacgctgggtgaaggcacccgcgtcgtgtcgagcgatgcactggccgcgcgtgcgcagagcctggcatccgagctgaccaagttcaccgacgtggacatcaaggccgcgaccggttcagcgacgggcaaagacatctcgctcacgttggatgcatcgaagaaggccgaactgggtgatgagggattcaagctgtccatcggctcgaagggccttgaggtcatcggcgcgaccgacatcggcgtgttctacggcacccgttccgtctcgcagatgcttcgccagggccagctgaccctgcccgccggcacggtcgccacgaagccgaagtacaaggagcgcggcgctacgctgtgcgcctgccagatcaacatctccactgactggatcgaccgtttcctgtcggacatggccgacctgcgcctcaactacgtgctgctggagatgaagctcaagccggaagaggacaacaccaagaaggccgccacatggtcgtactacacgcgcgacgacgtcaagaagttcgtcaagaaggcgaataactacggcatcgacgtgattccggagattaactccccgggccacatgaacgtctggctggagaactacccggagtaccagcttgccgacaactcaggccggaaggatcccaacaagctcgacatctccaacccggaggccgtgaagttctacaagacgctgattgacgaatacgacggcgtattcaccacgaaatactggcacatgggcgccgacgagtacatgatcggcaccagcttcgacaactacagcaagttgaagacgttcgccgaaaagcagtacggagccggcgcgacaccgaatgatgcgttcaccggcttcatcaatgacatagataaatacgtcaaggccaagggcaagcagctgcgcatctggaacgacggcatcgtcaacaccaagaacgtctccctgaacaaggacatcgtcatcgaatactggtatggtgccggccgcaagccgcaggagctcgtccaggacggatacacgttgatgaacgcgacccaggccctgtactggtcccgttcggcgcaagtgtacaaggtcaacgccgcaagactgtacaacaacaactggaacgtcggaacctttgacggcggacgacagatcgacaagaactacgacaaactgaccggtgcgaaggtgtccatctggcccgacagctcgatctaccagaccgagaacgaggtcgagaaggagatcttcgacggcatgcgcttcatctcacagatgacctggtccgattcccgcccgtgggcgacgtggaacgatatgaaggcggacatcgacaagatcggctacccgctggacatccgcgaatacgactacaccccggtcgatgccggcatctacgacatcccccagttgaagtcgatctccaaaggtccgtgggagctcatcaccacgcctgacggctactaccagatgaaggatacagtgtccggaaagtgtcttgcgctcttcaccggaagcaagcatctcgatgtcgtcacccaggtcggcgcgacgccggaactgcgcaactgcgccgacgtgtccgtcggtcaggatcagcgcgacaccgccaatgagcgtaacacgcagaagtggcagatccgcgccgacaaggatggcaagtacaccatctccccggcgctgacgcagcagcgtctcgccatcgccaccggcaacgagcagaacatcgatctggagacccatcgtcccgccgctggcaccgtcgctcagttcccggctgacctggtcagcgacaacgcgctgttcacgctcaccggccacatgggcatgtccgccaccgtggactccaagaccgtgaacccggcctccccgtccaagatcaccgtcaaggtgagggccgcatccaacgcgaacaccggtgacgtcaccgtcaccccggtcgtgccggaaggctgggagatcaagcccggaagcgtcagcctcaagtcgattccggccggcaaggccgccatcgcctacttcaacgtggtcaacaccactgggacgggcgacgccaccgtgcagttcaagctcaccaacaccaagaccggtgaagagctcggcaccaccagcgtggcgctgaccggcagcctgaccaaggacgtggaagcaagcgactacgcggcgagctctcaggagaccaccggcgagcatgctcccgtgggcaacgccttcgacaagaacgcaaacacgttctggcacagcaagtactccaaccccagcgccaatcttccgcactggctggcgttcaaggcgtcgcccggcgagggcaacaagattgcggccatcacccacctgtaccgtcaggacaagctgaacggcccggccaagaacgtcgcagtgtacgtggtggcggccagcgacgccaacagcgttgccgatgtcaccaactggggtgaacccgtcgccacggctgagttcccgtacaccaaggaactgcagaccatcgcgctgccgaataccattccgtccggtgacgtgtacgtcaagttccagatcaacgacgcatggggcctcaccgaaaccagcgcaggcgtcacctgggcggctgtcgccgagctggctgcgacggccaaggccactccggtcgagctcaccgagcccgagcagccgaaggacaaccccgaggtgacggagactccggaggctacgggtgtgaccgtttctggcgatggtgttgccaatggcgcgctgtcgctgaagaagggcaccaccgcgcagctgaccgcgaaggtcgcgccggatgacgcggaccaggcggtgacgtgggcctccagcgatgacaaggtcgtgacggtcgacaagaccggcaaggtgaccgccgtcgcgaagggcgtggcgaaggtgaccgcgaccacggcgaacggcaagtccgcctctgtgaccgtcaccgtcaccgaggactctgaggtgcccggcccgactggcccgaccgagccgaccaaaccgggtacggagaagccgaccacgaagccgaccacgaagccgaacgacggcaagctcagcgccaccggcgccgacacggcggtgctcgccaccatcgcggctctgttcgcgctggccggcggtgcggtcgtcgcggttcgtcgccgcagcgtccgctga

SEQ ID NO: 40 - DNA, 2022 bp, Bifidobacterium breve CCOS 586
atgaacggtcaaacatctctgcaaggatggaccatcatccccatgccgcaaaccatgcagcataaagcgaacatcgcattgctgccaatgtgcggacgaatcaacgaagcgcgcgcagtcggtgacgatcggcacatacttgccgtgcagctcatcgacgacatccgcgcagccaccggattggaatgggatatcgccaccggcgaccgctggccgggattcatcaccttgacgacctttgacgacccccatgcacacccgtccggtgcatatacgctcgatgtcaccccggacggcgtgaccgtagcgggagcggatttcgagggtgtgcgtaacggcgtgcagactttgcgtcagctcatccgccaatgcggcgccgccctgccctgcctgcacatcgaggaccgacccgccttcgaaacgcgcggctactacctcgacgtcacccgcgggcgcgtccccaccctcgactggctcaaacactgggccgacaagctctgcctgtacaaatacaaccagctccagctctacatcgaacacaccttcgcgttcgactcgatgagcgagacctggcgcggttccagcccgctcaccccgcgcgacatcctcgaattcgacgactactgcgccgaacgcggcatcgagctggtcccgtcggtctccacgttcggacacctctacatggccctgcgcacgcaatccctgcgcgacctcggcgagttccccgaaaccgccgacgagccgttcggattcatcgaccgcatgcaccaccacacattgaacatcagcgacgaccgcgccttcgacctgtcatgccggcttatcgacgactacctgcagctgttccgctccgacaaattcaacatctgcgccgacgagaccttcgacctcggcaagggccggtccaagcccctcgccgaccgcatcggcgtcgcggccatgtacgccgactacgtcacccgcctgtgccgccacctcgaagcccggggcaggcggccgatgatgtggggcgacatcgccctcgaacaccccgagatcctcgaccggctccccgaaaccgtcaccctgctcaactggcagtacgaccctcaggtcacggacgagaagatccgcaccgtcgccgaatccggtgccaagcagatcgtatgcccggccgtatggtgctggaacgcgctcctgccgcgcatcgacgacgcctggaacaacatcacccgcatggcccgctacggcgcgcaataccatgcgcaaggcatgctcatcaccgactggggcgacttcggccacgtcaacgacccgcgcatggccatccccggcatgatcatcggcgcacaggaatcatggaacccgggacgaatcccggatgaggccgacatgctccgccgcatctcccgactcgaataccacgacgccagcggcgaactgcttgatatccttgctcgcgcaagccatgcggccagtttcgaatggaaccacctgatcacttggctggaacttgatgacggacaaggcggagtcaacaccggggtcctgcaaaccatcccgggactgctgccggaaaacgaacgaccggacgatgtgatccgttccctccagaacgaaagcaagacaccgtcacttgcggaatcccgacgaatgctgctccgctatctgaaacaccgcatcacgctcggcgaaaccgcagatcaccttctgcaggccagtacccgtcgaatctccgcgatcaccgcgaccgcaggaccgcggaacgcaggaaacgccgctgcattccgcatagccgtcgaggggcagcgactgctgaaccgggttggcctccgacttgcgtccgagaccgggatcactgacactttgcagccgaacaccacgtctcaacatgacgatgaggcgaaccttgctgaagcattggagatctggatggaggcgtatgcgacgcaatggagcacggtcagccgagactccgaactccgtcggctgcaagatacggtgtggaagttaacggaccatctgcgcttccaatccgtctga

SEQ ID NO: 41 - DNA, 525 bp, Bifidobacterium breve CCOS 586
atgaaatatcccgacatcccgaacgtcaccaaggaatatctggacgaagtgcggcccgccatcaacgccggcggatcatgctcggccacggccggagccaccatcggcgcccttagcccgcccttggtcgtcgatggcaccagcatcgacatcgacgccagcggcgtgcccgtggcctcgatcaactcatacagcgtgggccaatgcacctggtgggccgccgcccgacggcaacagatcggcaaaccggtggacccctacatgggccacggctacatgtgggcggccagcgccgagaaacacggataccccaccggcggcacaatccaactgggcgacgtgatgagcttcgagcgaggagtgctgggagccagcggcgaatacgggcacgtcgccatcgtcgaggaaatccacgaggacggttccatcctcatcagcgagtccggcgtcgaccaacgccgcgcctggacacgcctgctgacacgcgagcaggccgagaaccccggcatcacctacatccactag

SEQ ID NO: 42 - DNA, 1851 bp, Bifidobacterium breve CCOS 586
atgagattgtcatcaggtgatcacgctgggcgtgcttctgctcggactcgacacaggaaatggctgcggtctggcttggcagcggtgctgtcgatggccacgctggcggcattggccgcaccggcaagcgccaccgacaccatgccgtggggaggccagtatgccgataccagccatccggagcagtctgcgggagccaaccagccatatcagcatggctataccggtctggatattctgaactggaacccggacgcggataaggactcggaatacctgcgctcccgtgtaccgttgcagacccgcatcgccgccaacgccgcgacgcagaaagacccgaacctgccggccgatacggagatgttcaaccttgctggcgactacggcaacgcgttcttcgagtcgttccacgacaacagcgtgttctcgcagtacctgttcaactactggcagtacacggattattacggtacctggcatggtcagccgactgcgaacgtgccaaagagcctctacgacgagaaggcccagtctgactggactcagaaatggtttgagttcggtacgttgaatctgccgaatgccgcatataccaatgtcgcgcacaagaatggcgcgaagtcgattgcgacgatcttctattctggcaacgaccgaggagaacagacctataaggacctgcttcaaggcaagcgtgccgacggcacctatccggtggctgacaagctggtggagattgccaagtactatggttttgatggttacttcgttaaccaggaatccagtgtgaattctgctgatgtgccggcctaccaagacttcatgaagcagatcatcgatcagggcatttatatccagtggtacgactccgccacatacccgaatggcggcgtcagctatcaaaacatgttcaacgatgccaattcgccgtgggtgcaggatccgaacaagggtaaaatctctgattcgatcttcctgaactactggttcagcggcaacatgctacaagattcagctgatcacgccaagagccttggcattgatccgaagtacgcggtattcgcgggtatcgaggccggacagaagaaatttggtagcatcgccagcaacgcgaattatatgaatgtcaaccttgacgctgacggcaagccctatgtgagccttgcggcacttggcaccgatttcgtctcccacgagttgggtgacgacaagaaggtctacccgaagtatcagaaccaggtattcgaccgcgaacgccgtctgtggactggttcgtccaccggtgagaagggcacgacggatatatctgatccgtatattgatgatggtacgagcagcgatagctggaagggtttcgcttcgcagatcgccgagcgctccgtcatcgacggtccggtcttctccacatcgttcaacaccggtcatggtctcgaatggcgagacaacggcgaacagaccagcaaccagcagtggggcaatatcaacctccaagacattctgccgacatggcagtggtggattgatgccgattccgacccgctgcaagccgacttcgactatggcaagaaatatgaagcggcaccacgctttaactacaccaaggtcggcggctacgaaggcggcgattcgctggtgttgagcggcaagctgtccagcgacaacaccgtccgtctctacaagaccgacttgagcgtcgctgccggctccaaggtcgaactgacctacaacaagctcaacagcgacgattccaagctgcaactcggcctcattttcgccgacgacaccaagactatagtgccggtggacatggagacggtggggcaagcaacggctggaagaccgcaactgtag

SEQ ID NO: 43 - DNA, 1884 bp, Bifidobacterium breve CCOS 586
atggaattcaccgtatccggcactaccgtgcgattcgatgaacgaacgatgcagttcgcttttacgcgcgacggtgccgaatggaatacctgcgctgatttcaagccgaccctgcaatgcacgcaaggcaccttcgcgttcgccgatgccacttccatcacccacgaacaacgcgaaaccggcacgggaaccggcattcgcagcatcttcaccggctttgggcacagcgcatactcctttgaaacctatgtatgggtggagcgcgcctccggcgatgtgctcttcgaatggattccgctcaatgagcaagggctgaccgtcaccggtgtgacgtggcctgcggcaatcgccttcgaccgtgacgactcccacgacgtgacgcttattacccacgaacagggcgtgatgattcccaacacatggcctaccgccgtgagcaccaaagatatcaccttcgacggccgcttcgaaacggctggcggttacatgccgtggttcgcgcagctccgcgcagacggacacgggtatatcgccatctgcgaaactccatggaatgccggttacggcatcgaccatcccagcaatggcccgtacacccatatcaatacttggtttgagccaagcctcggcacaatgaattatcgccgcgtggtacgctaccagttcctcgaccacgccgatcatacggcggtgtgcaaggcctatcgttcgtacgtcaacgaacgaggtcgcctgcgtacgctcgccgaaaaggcggcgcgcaatccctccgtgcgcgacctgattggtcgttcatgggtgcacgtcggcatcaaaaccaaagtgcagcccgactcgttctactatgacaaggaccaccccgaaaagaacgattcattggtcacctttgcgcagcgcgaaaagcaaatgcgaacattgcacagcatgggtgcaggccgactgtacatgcacttggatggttgggcacagcccggatacgacaacgcacaccccgactatttgccggcttgtcaggaggcaggcggctgggaaggcatgaagtcgctggtcgacgcctgccatgagcaaggcgatattttcggcacgcatgaccagtaccgcgattactacttcaccgcgcaaacctttgatgccaacaatgcgattcggctggcagacggtacgatgcccgaacacgcacgctgggcgggcggccaccagacctacctgtgcgccgagctcgcaccggactacgtacgccgcaatttcacccagattgccgcgcatggcatcaagctcgactgtgcatacttggatgttttcacctgcaacgaaggcgacgaatgctcgaaccccgaacaccgcatgacccgccgcgaatgctttgaccgccgcaccgaatgcttcgaatatctgctctcgcacggcatcctctcctcgtccgaagaggtatcggactgggcagtgccaagcctgatattctgccattacgcgccatacgacttccagatgcgctcacccaacgagccgcgccaaggtgtgccggtgccgctgtataacctcgtctaccatgattgcgttatcgaaccatggatgatggagcgtgtggtgaacggcgacgattacatgctgtacgccttgctgaacggcggagctccatacctgattcgcgatgccgcatacatcggcgttgacggcgacatggacgacgaacagcgcgctcgcacggaaaacgacatcgaacgctgccatacggtcgctgcattccatgagcgggtcggcatgcaggaactggttcgtcacgagttcgtggatgatgatccgctggtgcagcgttcggtattcgtggacggcactgcggtcacttgcgacttccatacgcaaacctatcgcatcaccgattga

SEQ ID NO: 44 - DNA, 714 bp, Bifidobacterium breve CCOS 586
atgtcgaccgatcagttacgtcaatcggccagcgtatggggctcacagctggcagccgccggcattaacgtcgatcttgcacccgtgctgggcacggtagtggcgaatcgggccgccaacgcccccattggtgcgctctatcgcgatttcggactggacgcggcaggcaacgcggctcagggcacggcgtttgtgcagggcatggccgatgccggagtccaatccgccatcaaacattatccgggattgggcgcggtaaccggcaacacggatttcaccgccgacggcatcctggatacgaccaccaccttggatggcacggaaatcaaggcgtttgacaccaccatcgaccaggccgaccctgccatggtgatgatggcattggccacctatcaggccattgaccccaatgatcccgcggtgttttcctcaatcatcattgacgggcatcttcgcggcgatctgggatatgacggcgtagtgatttcggattcgatgtcggcagcggccgtgagcgcctacgacaccactcaattgggagtcaaactcgtggaagccggcggcgatttggcctgcatcggatacaccaactatgtcgcgccgattctggatggattgtctacgcgagcggcatcggatcccgccttcgccaatgaggtcactcagtcggcgattcgtgtgatgacgttgaaaatcaagatgggattggcctaa

SEQ ID NO: 45 - DNA, 402 bp, Bifidobacterium breve CCOS 586
gtgtcgatcggcgaggacacggccggtgtgcggttgtgcggcgaagttcgcggcggcggtctgttcctgtatcctctgggagaagggcagattcgcaaaatctccgacgtgccgcccaccaccgataccgcgttgttcgacaaaggatatgaaggatccgcaagctaccgcatcccgtctttggtgactacgccctccggtgtgacgattgccggtgccgaccaacgtgtggtcatctccaacgatgccccaatgagatccatttcgttgtccgccgctccttggatagcggacagacgtggctgccgctgcaaaccgtcatcgcctttcccggtgatgggctggatggcgcgagcgtcatcgactcatgcatcgtctgtgatcgtgagacaggccgtgtga

SEQ ID NO: 46 - DNA, 1302 bp, Bifidobacterium breve CCOS 586
atgtccacctttccacagctggccacccatccgggcatgaacccggccgcggtcatccaaggcgaccgttggcgcatcggcatcatcaccgaatcgctcgtccgcctcgaatggcaggacaacggcaagttcgaagaccacgccacccaaatgatcgtcaatcgcgattggttgtcggatgacgcgaacggtgcggatggcgcgaaccgtgcggacggcacttcaaacccgccgaagttcacgaagaccgagcgcgacgggctgctcatcatcgatacgccggcgctgcgcctcacctacgacatgcagccgttcagtaaggaaggtctgagcatcgtcgtcaaaggcgtggcgaattcccagatgaatacgtggcactacggcgaagcccaggacggcaacctgcgcggcaccgcgcgtacgctggacgcggtcgacggtgagatcgaactggggctcggcgtgatctcccgcgacggctgggccgtgctcgacgattccgcatcaaacgtgatcgtcgaaggcgccgaagccgccaccgtcaagggcgaggccaacccattcggtatgtgggtcattccgcgcgagcaccccggcaaggatctgtatgtcttcggatacggccatcggtacatcgaagccgtgcaggacttctacaagctcaccggcccgacgccgctgctgccgcgcttcgcgctcggcaactggtggagccgctaccaccggtacacggaagccgagtatctggagcttgtcgatcgcttcgagcaggaaggcctgccgttcaccacggccgtcatcgacatggactggcatctggtcgacaatgtcgacccgaagtatggatccggatggaccggctacacgtggaaccgtgaattcttccccgaccccgagcgattccagcgcattctgcacgagcatggactgcgcacgacgctcaacgtccacccgcgcgacggcgttcgagcatttgaagacggctatgccaaagtcgccgaacacatgggcattgacccggcgggcggcgagccggtcgagttcgatctgaccagtccgcgattcatggaagcgtacttcgacctgcaccatgggctcgaaaccctgggcaccgatttctggtggctggactggcagcagggcggcgtgacccgccagaagggtcttgacccgctgtggatgctgaaccacatgcattatctcgactccgccgtgacgggcgctggccgctcacgttctcgcgatatgccggcccgggctcgcaccgttatccggtcgggttctccggcgacacagtcgtga

SEQ ID NO: 47 - DNA, 1017 bp, Bifidobacterium breve CCOS 586
gtgattgatgtttctgcctggcagggcaatatcaactggcaggccgtgaaaaactcaggcgtggaaggcgcaatcattcgcattggctacgggtgggacaacgggtttgacaagcaggcacttcgcaatatcagcgagtgcaggcgtttgggtattccgtttggcatatacctctattcgtacgcttatgacgccaataccggtgctgctgagggatccagtttagtgaacctgctgcagaaagccggtgtgagctcaagcgatttgggctatccggtgtattacgacttagagaggtggacctggacgggtcatgaggtgcccaacgaccctgggacgtatgacggcattgtcaatgcttggtatggcaggttgcaatccgctggatacaacaatcttgctgtgtattcatacacttcttatctgaatactgcgctcaatagtggcaatatccactctaagacccgttgggttgcgcagtatggttcctcgatgggctatacggcattccccaccaacgaccgtggctggcagtacaccagcaggggcagcgtgagcggcattagcggcaccgtggatttgaatgcgtttggtaatcaaactgccacgtcctcggctcctagcgttcctgtctaccgtgtctacaatcccaacagcggattgcaccattacacgatgaattacaacgaagtcataatgctggttggtaaggggtggcgatacgagaaaaccgcctttagagcgggccaatccggcatacctgtctaccgtgtctacaatccgaatgacggaaaccatctgttcacgatgaatagttacgagcgagacaatctggctcgtttggggtggcacgatgaaggcgtgtcttggtacgtgccttccggcggatccattaacgtataccgtttgtataacccgaacaatggtgagcatgttttcaccacggaatatggcgagtatgtgcttgttggcagggctggatggcatcaggaaggcgttgcctggacatctctgtga

SEQ ID NO: 48 - DNA, 375 bp, Bifidobacterium longum CCOS 974
gtggggattccagttcgatccggcgggtatcagctcatcggagccaagaagaccttcatcgacgagatgaaccaatggatgaaaaccgaatccaacaagccgttcctgttcaccgaatacggtgcggacaccgatgccggtgtgcacaagctgccgagcgtgcaatggagtgaagagtaccaatgtgagtacctcgccatgcagcacgaagtgttcgacatgttcgaggcagtagtgggcgagcaggtatggaacctctgcgacttccaaaccggtgaaggcatcatgcgcgtcgacggcaataagaagcgtcttcactcgcgaccgtcagcccaaagccgccgcctatgtactcaaggagcgttgggagactaa

SEQ ID NO: 49 - DNA, 1203 bp, Bifidobacterium longum CCOS 974
gtggcgacaatatgtgctttggcagtggtgttggccggcgtggcagcctacggatggcatgtcggatggttcgccaaatccacatcaaacggcaacaccaccactccccagacctcccagacaagtgcgttaccacgcgccgacgttccttccccgaagaagaacgaaccggccgcacaagcccaacgtgcggtatccgccatgacacttgaggaacgtgtgggacagttagtgatggtgccgttgcttgccggttccgatccctcctcgttggcttcaacaatcgccgatgagcacattggctcggccattctcattggcaattggaataccggcgtcgatacggtcaagaccgcgaccgcgcaactccaaggatatgcgccggccggcaatcgtctcatcatcgccaccgatcaggagggtggtcaggtgcagcatctgactggtaccggtttcgacacaatgcccagtgccgttgagcagggcacaatgtccgctgacgcattgcgtcaatcggcaggcacgtggggttcgcaattagctgctgctggcataaatgtcgatttggcaccggtgctcggcacggtggtgggcgatcgtgcctcaaatactccgattggcgcgctggatcgtgatttcggattggatgcggccggcaacgccgaacatggcatcgccgttattgaaggtttgcgagacgctcaggtcggcgcggcggtcaaacattatcctgggttgggcgcggtaagcggcaataccgacttcaccaccgaaggcattctggatacgaccaccacgttggacggggccgaggcaggtgcctttgaccaggcgatcaccaagaccgatcccgcaatggcgatgatgtcgttggccacgtatcaatccatcgacccgaataatccggcggtgttttcttctacgattatcgacggtcatattcgcaacgccctgaagtacacgggcgtggtgatttcggattcgatgtctgccgaagcgttaagcagctacgatgtaagccaattgggagtaaagcttgtcgaggcgggcggcgacatgtcctgcatcggtcagacggattacgtaaagccaattgtggacggcctcaacgaacgggcgaagtccgatccggctttcgcttcgaaggtgacggcggcggcgactcgcgtaatggcattgaaaatcaagatgggactggcctga

SEQ ID NO: 50 - DNA, 1896 bp, Bifidobacterium longum CCOS 974
atggaattcaccgtatccggcactaccgtgcgattcgatgaacgaacaatgcagttcgcttttacgcgcgacggtgccgaatggaatacctgcgctgatttcaagccgaccctgcaatgcgcgcaaggcaccttcgcgttcgcggatgccacttccatcacccatgagcagcgtgaaaccggcacgggaaccggcattcgcagcatcttcaccggctttgggcacagcgcatactcctttgaaacctatgtatgggtggagcgtgcctcaggcgatgtgctcttcgaatggattccgctcaatgagcaaggcctgaacatcaccaatgtgacgtggcccgcagccatggacttcgattgcgccgacgaccatgacacgacactcatcacccatgagcaaggtgtgatgatccccaacacatggcctaccgccgtgagcaccaaagacatcgccttcgacggccgcttcgaaacggctggcggttacatgccgtggttcgcgcagctccgcgcagacggacacgggtatatcgccatctgcgaaactccatggaatgccggttacggcatcgaccatcccagcaatggcccgtacacccatatcaatacttggtttgagccaagcctcggcacaatgaattatcgccgcgtggtacgctaccagttcctcgaccacgccgatcacacggcggtgtgcaaggcctatcgttcgtacgtcaacgaacgaggtcgcctgcgtacgctcgccgaaaaggcggcgcgcaatccctccgtgcgtgacctgattggtcgctcgtgggtgcacatcggcatcaaaaccaaagtgcagcccgactcgtactactacgataaggaccaccccgagaaaaacgagtcgctggtcaccttcgcacagcgcgaaaagcaaatgcgaacactgcacggcatgggtgcaggccgactgtacatgcacttggatggttgggcacagcccggatacgacaacgcacaccccgactatctgccggcctgtcaggaggcaggcggctgggaaggcatgaagtcgctggtcgacgcctgccatgagcaaggcgatattttcggcacgcatgaccagtaccgcgattactacttcaccgcgcaaacctttgatgccaacaatgcgattcggctggcagacggtacgatgcccgaacacgcacgctgggcgggcggccgccagacctacctgtgcgccgagctcgcaccggactacgtgcgccgcaatttcacccagattgccgcgcatggcatcaaactcgactgtgcatacttggatgtcttcacctgcaacgaaggcgacgaatgctcgaaccccgaacaccgcatgacccgccgcgaatgctttgaccgccgcgccgagtgcttcgaatatctgctctcgcacggcatcctctcctcgtccgaagaggtatcggactgggcagtgccaagcctgatattctgccattacgcgccatacgacttccagatgcgctcacccaacgagccgcgccaaggtgtgccggtgccgctgtataacctcgtctaccatgattgcgttatcgagccgtggatgatggagcgtgtggtggacggcgacgattacatgctgtacgccttgctcaacggcggagctccatacctgattcgcgatgccgcatacatcggcgttgacggcgacatggacgacgaacagcgcgctcgcacggaaaacgacatcgaacgctgccatacggtcgctgcattccatgagcgggtcggcatgcaggaactggttcgtcacgagttcgtggatgatgatccgctggtgcagcgttcggtattcgcggacggcactgcggtcacttgcgacttccatacgcaaacctatcgcatcaccgactgcccgcatcactga

SEQ ID NO: 51 - DNA, 948 bp, Bifidobacterium longum CCOS 974
gtgggaatcctcaacaaaggcaagccgaaacacggacacctgcaccggcgcgtgggcatgacgctgaccgcgcttgccgtcgcggtctccatggcgttcgccccggcggcgatggccgacatgcagggcgtggacatgagcaactggcagtgcggcgcggacgtgtacaacatgcaggccgatttcatcgtggtcggcaccacatggggcaccgggcaagtcaacaacaactgcttggtgtccggcgtcaacacggacgccaaccgcatgatcgcccaggcacaagcatccggcaagaaattcggtttgtatcactacgcgatgggaggcaacccggaggcggaagcccaattcttctatcgcaacacgtcgaactattggcgtcacggcatcgtggcgttggattgggagatggacgacaaccccgcatggggcgattgggattgggtacgccgattcacggcggagtgtgaacggctctcgggcggcgtcaagccgctgctctacaccggccccgtggccggcaccatccccggcgacatccgcgccaactacggtttgtggatcgcgcagtacgcgaacatgagcccgaccggctaccaggccaacccgtggatgctgggcgcgtacggcgaggccatgcgacagtacagcggtaccggcgtggtcaacacgtggagtcccatcgacctcaacatcttccgtggcgaaggctggcagtggatctgtacgccaaccccaccggctccacagccccggccccggcaacgcccgcgcccgtgcagccgagcactcccacggccaacaccaacacgggtggcatcagccacgtcatgcaatggggagaaaccatctggggactcgccgtcgcctatgatgcttggcccctgtccgcgtggcatacgccgagcggtgacatcaaccgctactacgtgggcgacgtcgtaa

SEQ ID NO: 52 - DNA, 2136 bp, Bifidobacterium longum CCOS 974
gtgcccacattcgaatataaggctgatgccgcaacgccgtgtctcaccctgattcccgctccggtgacattggaatacacgcatggcacggctatgatcgggtccttggtgacgatcgagaaacgaattcccgaatatgccgtcaccgaagatgccgatgagacctgggaaacgctgccaatcgagcagctgtccagcgaactcgagcgttactgcggcgtcgccgtccgtacgcgccgagtactcacagccacagatgaagccgacgccggtgccaatgccgccgaaaaagcgcgagatgcgggcgtgggtgcgggtgcgggcgcgggtgcgccggcagcgatgaacggcaccgtcatattgctgtgtgtggatgcgcgattggcgcatgacgaatacacgctggatgtgttcgcctcagataccatcgccgtgcgtggtggcagcgaaagcggattgcggtacggcatgcagacactgcggcagatgatcaggcaaacctcgcggaccttgccctgcctgcatatccaagacaagcctgcgttcgcggtgcgcgcctacagtcttgacgtgacgcgcgggcgtgtgccgacgatggcgttcctcacctggttcatcgaccagctggcgttgtataagtacaaccaattccagctgtacgtggaacatgccttcgctttcggcgagctcagcgaagcgtggcgcggcactgacccgctcacggccgacgacatcatgttcctggacgaatactgcgcacaccacggcatcgaactggtgccgtccttggccactttcgggcacatgtatatgaacctgcgcacccgtgaacatcgtggactgggagagttccccgaagacgccgaccgtccgttcagtttcatcgaacgaatggaacaccacacactgaacgcagccaaccccaagtcgcacgatttcgcctcgcgcctaatcgaggaatacgcgccgctgttccgctcgcggtccttcaatattggtggcgatgagactttcgacttgggccgtggccggtccgtacaggactcgccgggcgccagtcgcgatgagctgtatgccgatttcgtcaaagacctatgcagcacgcttgcccatcgtggtctacaaccgatgctgtgggcggatatcgcgctcgagaatccgcacaccatggacttgctgcccggcgacatcacgatgctcaactggatgtatgagccggatatcgacgaaagcaagatccagaccatcgcatcacaaggccgccgccaattcgtgtgccctgccgtgcgtgcgtggagccggttcttccccgactatgacggtgcctggctgaacacgtaccgcatggcggtggctgggctcaaatatggtgcggaaggcatggtggtcaccgattggggtgactatgggcatgtcaatgatccgcggttgagcgtgccgggactgtgctacggtgcgcaaaacgcgtggaacccggttgcaattgacgcatgcgaaatgaaccatcggatttctaatctggcgtatggcgacgaatccggttggcttatggattcactcgctcgcatcgactccgatggagtgtcgttcccctgggacctcgccgtgcaagtgctggaactggaatacggttccggcaccggcatgctgaatacggatgtggcatcgtatgtggaacggtcgtgcgggggagagctcatgtttgaccgtgcgctgggatgcgccgacgcgcgccgccgattgctcctgcggaaccatgcccgtctcgaacgacgccgggattgcgaccgggcgttgattgattgcggcagtgcggttgtcgcggtgctcgatggcttggcacgaggaggattgaacccggagctgctgtgggtgatgctggatgggcagcggttgttcaatagactgggtgaggaactgctggtattggctggcggcgaggacgcctgtgacaccaaggatgtgaccggccgtgcgctggatgcctcgcgccgcgcccgtcttgccgccgatttggagttgtggttcgaacggtaccgtgtgcagtggctgtccatcggccgttacgccgaattggcgcgtatcgcccatgtggtgtggtcgtttgcggacatattgcgtaggggagcgctatag

SEQ ID NO: 53 - DNA, 1905 bp, Bifidobacterium longum CCOS 974
atggtggaaaagaagcggctcgacggctcggatgcgaagggcgcgacgggtgcggcgcgtgcgacgggcatgctgcgtgcgttgcgtgcgcgtgcggcggcgtccggtgcggggcgcggcgtgaccgcggcggtgacgtccgtcgcggcggtggcgatgttgggcgcggtgtgcgtcactccggccagtgcgctcgcggatgtgaacgccgacgcggacgcgtccggcgtccggtccgcggcctccgcgaccgcctcggacggaacctcatccgacgcgcgctcgcaggcgcggtccgcgacttccgcgacgcgtccggtcgcgaacggtgtgacggtcgccgatgagacggctgccgacgcgatgccggacaatccggatgccgagctgccggacaaggtgtccgccgagatctccgatgacgcgatggtggtgtccgagcaatatgcggctacgccggaaggcgagttgaaggacatcgagacgggcgagacggtcaccgatccgaagatcgtgggcacggagagcaagcagcccgatccgttggcgaagacggatggcgagtcgttcattccggtgagtgccgcggatgtgaaggagaaggtcgctgcgaacggcggtgacgtgaacgcggtctcctcgaagacgcgcgcggccaacgcgtcggtgaagctcgccgcgttgcagaacaacgagtacggtgcgcactggggcacgtacaacggtacgcaggcgttcttcgacgcgcgcaacaacctgttcgcccagcaggcgaagggcgtgatcgacgtgtccgcatggcagaacacgatcgactggcaggcggtgaagaacgcgggcgtcgagggcgcgatcatccgtctgagctacggctggggcaatggcttcgacgtgcaggcgaagcgcaacatcagcgaatgcaagcgtctcggcatcccgttcggcgtgtacgtcttctcgtatgcggaaagtgcggccgacggcgcatccgagggtgcggacgtggtgaacctgctgcgccaggcaggcgtgaatccgggcgacctgagttacccggtgttctacgatctggagaactggacgtacacggggcacaagagcccaacgagtccgagcgtgtacgacggtatggtgaactcctggtacggcaaactgcaggcggccggttacaacaatctgagcgtctactcgtacacgagctacctgaacagcgcgctcaacagctccaacatccacggcaagacccgttgggtcgcccagtatggctccaccatgcagtacaccgcgttccccacgaacgaccgcggctggcagtacacgagcggcggctccatcaacggcatttccggtcgcgtggatatgaatgcgttcggcaactatcaattcactcccgcggttcagataacttgggtttatcgctctgaagatattgctgtcggagcatcggttgattacccttcatcggatattgattacaaatggcaatcgtataatttatccagcaaacgttggaaaaccatcaccgattggacaggtgccaattgggcgggttgggtggaccagttaggagactattggctacacgtggaagcacgtgactctcggactcgcaagattatcggatcgcagacaatcgctttcaggtatgcacccggtacaacgcgtgtggcggcaacatatgcgggatggcagaacaatcatgtgttgctgggggaaagttcaaataatgcggctgcccattatgagattaaaatctatgatgttagacgcagcaaatgggtgcaaggtttcaagggaccgtgggcgatttggaagcccaaaaagggtatatattggactcattatgaggtatatacctctgatgggagactcgcggacactaagacttatgcgttcggtgtctaa

SEQ ID NO: 54 - DNA, 174 bp, Lactococcus lactis CCOS 949
atgagtacaaaagattttaacttggatttggtatctgtttcgaagaaagattcaggtgcatcaccacgcattacaagtatttcgctatgtacacccggttgtaaaacaggagctctgatgggttgtaacatgaaaacagcaacttgtcattgtagtattcacgtaagcaaataa

SEQ ID NO: 55 - DNA, 2982 bp, Lactococcus lactis CCOS 949
atgataaaaagttcatttaaagctcaaccgtttttagtaagaaatacaattttatctccaaacgataaacggagttttactgaatatactcaagtcattgagactgtaagtaaaaataaagtttttttggaacagttactactagctaatcctaaactctatgatgttatgcagaaatataatgctggtctgttaaagaagaaaagggttaaaaaattatttgaatctatttacaagtattataagagaagttatttacgatcaactccatttggattatttagtgaaacttcaattggtgttttttcgaaaagttcacagtacaagttaatgggaaagactacaaagggtataagattggatactcagtggttgattcgcctagttcataaaatggaagtagatttctcaaaaaagttatcatttactagaaataatgcaaattataagtttggagatcgagtttttcaagtttataccataaatagtagtgagcttgaagaagtaaatattaaatatacgaatgtttatcaaattatttctgaattttgtgagaatgactatcaaaaatatgaagatatttgtgaaactgtaacgctttgctatggagacgaatatagagaactatcggaacaatatcttggcagtctgatagttaatcattatttgatctctaatttacaaaaagatttgttgtcagatttttcttggaacacttttttgactaaagttgaagcaatagatgaagataaaaaatatataattcctctgaaaaaagttcaaaagtttattcaagaatactcagaaatagaaattggtgaaggtattgagaaactgaaagaaatatatcaggaaatgtcacaaattcttgagaatgataattatattcaaattgatttaattagtgatagtgaaataaattttgatgttaaacaaaagcaacaattagaacatttagctgagtttttaggaaatacgacaaaatctgtaagaagaacatatttggatgactataaggataaatttatcgaaaaatatggtgtagatcaagaagtacaaataacagaattatttgattctacatttggcataggagctccatataattataatcatcctcgaaatgacttttatgagtccgaaccgagtactctatactattcagaagaggagagagaaaagtacctcagcatgtatgtagaagccgttaaaaatcataatgtaattaatcttgacgacttagagtctcattatcaaaaaatggacttagaaaagaaaagtgaacttcaagggttagaattatttttgaatttggcaaaggagtatgaaaaagatatttttattttaggggatatcgttggaaataataatttgggaggggcatcaggtagattttctgcactctctccggagttaacaagttatcatagaacgatagtagattctgtcgaaagagaaaatgagaataaagaaattacatcgtgtgaaatagtatttcttccagaaaatatcagacatgctaacgttatgcatacatcaattatgaggaggaaagtacttccattttttacaagtacaagtcacaatgaagttctgttaactaatatctatattggaatagacgaaaaagaaaaattttatgcacgagacatttcaactcaagaggtattgaaattctacattacaagcatgtacaataaaacgttattcagtaatgagctaagatttctttacgaaatttcattagatgacaagtttggtaatttaccttgggaacttatttacagagactttgattatattccacgtttagtatttgacgaaatagtaatatctcctgctaaatggaaaatttggggaagggatgtaaatagtaagatgacaataagagaacttattcaaagcaaagaaattcccaaagagttttatattgtcaatggagataataaagtttatttatcacaggaaaacccattggatatggaaattttagagtcggcgataaagaagagctcaaaaagaaaagattttatagagctacaagaatattttgaagatgaaaatatcataaataaaggagaaaaggggagagttgccgatgttgtagtgccttttattagaacgagagcattaggtaatgaagggagagcatttataagagagaaaagagtttcggttgaacggcgtgaaaaattgccctttaacgagtggctttatctaaagttgtacatttctataaatcgtcaaaatgaatttttactgtcgtatcttccagatattcagaaaatagtagcaaacctgggtggaaatctattcttcctaagatatactgatcctaaaccacatattagattgcgtataaaatgttcagatttatttttagcttacggatctattcttgaaatcttaaaaaggagtcggaaaaataggataatgtcaacttttgatatttctatttatgatcaagaagtagaaagatatggtggatttgatactttagagttatccgaagcaatattttgtgccgattctaaaattattcctaatttgcttacattgataaaagatactaataatgattggaaagtcgatgatgtatcaatcttggtgaattatttatatctgaaatgcttctttgagaatgataacaaaaggattcttaattttttgaatttagttagtcctaaaaaggttaaagaaaatgtcaatgaaaagattgaacattatcttaagcttctgaaagttaataatctaggtgaccaaattttttatgacaagaattttaaagaattaaagcatgccataaaaaatttatttttaaaaatgatagctcaagattttgaacttcagaaagtttattcaattattgacagtatcattcatgtccataataaccgactaattggtattgaacgagataaagagaaattaatttattacacacttcaaaggttgtttgtttcggaagaatacatgaaatga

SEQ ID NO: 56 - DNA, 1801 bp, Lactococcus lactis CCOS 949
atggatgaagtgaaagaattcacatcaaaacaattttttaatactttacttactcttccaagcaccttgaagttaatttttcagttggaaaaacgttatgcaatttatttaattgtgctaaatgctatcacagcttttgttccgttggctagtctttttatttatcaagatttaataaactctgtgctaggttcagggagacatcttatcaatattattatcatctattttattgttcaagtgataacaacagttctgggacagctggaaagttatgttagtggaaaatttgatatgcgactttcttacagtatcaatatgcgcctcatgaggactacctcatctcttgaattaagtgattatgagcaggctgatatgtataatatcatagaaaaagttactcaagacagcacttacaagccttttcagctatttaatgctatcattgttgtgctttcatcgtttatctcattgttatctagtctattttttattggaacatggaacattggggtagcaattttactccttattgttccagtattatctttggtactttttctcagagtgggacaattagagtttttaatccagtggcagagagcaagttctgaaagagaaacatggtatattgtatatttattgactcatgatttttcatttaaagaaatcaagttaaataatattagcaattacttcattcataaatttggaaaattaaagaaaggatttatcaaccaagatttagctattgctcgtaagaagacatatttcaatatttttcttgatttcattttgaatttgataaatattcttacgatatttgctatgatcctttcggtaagagcaggaaaacttcttataggtaatttggtaagtctcatacaagctatttctaaaatcaatacttattctcaaacaatgattcaaaatatttacatcatttataatactagtttgtttatggaacaactttttgagtttttaaagagagaaagtgtagttcacaaaaaaatagaagatactgaaatatgcaatcaacatataggaactgttaaagtaattaatttatcatatgtttaccctaattcgaatgcctttgcactaaagaatatcaatttatcctttgaaaaaggagaattaactgctattgtaggaaaaaatggttcagggaaaagtacactagtaaagataatttcaggattatatcaaccaactatgggaataatccaatacgacaaaatgagaagtagtttgatgcctgaggagttttatcagaaaaacatatcggtgctgttccaagattttgtgaagtatgagttaacgataagagagaatataggattgagtgatttgtcttctcaatgggaagatgagaaaattattaaagtactagataatttaggactcgattttttgaaaactaataatcaatatgtacttgatacgcagttaggaaattggtttcaagaagggcatcaactttcaggaggtcagtggcaaaaaattgcattagcaaggacattctttaagaaagcttcaatttatattttagatgaaccaagtgctgcactcgatcctgtagctgaaaaagaaatatttgattattttgttgctctttcggaaaataatatttcaattttcatttctcatagtttgaatgctgccagaaaagcaaataaaatcgtggttatgaaagatggacaggtcgaagatgttggaagtcatgatgtccttctgagaagatgtcaatactatcaagaactttattattcagagcaatatgaggataatgatgaat

SEQ ID NO: 57 - DNA, 1113 bp, Lactococcus lactis CCOS 949
atgttagcggagttaaaaaataaagataactcaaagatatatcagaaaaagatagacaattatattgaatatattgttagcaaactttcaacatatgggcttttaacaggatcactttattcgggagcagctggcattgcattaagtatcctacatttacgagaagatgacgaaaaatataagaatcttcttgatagcctaaatagatatatcgaatatttcgtcagagaaaaaattgaaggatttaatttggaaaacattactcctcctgattatgacgtgattgaaggtttatctgggatactttcctatctattattaatcaacgacgagcaatatgatgatttgaaaatactcattatcaattttttatcaaatctgactaaagaaaacaaaggactaatatcgctttacatcaaatcggagaatcagatgtctcaatcagaaagtgagatgtatccactaggctgtttgaatatgggattagcacatggacttgctggagtgggctgtatcttagcttatgcccacataaaaggatatagtaatgaagcctcgttgtcagctttgcaaaaaattatttttatttatgaaaagtttgaacttgaaaggaaaaaacagtttctatggaaagatggacttgtagcagatgaattaaaaaaagagaaagtaattagggaagcaagtttcattagagatgcatggtgctatggaggtccaggtattagtctgctatacttatacggaggattagcactggataatgactattttgtagataaagcagaaaaaatattagagtcagctatgcaaaggaaacttggtattgattcatatatgatttgccatggctattctggtttaatagaaatttgttctttatttaagcggctattaaatacaaaaaagtttgattcatacatggaagaatttaatgttaatagtgagcaaattcttgaagaatacggagatgaaagtggcacgggttttcttgaaggaataagtggctgtatactggtattatcgaaatttgaatattcaatcaattttacttattggagacaagcactgttactttttgacgattttttgaaaggagggaagaggaaatga

SEQ ID NO: 58 - DNA, 738 bp, Lactococcus lactis CCOS 949
atgagaagatatttaatacttattgtggccttaatagggataacaggtttatcagggtgttatcaaacaagtcataaaaaggtgaggtttgacgaaggaagttatactaattttatttatgataataaatcgtatttcgtaactgataaggagattcctcaggagaacgttaacaattccaaagtaaaattttataagctgttgattgttgacatgaaaagtgagaaacttttatcaagtagcaacaaaaatagtgtgactttggtcttaaataatatttatgaggcttctgacaagtcgctatgtatgggtattaacgacagatactataagatacttccagaaagtgataagggggcggtcaaagctttgagattacaaaactttgatgtgacaagcgatatttctgatgataattttgttattgataaaaatgattcacgaaaaattgactatatgggaaatatttacagtatatcggacaccaccgtatctgatgaagaattgggagaatatcaggatgttttagctgaagtacgtgtgtttgattcagttagtggcaaaagtatcccgaggtctgaatgggggagaattgataaggatggttcaaattccaaacagagtaggacggaatgggattatggcgaaatccattctattagaggaaaatctcttactgaagcatttgccgttgagataaatgatgattttaagcttgcaacgaaggtaggaaactag

SEQ ID NO: 59 - DNA, 2049 bp, Lactococcus lactis CCOS 949
gtgaaaaaaatactaggtttcctttttatcgtttgttcgttgggtttatcagcaactgtgcatggggagacaacaaattcacaacagttactctcaaataatattaatacggaattaattaatcataattctaatgcaattttatcttcaacagagggatcaacgactgattcgattaatctaggggcgcagtcacctgcagtaaaatcgacaacaaggactgaattggatgtaactggtgctgctaaaactttattacagacatcagctgttcaaaaagaaatgaaagtttcgttgcaagaaactcaagttagttctgaattcagtaagagagatagcgttacaaataaagaagcagttccagtatctaaggatgagctacttgagcaaagtgaagtagtcgtttcaacatcatcgattcaaaaaaataaaatcctcgataataagaagaatagagctaacttcgttacttcctctccgcttattaaggaaaaaccatcaaattctaaagatgcatctggtgtaattgataattctgcttctcctctatcttatcgtaaagctaaggaagtggtatctcttagacaacctttaaaaaatcaaaaagtagaggcacaacctctattgataagtaattcttctgaaaagaaagcaagtgtttatacaaattcacatgatttttgggattatcagtgggatatgaaatatgtgacaaataatggagaaagctatgcgctctaccagccctcaaagaaaatttctgttggaattattgattcaggaatcatggaagaacatcctgatttgtcaaatagtttaggaaattattttaaaaatcttgttcctaagggagggtttgataatgaagaacctgatgaaactggaaatccaagtgatattgtcgacaaaatgggacacgggacggaagtcgcaggtcagattacagcaaatggtaatattttaggagtagcaccagggattactgtaaatatatacagagtatttggtgaaaatctttcgaaatcggaatgggtagctagagcaataagaagagctgcggatgatgggaacaaggtcatcaatataagtgctggacagtatcttatgatttcaggatcgtatgatgatggaacaaatgattatcaagagtatcttaattataagtcagcaataaattatgcaacagcaaaaggaagtattgttgtcgcagctcttggtaatgatagtttaaacatacaagataaccaaacaatgataaactttcttaagcgtttcagaagtataaaggttcctggaaaagttgtagatgcaccgagtgtatttgaggatgtaatagccgtaggtggaatagatggttatggtaatatttctgattttagtaatattggagcggatgcaatttatgctcctgctggcacaacggccaattttaaaaaatatgggcaagataaatttgtcagtcagggttattatttgaaagattggctttttacaactactaatactggctggtaccaatatgtttatggcaactcatttgctactcctaaagtatctggggcactggcattagtagttgataaatatggaataaagaatcctaaccaactaaaaaggtttcttctaatgaattctccagaagttaatgggaatagagtattgaatattgttgatttattgaatgggaaaaataaagcttttagcttagatacagataaaggtcaggatgatgctattaaccataaatcgatggagaatcttaaagagtctagggatacaatgaaacaggaacaagataaagaaattcaaagaaatacaaataacaatttttctatcaaaaatgattttcataacatttcaaaagaagtaatttcagttgattataatattaatcaaaaaatggctaataatcgaaattcgagaggtgctgtttctgtacgaagtcaagaaattttacctgttactggagatggagaagattttttaccggctttaggtatagtgtgtatctcaatccttggtatattgaaaagaaagactaaaaattga

SEQ ID NO: 60 - DNA, 687 bp, Lactococcus lactis CCOS 949
gtgtataaaattttaatagttgatgatgatcaggaaattttaaaattaatgaagacagcattagaaatgagaaactatgaagttgcgacgcatcaaaacatttcacttcccttggatattactgattttcagggatttgatttgattttgttagatatcatgatgtcaaatattgaagggacagaaatttgtaaaaggattcgcagagaaatatcaactccaattatctttgttagtgcgaaagatacagaagaggatattataaacggcttaggtattggtggggatgactatattactaagccttttagccttaaacagttggttgcaaaagtggaagcaaatataaagcgagaggaacgcaataaacatgcagttcatgttttttcagagattcgtagagatttaggaccaattacattttatttagaagaaaggcgagtctgtgtcaatggtcaaacaattccactgacttgtcgtgaatacgatattcttgaattactatcacaacgaacttctaaagtttatacgagagaggatatttatgatgacgtatatgatgaatattctaatgcactttttcggtcaatctcggaatatatttatcagattaggagtaagtttgcaccatacgatattaatccgataaaaacggttcggggacttgggtatcagtggcatgggtaa

SEQ ID NO: 61 - DNA, 1345 bp, Lactococcus lactis CCOS 949
atgggtaaaaaatattcaatgcgtcgacggatatggcaagctgtcattgaaattatcataggtacttgtctacttatcctgttgttactgggcttgactttctttctacgacaaattggacaaatcagtggttcagaaactattcgtttatctttagattcagataatttaactatttctgatatcgaacgtgatatgaaacactacccatatgattatattatttttgacaatgatacaagtaaaattttgggaggacattatgtcaagtcggatgtacctagttttgtagcttcaaaacagtcttcacataatattacagaaggagaaattacttatacttattcaagcaataagcatttttcagttgttttaagacaaaacagtatgcctgaatttacaaatcatacgcttcgttcaatttcttataatcaatttacttaccttttcttttttcttggtgaaataatactcattattttttctgtctatcatctcattagagaattttctaagaattttcaagccgttcaaaagattgcattgaagatgggggaaataactacttttcctgaacaagaggaatcaaaaattattgaatttgatcaggttctgaataacttatattcgaaaagtaaggagttagctttccttattgaagcggagcgtcatgaaaaacatgatttatccttccaggttgctgcactttcacatgatgttaagacacctttaacagtattaaaaggaaatattgaactgctagagatgactgaagtaaatgaacaacaagctgattttattgagtcaatgaaaaatagtttgactgtttttgacaagtattttaacacaatgattagttatacaaaacttttgaatgatgaaaatgattacaaagcgataatctccctggaggattttttgatagatttatcagttgagttggaagagttgtcaacaacttatcaagtggattatcagctagttaaaaaaacagatttaaccactttttacggaaatacattagctttaagtcgagcacttatcaatatctttgttaatgcctgtcagtatgctaaagagggtgaaaaaatagtcagtttgagtatttatgatgatgaaaaatatctctattttgaaatctggaataatggtcatcctttttctgaacaagcaaaaaaaaatgctggaaaactatttttcacagaagatactggacgtagtgggaaacactatgggattggactatcttttgctcaaggtgtagctttaaaacatcaaggaaacttaattctcagtaatcctcaaaaaggtggggcagaagttatcctaaaaataaaaaagtaat

SEQ ID NO: 62 - DNA, 678 bp, Lactococcus lactis CCOS 949
atgcaggtaaaaattcaaaatctttctaaaacatataaagaaaagcaggtgctacaagatatcagttttgatattaaatctggaacagtctgtggtttattaggagttaacggtgcaggaaaatcaactttgatgaaaattttgtttggtttaatttctgcagatactggaaaaattttttttgatggacaagaaaagacaaataatcaacttggagccttaatcgaggctccagcaatatatatgaatttatctgctttcgataatcttaaaactaaggctttgctttttggaatttcagataagagaattcatgaaactctagaagtgattggtttggcagaaacaggaaagaaaagagcaggaaaattctctttagggatgaaacaacgtttgggaattggtatggctattcttacagaacctcaatttttaattcttgatgaacctactaatggtttggatcctgatggtattgcggagttgttaaacttaatcttaaaacttaaagctaaaggtgtgacaatcttgatttctagtcatcagttgcacgaaataagtaaagtagctagtcaaattattattttgaacaaaggtaagattcgttataatcatgcgaacaataaagaagacgacattgaacagttattctttaagattgtgcatggaggaatgtga

SEQ ID NO: 63 - DNA, 729 bp, Lactococcus lactis CCOS 949
atgaaaagaataatagcatcagaagcaataaaattaaaaaaatcaggaactcttagattggtattaattatcccttttgtgactctatttatagcatttcttatgggtggaatacagatttttagtgttttttcaatttattggtgggaaactggttttttattccttttgatgagtttgctttttctttatgatataaaatcagaggagcaagctggaaattttcaaaatgtgaaatggaaaaagctgagttggaaaattcatttggccaaaatgttgttgatttggctaagaggtatactagcgagcatagtcttgattattttgctttatttggttgcttttgtgtttcaaggtattgtagtggtggattttatgaaagtaagtgtggcattgattgctatattactagcagcttcttggaatttaccctttatatacttgattttcaagtggattaatacttacgtattgttagctgcgaataccttgatttgtttaattgttgccccttttgttgcacaaactccagtatggttcttgctaccatacacttatcactataaagttacagaaagtttgttaaatatcaaaccatcaggagatttgttaacagggaagataaatttcagtatttgggaagttttattaccatttggactttccatagttgtaacgataggagtttcgtatttacttaaaggagtgatagaacatgataagaagtga

SEQ ID NO: 64 - DNA, 645 bp, Lactococcus lactis CCOS 949
atgataagaagtgaatgtctcaaattaaaaaatagcttagggttttatttagtttttctctttactttattagagcttttaacggttcctatttatttagcttttggaagaagtcatgtttcaatgactgatttatcgctcatgatttttttgttttttccgttactggttacaattttgtctattctaatctttgaacaggagagtctggccaatcgtttccaagaaataaatgtaaataaaaaaagtagcagaatttggttatcaaagctaatagtagtggatttccttttgttctttccatcagcaatgatctggataattacgggagtttcacaggcagtagggcaacaaggaatgatgatcgcaacagctagctggttgatggcaatttttcttaatcattttcatcttttattgacctttataatcaatcgaggagggagcatgattatcgcgattattgaaatattactcattatttttgccagtaataaagttttattagcagcttattggtgtcccattgctttacctgttaattttatgataactgggcggtgtgcttatctgatagctgccgtagggtggattgttttatccacaataattcttgtagcattatctaaaaaaaagattagataa

SEQ ID NO: 65 - DNA, 1320 bp, Lactococcus lactis CCOS 949
atgccagtttctcgtattaaagttaaaaatagacatttaaaaaagaaagccaaaaaaccactggctttttataaaccagcgaccaaatttgctggcgctgttctcattgcaggaactttgacgaccactcatgagcttttgctccaacaaacaagcccaatggttcaggctgcaaccaattccacagaagcttttattgaaagtattgctgcatcagcaaaaccagttgccgatagtaatggtctttatccttcagttatgattgctcaagctattttggaaagtaactggggttcaagccaactttctcgtgccccctattataatttattcggtattcaaggaacttatcaaggaaaaagcgttgtttttaaaactcaagaatatctcaatggtaaatgggtcacaaaagatatgccatttagggtttatccttcctttaatcaaagtttccaagacaatgcttatgttttaaaaactacaaactttggaaatggtccttattatgctaaagcttggcgagcaaacgcggcaacctatcaagctgcaaccgcagccttaacaggaaaatatgcaactgaccctaattatggtgcttccctgaatcgaattatttctcaatataatttgactcgttttgacggtgcttcttctgctggtacttctaattccggtggttcaacagctacaaataccaataataattcaaatacaagctcaaccacttatacagttaaatctggcgatacactttggggaatttcgcaaaaatatggaattagtgttgctcaaattcaaagcgcaaacaatcttaaaagtacagtcatctatattgggcaaaagcttgtattgacaacttcaagttcttcgtctaatacaaatagttcaacttcttcaggaaattctgccggaactacaacgcctactacttcggtcactcctgccaaaccagcttcacagacgacgattaaggttaaatctggtgatacgctttggggactctctgtcaaatataaaacgacgattgctcaactcaagagttggaatcatttgaattctgatacaattttcattggacaaaacttgattgtttcacaatctgccggttcttcaagttcttcaacaggttcaagctcagcctctacgagttcaacttctaactcttctgcagcttcaaatacctctatccataaggttgttaaaggagatacgctttggggactttcacaaaaatctggtagcccaattgcttcaattaaggcttggaatcatttatcaagtgataccattttaattggtcaatatcttcgtattaaataa

SEQ ID NO: 66 - DNA, 1044 bp, Lactococcus lactis CCOS 949
atgaaaaaggtgattaaacggaaggttatattatttagccttccttttttattgcttttattgccaattctagctttctttgctctatttgtaggttcaagtgatttatcttcagatacagatattaataccaatacaccacagcaacaaactgccaaagtgatttgggatagagttctaaaagaaggtggaacgaaagaaggggcagctgctttacttggtaataatcaagcagaaagtgaacttcaaccttcaattattcaatctaatgcaacctataatgaagcaaaagcaatggataccactttaggcggttatgctttcggtttggctcaatgggatagtggcaggagagtaaacttgctaaactatgcgaaaagtcagaaaaaatcttggacagatactaatcttcaagttgagttcatgtttgagcaagacggtacagattcaacgttacttaaacaattaatcaaaggaactaatgttaagcaaacgactgaagatattatgcgaaagtgggaacgtgcaggggcggttgatagccttccaaaacgtcaaggttttgcggaatattggtacacgttcatgacgactggtggtgatagtggaactggtggtggttcaggaattactccagatataccttcaggttggactttagataaaccaattaatacaagtggttatcttgcgacaagttatgagtataaacaatgtacgtggtttacatggaatcgagcccaagatttcggtattacttttggaatgtatatgggaaatggtgctgattggcaacatcaagcaggatatactgtaacgactactccaacacttcatagtgcggttagctttagtggaggtcaaacagtaggcggtcaatggactgctgacccacaatacggtcacgtggcctttgtggaaggaatacattcagacggttcagtcttgatttcacagtcaggaactggttttagtacagtttatactttccaagtattaacaaaagcacaagctagtcaattacattatgtgataggaaaataa

SEQ ID NO: 67 - DNA, 894 bp, Lactococcus lactis CCOS 949
atgcagtataaaaaaaaagaaaacaaggttttggtaatttttgtactggtcgtaatttttattttgtgtggatgcatatatgtcttactagtcagatatacccatactgataaaataacgacgatcagttataagcagccaactaaaacatcggcttctaacggttatgtagagcaaaaaggtgaagaagctgctgtgggtagtataacacttgtagatgatgctggtgtaccagaatgggttaaagttccctcaaaggtaaatctagataaatttactgatttatctacgaataatatcactatttatcgaattaacaatccggaagtcttaaaaacagttaccaatcgtacagatcaacggatgaaaatgtcagaagttatagctaagtatcctaatgctttgattatgaatgcttccgcttttgatatgcagacaggacaagtagctggatttcaaattaataatgggaagttgattcaagactggagtccaggtacaacgactcaatatgcttttgttattaacaaagatggttcgtgcaaaatttatgattcaagtacacctgctttaactattattaaaaatggagggcaacaagcctatgattttggtactgcgattatccgtgatggtaaaattcaaccaagtgatggctcagtagattggaagattcatatttttattgcgaatgataaagataataatctctatgctattttgagtgatacaaatgcaggttatgataatataatgaaatcagtatcaaatttgaagctccaaaatatgttattacttgatagtggcggctcaagtcaactatctgtcaatggtaaaacgattgttgctagtcaagatgatcgagccgtaccggattatattgtgatgaaataa

SEQ ID NO: 68 - DNA, 1500 bp, Lactococcus lactis CCOS 949
ttgactaataatgataaaactaagcgcttaaaaaaggaaaaatttattgcgggaacagcgctgattttaggaatgacgacttttggcgtggctggccatgctgatggagtaactgttggaagtagttcagatgcatcatcaagcacaggtagctcaagttcatcatcaggtacagggggttcaagttcatcatcaagtacaggtagctcaagctcatcatcaaattcaaatgcttcaagttcatcgtcaagtacaggtaattcaagttcatcatcaaaaccaagtacttcaggttcgacatcaaaaccaagtaatccaagttcatcaacaaataataattcaactagtaattcctctacaacaactcaagcaccatcaacttcagtttctaccatagctccttcagcatcaacttctacagttgcaccctctaattattcacaggataatgcctactatcaaacatcaactgcagcacaaattcctaattcttcagcagattcagctccttctatttacgctggccctgttttgaaaacaattgaagcagctaagtcaattgataaaattgatacttctagtacagaagcctttattaaaagtattgcagaccgcgtgagaattttagctggtaagaataatttgtatgcatcaattatcttggcacaggcgattttagaatctggttctggtcaaagtaatatgagtcagcagtattttaatattttcaatattacaggtgcttatttaggaaaatcaatttcatttaagacggaagaattttcgggaaataatccttattatattgaacaaagttttagagtttatagtaattatgaccaagccttggatgattatattaatttaatgattaaagggacaacttggaactcagaaatttatgctggcgcatggaagtcacatgctaagacttaccaagaggcggctcaagcattgcaaggaatttttgctactgacccagcatatgcacaaaaattaattgaaattattcaagaatataaattagatgcttatgataatgttgatagtacaacacaagttgtagatagtaaaattcctgaaagtccattggcggcatcaaaattagataattcagcttatccagaatataatggggtagaatatccaggtgctgatagttatgcttttggtaattgtacacagtatgtttataaccgtatcattcaattaggtgggctcgttggaacacatatgggaaatggtggagaatggggaattaatgcccaagctcaaggttatttcacaacaactgttccaactgagggttatgctgttagcttcccaccaggagtagctggttcaagttcagaatatggtcacgtagcttttgttgaaaaggtttattcagataactctattctcgtttcagagatgaatgttaaaggtaataatattgtcagcgaacgccatatttctgctggtgtagctgctttggcaacttatattcaacctaaataa

SEQ ID NO: 69 - DNA, 780 bp, Lactococcus lactis CCOS 949
atgtcaagtattgaaaatatgattgcttggatgcaagcacgaaagggtaaggtaacttactcaatgaccttgcgaatgggtcctagaagttatgactgcagctcgtcagtattctttgcaatgattgctggaggttttctgtcagaaggttcaatgggtaatactgaaaccttgtttggaatgtcaggaacgaagctgaaagaaatcagtcgtggagaggtccatcgtggcgatatcttcatctcaggcactccaggaggttcggctggttcagatgggcatactggtattttcctaagcaatggctcattcattcactgctcttatactcacaatggaattgcggttgatacgaatgatgcatacatgagtactcgcttgccacatcacttttatcggattgttggttcaggttcagcaaatactgacagcaagcctcaaatggttacattaaatgttgatggacagtttggaaatgcgactgctaaacgattgcaagaatactttgatacagctggtaaagatggagtaatcagtcaccagtacaaacaaacctttaatcaaaatatctatgctgcgcagtttgattcatcactgactggttcaaacgtggttaaagcattgcaaagattcttaggcattggccaagacggcttgtttggccaaggtacaattaaagcactacaaaaacatcttggaacgacgcaagacggaactatcagcccagtttctgattctgttagagaattgcaacggcgattgaatgcgaataaattataa

SEQ ID NO: 70 - DNA, 816 bp, Lactococcus lactis CCOS 949
atgaaacctaaaatgagacgtaaacttaaaaaaatgggagcttttatctttacagcatccatgattgcaatgatcgccttacttggtttagtacgaattcgaccggtagaacctcctaaaaaagcagcaactgaaaaaattgttgtaaatcatattttggatgagaaggttttggatttgaataaaccagttgttgacctttcgggttggcaacgtccagaagatattgattacaacaccttaagtcagcatgtgattggtgcggttattcgtgtcaatggttcttatggtcatgctgataattcagcaagcaaggatggagaagatactgcctataaacagcacattaaagctttccaagagcggggaatcccgactgcggtttatgcttttgtgactggagaaaacacttctgaaatgaggaagcaagcaagagacttttatcgtcgagcaagcccttataagccgacctattattggcttgatgtcgaggtaaccaatatgaaaaatatgaaccaagggattgaggcttttcgctctgagttggagaaacaaggagctaaaaacattggtatttatgcccaagactggttcttgcgagataatcaaataaaagttgataaatttaaagcgatttggattgctgcctatggacgaaatacaggttattgggatgcttcaccagaaacgactttaagttataaaatgcaacaatttactgaccaaggaactttaccaggttactcgggaaatgttgatttgaatatggttaataaccaaaccaactataatgaattgtttaaaaatcaaaaataa

SEQ ID NO: 71 - DNA, 2613 bp, Lactococcus lactis CCOS 949
atggataaaagaagcaaagaaaactttaaagcttcgctcaatgtccagaaacgtgtctctgatggaattgatgcgaatgcctttagaaaacctcgacaagccacgcaattaagtaaacaggcgtttaaagaagggaaaaaaacactcaaaattcgccgaaaaaactatcgaaaattaaaagctggttcaggtttacaagttgtcgcagccaaaaagaaagttcttgaagcaaaagcagataaaaccgtttctaaagcggtttttaaaaatgcaaagaaatctgatccaacacgagcagctaatcaagcgaaaggctatgccaagaatcaagccaagcaaacagcagtcaaccacttagtgttatcgcctcttgaaaaagatgatactttaagagaaggttcagacctctatagaaagactcaacgtaccaaaagtgggttaaaactttctaaggatgttgtcacttcttccgctaaagcttcggttaatctttcaaaccatacttacggtttagccaatcgaagtgttaatattgttcgaggccgtgggtttgtcagaactccttctgaattggggttcagaaggcaagccgcaaaaagaatgcggaactttcaaaataagctgagtgccgcaagaaaggcaaaaaaggcggagcaaggattttctttgattcggtcaatcttaaaaggccaacaaaccctgagtcgtgcgtttactttaatcgtgacctccaaagggttactcgtcgttcttgctgttatgtttatattgtgtctcttgggaatccttaacatggcctcctctgttccaacaaagcaagatgactttcaactgacaaagtcttggacatatttcacaaaacttgatgcagacaattcagagaacggaaactctttttatacgcctttggatgatgtgatgttttatatgaatgatcaatttgaagattataatttacaagatcaagtgcctgtaggttcaaatggcgcagcacttcctaatcaaaattatgaacaatatcttacaggcctttggtcagccttaaatggctcttctcctgattataagctaacaacaatggaggctttggagacggataagcgttctaaatattatctttctcctgatgattattcagattttaaagaacgtgttaatgaagtcggttatgatagccttgatggtcaacttcagtttccttatcaaacagagagtttggttatcaatcgtagatatggctacgaacggaatggagataaaactgaactccacgcaagcattgatgttagttcagccccagggcaagatttaacttcaccaatgcacggaattgttaattctgtgactgaccctaatacattggtcatttctgaagctgaaaatgcacggttgacaattgttgggattaatagcggacggtttattggtggtgaaacagtagatgctggaacacttcttggcaaggccacaaagtcaagtcttaatatgacctatgaaaaatataatgaagatgataaaaaatgggaaaaagttaatccagcattttattttcctaaagtgacctatactcagtttacctctttagcttcagatagctttgatccaggaaaaagtgtttctgaacgtgcggaggccgtttataatttcttaaccaaacttggctataaaaaagaaggaatttgcgctatcttaggttcttttactgaagaatctcaaatcaatcctaagcgagctgaaggagattatttatctccaccagttggtgcttctggtaattcttgggatgatccggcttggttagctatgggtgggttggatatttacggaaaatatccaaatattcttcatagagggttggggttaggtcaatggacagatacatctgatggttctgaaagacacactttacttttaaattatgccaaagcaaaaaataaaaaatggtacgacttagaccttcagcttgattttatgctcaatggagatactccagggaatcaaaccatgtttaaaaataccgctagtaatgccgtctcttcttcaattccagaactgaccaactacttcttgacttactgggaaggaaatccaggtgacaagattcaggcacgtgtacaagccgcccaaaattggttcacttacttctcaaataacggtggctccgatgcggatatgagcgcttcatcaaaagaactctttgagaaatataaagacaaaattaaacctctcccttctaataaagaaacacaacaagggcaaggatggcctgggaatggctatgaacctgggaattgtacttggtatgtctttaatcgtcaagctcaaattggtcataatattaatggctatatgggtaatggtggccaatggggttataactatactaaaactccaggagctacaattgattctaaaccacaagtgggagatgcggtaagtttctctccaggtgttgcagggtctagttcagaatatgggcacgtggctcaagttgaagttgtcaatccagatggtacatttttagtttctgaaatgaacactttaggcctttattcaatgggctatcgaatgtttaaaccaggagcaggaatgacatttgttcattttaaataa

SEQ ID NO: 72 - DNA, 978 bp, Lactococcus lactis CCOS 949
atggaaaaaggattattagtcgatattggacgaaaatattggtcaatagcagagttaaaaagattagttcttttacttcaagagcataagctgacacatttacaacttcatctcaatgaaaatgaaggatttgcgctaaattttactgacagccctgtcagtaaaaaatattcagaaaatatgctcaaagaattgaaagaatttgcaaaaacacacgaaatcactttgattcctgattttgatagtccaggtcacatgggctccttattagagcaaaatcctgaatttgcactacctgacagcaatcaacaagcggtagatgttactaatccagcagtcattgattggattatgggaataattgataagatagtcgatattttcccagattcagatacttttcatatcggggctgatgaatttattgattttcggcaaattgaaaaatatccttatttagtggagaaaactcgggaaaaatatggaaataaggcaagtggtttagagttttattatgactatgttaatcaattgaccgagcatttgcagaaaaaaggaaaacaagttcgtatttggaatgatggatttttacgaaaagaccttcagtcattggttcctttgaataaaaatgtggaggtttgttattggacaaactgggacaaagggatggcagaagtcaaagaatggttaactaagggttataccttaataaatttttgtgataatgacctttattatgttttaggtgaagaagcaggctattcttatccaacggctgaaaaactggaaagggaaggaaaaattcaaaaattttctggtcagcaatatttaaatcaagaagagatgaaagctgtcagaggaacttacttttcgatttgggctgacaatgctgcagctaagtctgtcagtgaaattttagacgatcttagcaaggtacttccggtatttatgaaaatttatggaggaaatgatgaataa

SEQ ID NO: 73 - DNA, 1641 bp, Lactococcus lactis CCOS 949
atgaaaaaatcgaaaaaattttttattagaatatgcctttctacaggaattttggcatctgcaactttactgacagcttgttttggaactccagcaaaacatgtgaaagctaattataaagtgacagcagaagcaattccagattaccaaagtaagaatgctcccatttcatcttattggatgcctgataaatttctagaatggtcagcggaaaatgacaaagatttagtttacaatcaatcccgagtgccacttaccaaaagaatttctcctgataaactaagtccatccaatcaaaatcagaacaaaaagacaaaaattgtcgccttgtcgatgatgaactcacaaacttctggaaatccttcgcggggcacgacaaaatttgagagctatacttttgattattggcaatatattgacacactggtttattggggtggctcatctggtgaaggaataattgtaactccgtcagcagatgttattgatgaagcacacagcaatggtgttccggtacttggaacaattttcttgccgcctaaagaatacggtggaaaagtagattgggtcaaaacaatgctcaaaaaagatgagcaaggacaatatccatttgccagtcaaatggttaaggttgccaagacttatggatttgagggttggtttatcaatgaagaaacccaagggctaaatgctgacgatgcagctaacatgaaagccttgattcaacaggtgaaaaaagaagattctagtcttcaaatcatgtggtatgatgccatgactaaagatggaaaagtggattggcaaaatcagttaaatgaccaaaatgcgacatttgtacaagataaagcagcagacgcgatgtttttaaatttctggtggactcaaaataatttggccgaccaaaaattacttgaaaaatcgaatctctatgctaaaaatcacaatattgacccttataatatttatgccggaatagatgtgcaagcgaaagacgtccaaactccagttaaatggaaccttttagaaaaaggaaatcaagccactcaaacatcaattggactctatgcagcaagcgctacctacactaacgcaagtaattgggatgattttcaaaatcgtgaatcagcattctgggtcaatcaaaaagcagaccctcgtcaagttgatcactctgttaatgaatcatggacaggactttccaaatatgttctggaaaaatcagcaataagcggtaatgaatttaatactaattttaatttaggaaatggttataactattttaaagctggtcaaaaaatctcagaaatggattggaacgaccgcagtttagcaggtattttaccatcttaccgctggattattgacaacgaaggaaaaaataaaataagtccaagcttcgactttgcaaatgcttataacggtggaaattcactgaaatttatggctgaacatttagatgcaggcaaaagctcaaacatcacattgtttgctagtgatttgaaaattgctatgggagcaaaattctctgttagtatgcgctcagaccaagcgcttaaagtttctgcaatcttagaactagcaaatggtcaaaaagttagcattgcaggagataaaagcctgactgagaattggtcaaaataa

SEQ ID NO: 74 - DNA, 630 bp, Lactococcus lactis CCOS 949
atgaaatataaaactcgacgaagaaaaccaaatcgacgtcaatccttgttaaaacagctcatctttattttcctagttattttaggaatcttagtctataataaaatttttaataaccaagcacaaaagccgtctgaagcacaacttcaagaaattaatgaacataaattcatcaaagaaattgctccactcgctcaaaaatcacaaaaagaaagtcaagtactagcttctatcaccattgctcaggcctgtcttgagtctaattttggcaaaagcgaacttgcaagtaaatatcataacctttttggtgtcaaagcatctgatgatgtgccaaaggtttcgcttgctacgcaagaatatgaaaatggtcagtgggtcactgtccaaggtgttttccgtgtttatccaaattttgctgattcagtttcggcacacacccagcttttcctttacggaacaacatggaattctaaacaatatgcttcagttcttagtgcaactgattataaaactgctgctaaagccgttcaaaattctggctatgcaacagaccccacttatgctgacaaacttatcaatatgattgaaacttatcatttaaatcaatatgataaaagttcaagtatttaa

SEQ ID NO: 75 - DNA, 780 bp, Lactococcus lactis CCOS 949
atgtcaagtattgaaaatatgattgcttggatgcaagcacgaaagggtaaggtaacttactcaatgaccttgcgaatgggtcctagaagttatgactgcagctcgtcagtattctttgcaatgattgctggaggttttctgtcagaaggttcaatgggtaatactgaaaccttgtttggaatgtcaggaacgaagctgaaagaaatcagtcgtggagaggtccagcgtggcgatatcttcatctcaggcactccaggaggttcagctggttcggacggacacacgggtattttcttaagtaacggttcattcattcactgttcttacactcacaatggaattgcggttgatacgaatgatgcatatatgagtactcgcttaccacatcacttttatcgaattgttggttcaggttctggaaatactgacaataaacctcaaatggttacattaaatgttgatggccagtttggtaatgcgactgctaaacgattacaagaatactttgatacggctggtaaagacggagtaatcagtcaccagtacaaacaaacctttaatcaaaatatttatgctgcacagtttgattcatcactgacaggctcaaaagtggtcaaagcattgcaaagattcttaggcattggccaagacggcttgtttgggcaagctacgattaaagccttacagaaacaccttggaacaacgcaagacggaactatcagcccagtttctgattctgttagagaattacaaagacgattgaatgcgaataaattataa

SEQ ID NO: 76 - DNA, 780 bp, Lactococcus lactis CCOS 949
atgtcaagtattgaaaatatgattgcttggatgcaagcacgaaaaggtaaagttacctattcaatgacttcacgaatgggtccaaaaagttatgattgtagttcatcagttttctttgcaatgattgctggaggttttctgtcagaaggttcaatgggtaatactgaaaccttgtttggaatgtcaggaacaaagctgaaagaaatcagtcgaggagaagtccagcgtggcgatatcttcatttcaggtactccaggaggttcagctggttcggacggacacacgggtattttcttaagtaacggttcattcattcactgttcttacactcacaatggaattgcggttgatacgaatgatgcatatatgagtactcgcttaccacaccacttttatcgaatcgttggttctggttcaggaaagactgacagtaaacctcaaatgattacattgaatgttgacggtcaatttggtaatgcgacagctaaacgattgcaagaatactttgatacggctggtaaagacggagtaatcagtcaccagtataaacaaacctttaaccaaaatatttatgctgcacagtttgattcatcactgacaggctcaaacgtggtaaaagcattgcaaagattcctaggaattggccaagacggattatttggtcaaggaactatcaaagctttacagaagcatcttggaacaacgcaagacggaactatcagcccagtatctgattctgtgagagaattacaacggagattaaatgcgaataaattataa

SEQ ID NO: 77 - DNA, 1212 bp, Lactococcus lactis CCOS 949
atgactaagcgcttaaagaaaaaagcaaaaccagttgtttttctagctcttgttcttggttgtgcattaattttatcaggagttcttggtttggcgggacatttaaacgaacaagaatcgtctaaaacaaaaaagaaaagtcaattgtcagaaactaaaaggagttcaacttccccaaaaaatatggataaaaatattgagcagatgactttggaacaaaaagttggtcagttatttatgacaggaatgccagcaaataactataatcaggcaacttttgatgcgattgaaaagtatcaagtaggtagtattattttgactggtcgctctaatctcagtgtcccagaaatgaaagatattactgacaaactacaaggcttagaaccggctaatcgcaaactcttgatatcctgtgaccaagagggaggaaatgttcaagttctccaaggtcagggtttttcacagattcctgatggattaactcaaggaagttggacagctgataaattacaaaaggaatcacaaacttggggaagtgaactttacgcagctggagtgaattttgacttagcaccagttgctgaccaagttttatctgccgactttgctccacaaaatgctccaattggctattggagtcgccaatatgcttatgataaagcaagtatcataagccatgctcaagcatttacggaaggcatgaaagcagccaaggttttgacaactgctaaacattttccagggcttggagcggtgacaggcaatacagatatcagtgcaggtgttagagatgaccaaacgaattccaatagcgaatctgttcaaattttcaaagatttaatctcttctgggacaccttcgattatgaccgcaaccgctatttatgataaaattgaccctaatcttcccggtgctttttcatccaaaatggttgatggtttactacggaaacaattaggctttgatggtttggttattacagatgatttatcaaatgctgtccaagtacaatcatggacgcctggtcaaagggcagttttagcattgtcagcaggaaatgaccttgttttagcaaatgagcctacacaaattccagaaatgatctcagaagttttgcaaaaggtaaaagcagacccagactttgctaaaaaaatcagtcaatcagccacaagagtgattaaagtaaaagaagaaatgaaacttgtagaatag

SEQ ID NO: 78 - DNA, 939 bp, Lactococcus lactis CCOS 949
atgattgcccaagggattttagaatcaagtggtggacaaagtgccttagcaagcaattataataatatttttggagttaaatacacttctggtacacctgtttatctaccaacacaagagtatttgaatggaacaatgacaaatgttgttgaacccttccaagcttatagctcagtttatgacgcatgtgttgcccaagctaaaatgttacgtgcttcatcatattattctggggcttggcgtgaaaatacaagttcttacttagatgcgacagcttggcttgaaggacgttatgccacggatccaacttatgcttctaaattgaatagcgtgatttctgaacttggtttaagtgtttatgaccaaggaggagaaatatcaggaggaactgctgttacaactagttcatcagcctcaacaaattcagctggcacatacaaagtacaagagggtgattcattatcagcaatcgctgctcaatatggtacaactgttgatgcacttgtgtcagcaaatagtttagaaaatgcgaacgatattcatgtaggagaagttttgcaagttgctggtgctagcacaactacaacaagtaccaatacaacttccaatgtatcgtcaagttctacttataccgtcaaatcaggagatagtttatattcgattgcggaacaatatggaatgactgtttcatcactgatgtcagccaatggaatttatgatgttaattcaatgcttcaagtaggacaagtattgcaagtaactgtaagtactagtgcaacaacttcaaacacaacgacttcaaacagttatacaattcaaaatggtgacagcatttattcaattgccacagcaaatggtatgacagctgaccaattagcagccctcaatggatttggaattaatgacatgattcatccaggacaaacaattagaatctaa

SEQ ID NO: 79 - DNA, 1041 bp, Lactococcus lactis CCOS 949
atggaaaaagcaattaagcggaaggttatattagttagccttccttttttgttgcttttattgccaatattagctttcttttcattatttgttggttcaaattcttcttcagatacagatattaatactaatacaccacagcaacaaactgccaaagtgatttgggatagagttctaaaagaaggtggaacgaaagaaggggcggctgctttacttggtaataatcaagcagaaagtgaacttcaaccttcaattattcaatctaatgcaacttataatgaagcaaaagcaatggataccactttaggcggttatgctttcggcttggctcaatgggatagtggcaggcgagtaaacttgctaaactatgcgaaaagtcagaaaaaatcttggacagatactaatcttcaagttgagttcatgtttgagcaagacggtacagattcaacgttacttaaacaattagtcaaaggaactaatgttaagcaaacgactgaagatattatgcgaaagtgggaacgtgcaggggcggttgatagccttccaaaacgtcaaggttttgcggaatattggtacacgttcatgacgactggtggtgatagtggaactggtggtggttcaggaattactccagatataccttctggttggactttagataaaccaattaatacaagtggttatcttgcgacaagttatgagtataaacaatgtacatggttcacatggaatcgagccaaagatttcggtatcacttttggaatgtatatgggaaatggtgctgattggcaacatcaagcaggatatactgtaacgacaactccgacactccatagtgcggttagctttagcggtggtcaaacagtaggcggtcaatggaacgcagaccctgtttacggtcacgtggcttttgtggaaggaatacactctgacggttcagtcttaatttcacagtcaggaactggttttagtgcggtttatactttccaagtgctgacaaaagcacaagccagtcaattacattacgtgataggaaaataa

SEQ ID NO: 80 - DNA, 2154 bp, Lactococcus lactis CCOS 949
atgaagataaacaaaattgatacccgtcatggtactgctaatcaatccactttttcacatgggaattgccttccttacactggttttccttggggaatgaattatttttccccttcaaccggtgctgctcgtggagcttggtggtttcatccagaagaccgtacctttgaaggctaccgaatcactcaccaacccagtccttggatgggagatttctcacatttgacaatgacgcctgttgcaggtcctttgcctgaaacttccttgtggcacacagtgagttcataccgtccagaagaatcaacttttaatccaacgcaactcaaaattactcaattacgttatcagattacatctcagttaattccatcaatgtatggtggaattctatcaatgaattatcaaaatttaagccttaaagataatggcttgatgcttcatctccccggttcttatgaacttcaacaacttgacgattacagcttagagctttcaattattaattttgcgggttgtgaagatgaaaattttactttctatctcaaatttactgctgaccaaccttttgttttaagtggaaatttatctgatgaagattcttctgttcgcttagatttcaaagcagccaagcaggttcaaatacattttgctacctcttttatttccaaggaacaagccgctcttaatctggagcgtgaacaagataattcagcagaaacatatttggaaaatgctgaatcagcttggaataaccttttttcacgtatcgaaattgagcatcataatcaacaagaagtttccactttctatcacaatctttatcgctcatttctctttccacaaactttttatgaatttgaccaagagcatcaaaaaatccattacgatacaagctctaaaactgtcaagaaaggcccgctctatacaaacaatggcttctgggatactttccgaacagtctatccgctttatagtctaatagccgttgacgagtacggtgatatgctcgaaggtttcctaaattcttatcgtgcgactggttttcttccaaaatggctttctcctgatgaacgtggtctaatgcccggtaccttgatagacgctgtcattgctgatgctgcaagcaaaaacattcgtcctgatttgatgcccgagtttttggaagcaatgaaaaaaggagccacaagtcaatctgaaaactctaattacggccgtcgtggcacaaaagattatctaaaacttggttatgttccgctcactcaccatgaatcagttaatcacactttagattacgcattttctgattattgtatttctcaagtggcgaaacaaaccggtgacaaagaaatttcagacttctatgcccatcaagcaaaagactatcaaaatatttttgattctgaaactggttttatgcgagcaaaagatgctgacggaaatttcagagctgactttttagatattcgttggggtcgtgattatgcagaaggttctgcttggcagacttcttggtcagttcttcatgattttgctggattgattaaactacatggctcaagagaaaattttgaaaacaaactcatcgagctttgcaaccaacgaccaaatttcaatgttgaaggatatggttttgaaattcacgaaatgagtgaaatggctgctatcgaatttggacaagtggctatctcaaatcaaccaagtttccattacccatacctttttagctacattggtaaaccttggatggctacgcctttaatcaaaaatttactgacagaaacatttaatgatagtccgaagggctatcctggtgacgaagataatggaacaatggcagcttggtatattttttcaagtttaggattctatccagtcacagctgcttctaatcaatatgtattaggaattccactctgggacaaagctagaatcaacctttcctctggtcagcaacttactattcttgcagaaccaaatgctccgcaacaagttttcgtcaaccaaatcacatttactgacaaaaaagtcaatgatacttttatcaagcacgaagaattgataaaaggcggaaccctaaaatttgatttaggaatcgtaccaaatccacttaaatatacgaacgaacaacttccttattcactgacagaaaattaa

SEQ ID NO: 81 - DNA, 1155 bp, Lactococcus lactis CCOS 949
ttggtcaaaataagttttgatgttaagaaatttgaaggtcaaacaatcaaaaaaatcggtttaagcataaaatctgatcaagcaatggattttaaagccattaatctaggagaaatgactttgaccaatggtcaaaaagtcgctccaatcgcactttcggatgcaaaagtaactgatgaagcttttgaagaagaaggaacagtaggcggttttagactttcttggaaatcagatgcaaataaaaataatttttctacttatgaaatctatcagttgaatgatgatggaagtaaagaatttttaggagcaagcaatatcaatgccttctttgttaatgccttaaaacgcggcaaaaatatcaattcaacaaaatttgaaattgtcccaattaataaggctggagaatctggacattcagttacgacctctgtgaaatggccagataattcattagctaaagcggcatttgtagcagataaaaccctagttacaattggtgaaaaagtaactttaatgaatcaatctaatctagcttccgtcaaatataaatgggatattgatggtgcaagtcccgctacttctacagaaaagaatcctcaagtaagttttgataaagcagggagttattccgtcaaattaacggtcatcaatgaaaaaggacaagaagattcagtcactcaaactgaactgattactgtaattgatcaaccagtagaattaacaaattttgcattaaatcaatccgttcaagtagacagtttcactaatgaatctgaatcaggaccaaaagcagttgatggaaaattaaataccaaatggtgtgccgttggcccaggtaaacacaatattacaattgacattggaaaatcagaaaaaatcaatcaagtcctgattgaccatgcgcaaaaaggaggagaatcgcctgacatgaatacttctgattacaccattgagatttcaaaggataatcaaaattggacagaagttgtcaacgttaagaaaaataaattgggagaaaccaaagattctttcaaacagacagaagcgcgttacgttagaatcacagccactaaaccaacacaaggagcagataccgctgttcgtttatatgaaatacaagtattaggacaaaaaaaagctgacaaagggctgtaa

SEQ ID NO: 82 - protein, 57 aa, Lactococcus lactis CCOS 949
MSTKDFNLDLVSVSKKDSGASPRITSISLCTPGCKTGALMGCNMKTATCHCSIHVSK

SEQ ID NO: 83 - DNA, 1191 bp, Lactococcus lactis CCOS 949
tagtacttgtacactcccccagtcatcggtctttaccttaggaagcgccctccttgcggttaggcaacctacttcgggtactcccaactcccgtggtgtgacgggcggtgtgtacaaggcccgggaacgtattcaccgcggcgtgctgatccgcgattactagcgattccgacttcatgtaggcgagttgcagcctacaatccgaactgagaatggttttaagagattagctaaacatcactgtctcgcgactcgttgtaccatccattgtagcacgtgtgtagcccaggtcataaggggcatgatgatttgacgtcatccccaccttcctccggtttatcaccggcagtctcgttagagtgcccaacttaatgatggcaactaacaataggggttgcgctcgttgcgggacttaacccaacatctcacgacacgagctgacgacaaccatgcaccacctgtatcccgtgtcccgaaggaacttcctatctctaggaatagcacgagtatgtcaagacctggtaaggttcttcgcgttgcttcgaattaaaccacatgctccaccgcttgtgcgggcccccgtcaattcctttgagtttcaaccttgcggtcgtactccccaggcggagtgcttattgcgttagctgcgatacagagaacttatagctccctacatctagcactcatcgtttacggcgtggactaccagggtatctaatcctgtttgctccccacgctttcgagcctcagtgtcagttacaggccagagagccgctttcgccaccggtgttcctccatatatctacgcatttcaccgctacacatggaattccactctcctctcctgcactcaagtctaccagtttccaatgcatacaatggttgagccactgccttttacaccagacttaataaaccacctgcgctcgctttacgcccaataaatccggacaacgctcgggacctacgtattaccgcggctgctggcacgtagttagccgtccctttctgggtagttaccgtcacttgatgagctttccactctcaccaacgttcttctctaccaacagagttttacgatccgaaaaccttcttcactcacgcggcgttgctcggtcagactttcgtccattgccgaagattccctactgctgcctcccgtaagaatttgggccgtgtctcagtcccaat

SEQ ID NO: 84 - DNA, 1710 bp, Lactobacillus jensenii CCOS 962
atgactaaacaaactttgcaagctgaagctaatggtcgtaatggtaagattaagtttgatattaatattgataataacgaaataaaagatataaaggttaccaaatctagtgaaacaccagcaatatttaatcaggtttttgataaattaaaaaattccattatagaggagcaatcatttgatgtagacgctgtatcgggcgctacaattatgacaagtgctttacttgattctggaaaaaaggctttgaatcaggcaggagttacaccagtagctaaagagagcgataaaacacatcgggaagtaaacctagatgtagatgttgccgtcattggctcaggtgccgcaggattgattgcagcttgccgagctctttcaatgggaaaaaatgtagtagttcttgaaaagaatggttatttaggtggagctacaatattaaatggttcaaatgtagtagctacaggttctaacttggctcagcaattatttggtactgaggcacaagaagatagtagtaaacggctttttgctgatattactcgtgaatgccgaggtacaaattatcctgaattatcaaaagttttggttgaaaatattggtaaagctgttgattttattaaagagtttgcgggtttgacttatcaaaaagcagaaacacaaacaattgagcattcagttaatcggcaagtggaaatgccaagtgaaagctcatatgaattaattaaaaagatagcagctgcctttgaagaaaagggtggcaagattttacttgatgctcgtgttgaaaaaatcaattctgaaaatggtgtacctattagtctagttgctgaaggaaagcaccaaactacaaacgttaagttcaaatcacttattttagctgccggtggttggggtgccaaagactttaaagaaaagcgaacttcgattccttattatggtccaatgacttcaactggagattatttcttctttaacaagggattaaatttggctagtcgtaatttagattggtataaagtttatccacatgggttagaagttgaacctggaattgctaaacttacaacttattcaacaaaagaagcaagtgatatgggggcaatttttattaatcgggctggtaatagaattgtaaatgaatcagatccatacactcattttagagatgcaattgctgctcaaaaagatcagatagcttttgttcttatggatcaaagaatttggaacagattttatgaattaatgcttaaatatggttttactgctgatgaaattagtcattattttgcacttgatggcaaacaaagcccaattttagtaaaaggcactcttgaaaccgtagctaataaagctggtattaattttgaaaatttacagcatactttatctaattatcaaaattatgccaaaaatggcaaagatcctgagttcggacgtgaagcaaaatttatgcatgaatattcaggtgatacttactacgttattgaacaaaaacttcgcttctgtacaactttaggtgggtatgaaactaatagccaaatgcaattattaaataatgatatgaagccagtggctaattattatgcagctggtgaagtaattggtggtgccaatggtcatgactctatgccaagtatgatgaattcatggagttatgcttcaggctttttagctggaactaatgccagcgacaattgtaataatcgataa

SEQ ID NO: 85 - DNA, 2154 bp, Lactobacillus jensenii CCOS 962
atgaaaactaaaaaaatcactggcgttgctaccgcagctttactagcctccgttgctgtgccagttaccaacaatttagctaatattcagacttcctatactgctaaagcagtcactggtcaacagcaagcatttttaaatacagctatacctaatgctgaagcagcttctgctaggtatggaacgtatacttccgtcatgcttgcacaatcaatacttgaatctggttggggcgcttcacttctcgccacacaggctaataacctatttggtatgaaaggttcatataatggacaaacttattatactaatacttcagaatgggcctctggaacaggttattacaatataaatgctggttttagaaaatatccttcttgggcagcatcttttgaagataatggttacaaattaagaacaggtactaccgataatccaagtcgttatagaatggcttggattgaaaatgctgcaaactatcaagtggctacacagggcttgaaagatgggggttatgctacttcaccaacttatcctcaatcgttaaatagagtaatttcttcttacggtcttaatcaatacgatccgtctgtagataccacaactaaaacaatgagagttttatcaaatggaacagtttattccggtccagccgattctagtgtagttagtgcaactggtaatattactgctggtcaagtggttactgttgataaaacagttacttataaaaatggactaagttatatgcatattagcaatggttggattaatggttcattgttaaccggaagttcaactcaagctaccacaacagaaaaagcaggaacaacaaccgatgcaggtaatgcagcaattaaggtagtatacacgagtgcaattgcagaatggaaaaatccaggtagtggagtagtaggctacttacaaaagggaacgacccaaacagtagttggaaaaatccaagtaaatggagcatggtggtataagctatcatcaggtaattgggtaccaggggaatatgtatatgtcacaggtgcatcaagaataccaacaattgataacaatgtagtaaatcaaaatacaaaagtaaaaataaaatatatatcaggctatagcatagcagtatggtcaaatccagcaataggaacaacaggccaatatttaaaagacggaacagaagtacaaacgattggatatactacagctaatggcaagaaatggtataaattagcgaataatacgtggataccagcagaatatactgaagtagtaagttcatcaacagtggtaacgaatattactaatgaaagtaatacagtagcgataaattatccgcactacagtatagctgtatggagtgaaccaggtagaaactcaacaggaaagtacttatcagatgggacaaaagtccaaacagtaggttataccacagtaaatggtaagaaatggtataagctagcagataatacgtggataccggcagagtatactaaagtagtaagttcatcaacagtagtaacgaatattactaatgaaagtaatacagtagcgataaattatccgcactacagcatagctgtatggggtgaaccaggtaaaaactcaacaggaaagtacttatcagatggaacaaaagtccaaacagtaggttataccacagtaaatggcaagaaatggtataagctagcagataatacgtggataccagcagaatatacgaaagcagtaagttcaacggatactactagcggaaataatacagtaacagtaaattatccaggctatagcatagtagtatggagtgaaccaggcagaaactcaacaggaaagtacatatcggatggaacaagtgtaaaatattacgcaaccgcaaattataatggtcaaacatggtataagataggtgaaaaccaatgggtaccaggtcaatatgtaaaagtaaatgcatcaaataatagtggaagcgtgacagtaaaatacatatccggatatggtatagcaatatggtcaaatccaggcagaaattcaacaggaaagtatctggagaatggcacaacagtaaaatattttgagacccaaaattacaatggccaaacatggtataaaataggtgaaaaccaatgggtaccagcacaatatgttagtgtaaattaa

SEQ ID NO: 86 - DNA, 2328 bp, Lactobacillus jensenii CCOS 962
atggcagagaataatcatcgttcagcaagtaatactgcacctaagaattctcgaatggccaacttgcatcatgatagtggtcaacccaagagacgcctctggctacaaattcttaagtggttttcaattggtattttgctgatactcgtttctggcgtcggtttatttgcttattacgccaaagacgctccatcaattagtcaagatcaactacaaagtggtggttcaagtagtttctatactagtgatggtaaattccttctttcattaggttcagaaaaaagaacttatgttaagaattctgatattcctcaaactttgaaagatgcagtagtatctgtagaagataaaagattttatcaagaaaatttagggattgacccaatcagaattgttggttcaatcgtctcaaatgccaagtcaagtggtattgcagctggtggttcaagtatcacccagcaattagttaagttaactgttttctctaccgctgcttcgcaaagaactctaaagagaaaggctcaagaagcttggctggcaattagagttgagcatgactacaccaaaaatcaaattttggaatactacattaataaggtttacatgaactatggtgtatatggcatgggaacagctgccgattactactacggcaagtcactaaaagatcttgacttagcacaaacggcattaattgctgggatgcctaatgccccagttgcttatgatccttatacttacccaaaggcagctaaatatcgtcgtgatattgttttaaatgcaatgtatgctaatggtaagatcagtaaggctcaattaaaggcagccaaggctgaatcaattacacaaggccttaaaacccaacaaaatagttcagaatcttcaattagaaggattgatgatccttatattaaggaagcaatttcagaagttaaatccaagggttatgatccttataatgataacttaaagattactttgaacatcgatcaagatgctcaaaacaaactttatgaacttgcaaatggttcaagtattccattttcatcaagtaaaatgcaagttggtgcaaccatcattaatccaagcaacggtcacgttgtagcaataattggtggacgtaatttaccatctgttcaattgggacttgaccgggcagtacaaactggccgctcaactggttcatctattaaaccagttttagattatgcacccgcaattgaatatttgaactggtcaacagcacactaccttgaagatactaaatatgtataccctggtacaagcatccagctttatgactgggataacaaatatatgggtaaaatgacgatgcgctatgcccttgaacaatcaagaaatgttccagctgttaaaaccttagctaaagtaggtatgaagaaagcttcactatttgctaaaaagatgaacatttcagttggttcaaatcaaggtctttcagtagccatcggtgcaaatgcttcttcccttcaaatggctggtgcatatgccgcctttgcaaatgaaggtgtttactacaagccacaatttgtatctcaaattgaaacagctgacggtgtggttcactcctactcagcaactggaacacgagttatgaagaaatcaactgcctacatgattactgatatgcttaaaggtgttctaactgaaggttctggtactaatgcgagaactggtctttatgaagctggtaaaactggtactgttaaatattctgatgatgaattagtaaaatatccttcatacgcaaacactccaaaagatgcatggttcgttggttatactaagaaatattcaattgggatttggaccggttatgacaatttaagcgatggtacaattagtggtcaaggccaatatgcttcccaatatctttataagtatatgatgaagtacttaatgagtgataaggaaaacagcaattggactaagccaagcaatgttgttagaaaacgaattgttaaaggttctgacccacttgaagttacttcctcaaagaaaaattcaacctctgagttgttcctacgtggtcacacaccagatggctcaaacgaggattctgatgaaagttcttcatcatcaaattcttcaagttcttctaaagataacgaagtagtaactaataagagcagcagttcttcaagttcttcatctagtgaaggacatgaagatggctcaacttctaactcaagtagtagtcaatcaagcagtggtggcagtcctaacaacaatcaaggaacaactactaataatcaaacgaataacaacaataatactggccaaaacaatggcggcggtaataattaa

SEQ ID NO: 87 - DNA, 6270 bp, Lactobacillus jensenii CCOS 962
atgttttcaaaaaataatatgaaaatgcgcatgcaaaaggttgctgataaagagcaacaacattttgctttgcgtaaattaaatgttgggttggtatccgttttaatgggtactacattatttttcgtgggacaaacatcaatagctaaggctgatacactagaatctactaagactagtgtcactgaaattagttctagctctaattctaatcaagaaaagttagaacaagctaaggctgtaagttctcaagagcaaactacaagtactgaagaaaatgtagattcagcttcatcaagtcaatcaaaaagtgaaaacaattctagctctagtgcgaagtcagaagtaagtactcaagatagaactgatagcaatgacaatgctactactaatcaagtagatactacgcaagtatctactacttcattgaaagctgttcaatcttctaatcaagctgctaacttattagctgaaagcaaagttgaagattcaacaacagctaatgttagtgatttcgattcatttaactcagctttgatgaatcaaaatattactactattaacattaatagtgactttacaagtggtaactatggtacaaatgttgaacaccgtagagttgttcctcgtactttagtaattaatggtaatggtcatacagttgaccttggttcaattggttacttcatgaatccaggtggtaatcaagcagctgattggacagtagaaaatggtactttctattctaagagtgctgttggtccatttgctcttactggtgatcacggtactgataaggcttggcaggcaaccaatggtgcagtacaccgtatgacttacaaggatatgacagtttatgctggtggtggtgcttatgctgcaaatgctgaaattgatttagaaggtactaacaatttaaacgctaccgcttcatatcaatctaagttctcaaatggtactgtttatactgaaactggtggtaacagatcaggtgttgaaggtcaatggattattattaaggataatgctaatgtgactgttaacactgatcacggtcaagctatttcaactgaatactctgatggaaatcacagaattgaagttggtgaaaatgccactttaaatggtaactatttatataccacttacggtactccttatggtggtggtaagatagctgttctttcaaacggtgcaaatggtggtactgtaatcttccataagggttctaagtcacactttactatgccaaatcaaaatgtaactggctttggtggtaatggttttagtaactatggtactggttctgttctttacttaggtgcagctaatactactattgaaaaaggtgcagaagttacaattgataaccctaaagaagctaataacgataacagtatcttcattcgttcagacggaacacaattaaatatctttggtaacttaattatcaatgatggtgcgcgtgactatactattcgtgccgataaccgtgtaagcatcaatgtgggtcaaagtattgcagatgatgattacagtaatgataatggtaaattaattattaatcgtaacggtgacttctacttgaataacgatggtggtgctctctcaatgtggggaccaattaccattaatgttaattcaggagctgctttagaagtttactcaactggaattaataatgtatctggttctggtgcaaatcctgctttaatgagagttggtggaagcagtaaattaaacgtttataaacgtggtactttcattttaagtgatagtagtaatggtaaagttagtctagttgatgattacaatgcaaatggtaacttcaacttcgacaatactgcaaaagttatttttgatatttcaaacaacaataaccaaaatagtagaatttttgctttaaatggtactgtatatgcaactcatgacaaggtaagagctatgctcacaccaagttctaatattgctgatatgggtacctttaagacggttcaatttaatactagtggtcaaggcggtgtgactggggatgcattacactctgagtatcaaaaccaagcctacaataacattgttgcgattagagatgcgattagaactggtcaattacgttaccttgaattctcaactcgttcagtaaataatgcaagtattactggtgaaggacatggctttactgataatggtgcacaaattaagggttcagtagttgatgaatcaactaacactggtgcggtagccgttgcctacgacaaagataataataaagttggttcaggtaatgttgatgaccaaggtaactttacaattaacttagataagccgcttcttaacaaagaagaagttaaagttagaattgaaacccctcgtggtgctagtggttttgtttcaactaccgctcctttaggtccaactgctaagagtccaattactgttgctaaagatgataatttagcaggtcaagatgctagccaatacatcaccaataaagatgaaattgcaaacattaagccaggtactactgactatgaaccaacctttaagagtgcagcttggaagagtgttgatactaataccaagaagggtattattactgtaacttatgcagataacactactactgacttagacgtagacttaaatgtagtagacaagattactgatgctgacaagttcactccagaaggtggaacaattaaagttgataatggtcataaattagatggtaatgatgcttatgaagcaatcaagaaccacgatgatttaccagcagataaagcaggctacaactgggttgtagatgaaaatcatccagccgttgatactactaagcctggtgatcaaactggctatgttcaagtaacttacaatgatggcagtaaatcagatttagttcctgttactgttcatgtaattgctgataatgaaaaatacactgctattggtaagactcaaaacctccaaaaaggccaaagtgcaaatcctcaagactttatcgctaataaagatggagaagttagccaagatggcaagacctatactaagttgcctgatggtactaaatatgaatgggtagatggaggaattgatacttctactattggtccaaaacaagctcaagttaaggtaacttatccagatggaaccactcaaattgttccagtaaaggctaacgtatattctgatgctaacttatcaactgttgttggtaaggatattaatgccggatacaaagaagacttgactaaccgtgcaattgatgcaattgataaggataagtcaactaaccttccaactgatccatcagcttatacttgggtaaatggcgcacctgatacatcaaagacaggtgatattccagcgactgtaaaggtaacgtatccagatggttcatacaatactgttgatgtaactgttcatgttactagtgatgctgaaaagtattcaccagttccagagaccatttctgttccaaagggtactgacttatcaggtcgagcaaaagatggtattgctaatgctgataaagatgctaatggtaaggaaaagttaccagatggtacaaaatatgaatgggacggcggagttccaaatacttcagtaactaataataagtatggtcatgtaaaggtaacgtatccagatggtagttctacagtagttgaagtacctttaaatattaccgataataataagtcagatgctgaaaagcataatccacaagctaatatccttcatgcaacattgaatcaagatcttagttcaaatgattgggctaaaaaaggcattttaaatgctgatgagcaagatggagcaacatttagatggagaaagggttatgttcctgatacttctaaagaaggccaagtttggggtattgttgtagtaagctatccagattcatcaattaatgaagttcgagttccagttatcgtccaaagtgatgcaagtaaatacggtattgaaactcaagaaatcaatgttcatgaaggaaccgatattagttcagatgaatgggctagaaaaggtattttgaatgccgatcaagctggaaaacagaatgaacaattaccagatggaactagctacacttgggcaaatggtaatgttccagatactacaaagccaaataagaagacaggttatgtaactgtaactttcccagataatagtagcagaactgttccagtaatcgttaatgtaattggtgatggtagaagtgatgctgaaaagtatcaacttaaggctcatgatatttggacttatataaacgatactcctgttgcagaaaaggcagtttcaaatcttgacgaactaaaagatgttagttcaattacttgggcaactacaccagatgtttctaaggttggtaacgttccagcgattgtagttgtaacttataaagatggtacttctaatgctgctcctattaacattgaggttaagggattagcaaatgattataagcctgaaggtacaactatttatgcaggtttaaatgaagatataactaacagagctgcagatggtattgctaataaagatcaaatgccagtagcaaataaaccagaaggtactgttcacacaacttattcatggaaggataatataattcctgatactactaaacctggtaccaagtatggaattgtagaagttaacttcccagatggttcaactaaggatgttccagttgaagttaaggtaactagtctagcatctgattaccaaaataagattgatactaagcaaattattgctaagtacaagggtaatatacctcaagcctctgacggtattgctaacaaagatcaagcaactaaagaaggagacaaagacttcccaagtttagctgatgtgttagctcctaatggtattcaatggaagaagaactttgaacccgatttgagtaagccaggcttaacaagtggtgaagcaattcttacctttaaggatggttcaactgccgaagttacaattccggtattagttcaaactgatgctgatcgcaatactccagaaactcagactattaagacacttcctggacaaacagtaaatcctgaagatggtgtaattaatttacataagcctggtgaaaataacccacaattgccagatggaacgaaggtaacttttgataatcaatcagatgttgatgactttactaagcatggaatgccaggttctgataagagcttcgatgctactgtaacttatccagatggaacaactgacaagattaagttgccggtacacattacagctgataatgaagttaatactccaattactcaaggtattattacacctaaggatagtgtgccagatgccaataaaggtattgctaacttaaagaaggctactaccaaagaaggtaaaacttatcctgcattgccagagaacaccacggttgaatgggttaaccctggtcaaatgaagactgagcttgaaaatgcaaagggtggtacaaccaagaattacgatgctgtagtaatttatccagataaatcaactgaaattgtttcaattccagtaactgttgctactgatgcagatacttataaagtagtaacacaaccaatcgatttgaaggatagaaacttacctgacaacgctgatgatggaattactaaccttcataaaccagcagactttaagactccacaattgccagatggtacacatgcagaatggcaagataaggatgctgctcaagaagtagttaagaacttgaagccaggtgaaactgtaaaacttccagctactgttgtcttcccagatggttccaagaagggtgaaggcattgatgtaagtgttcacttacatggtcaatctgatgattataatattgaaacacaaccagtaaatactgataaagatggtaatttacctgaaaatgctgactctggtattaagaacttaggaaagttacctgaaggaactcacgcaagctggggtgatggtgcccaagatattgccaagaatttgaagctaggtgaaactaaggatgtaccagcaacagttgtcttcccagatggctcaaagaaggaaattacaattccagttcatagagaaggtcaatctgatggttatgatgttgaaccacaactagtaaatactgataaaaatggacaactacctaatgcaaaggaaggtattaagaacttagccgatttaccagaaggaacaaatcaacctgggcagatagagctcaagataaaattaataagactaagcctggtacagatacaactgctcaagtag

SEQ ID NO: 88 - DNA, 645 bp, Lactobacillus jensenii CCOS 962
atggcacgttcaggatctcgagtaaaaaaaacaaccctaactttagttaaagtctttggagtattacttatcttagtagtggcgtttgtttgctttcggtattaccgtagacaagcaatcaataatgaattaattagacaagaacaactagcaagagaacaggctgcagctaaggaattaaagataaaaacagatttcataaaaaaaatagggccaattgctcaaaaagctgatcaaggctttgctcttttgccaagtattacaattgcccaagcttgtttagaaagtaactatggccaaagtgaactatctcaaaagtataataatttatttggcgtaaaaagtaatgatcccaatacttcaaaaattttatctactaaagaatatgttaatggcaaatggattacagtaaaagctagtttccaaatttatgattcatatgaatcttcaattcaagctcatgctagattatttcaaaatggtactacttggaacaaagatcaatatcaacatgttttagcagcaaaagattataaaacccaggctaaagcactagttacagatggttatgcaacagatcctgattatgcttccaagttaattaacttaattgaacaatttaatttaaataaatatgacaattaa

SEQ ID NO: 89 - protein, 558 aa, Lactobacillus gasseri CCOS 960
MLAQAAVESAWGQSGLAQSPNNNLFGIKGSYNGQSVNMNTGEYGSNGYYTTNAGFRKYPSYTESFEDNGSLLRNQMGNYYSGTWVENSKNYAQATQNGLQGKYATAPNYAQTLNSVIAANGFDKYDPVTQVVNENRTVAQTTPIMSAPVDASVGTQVGTARTGQNVNVTKYITYNNGVKRAYIGTGWINALAFSPITTNTTTKQNTAANTNNQASQAVKTPVAQTQQVKSQAPAAPVKAATVKVKSAAEVKTPVQTTTLNVKTENKAAQPVKQLAVSLAVAPKKVEVKKNVVKAEPAKTTPVKTETTKTENKEVKTATPVVKTTDTVKKVETPAVKPVESVKKESTPVVKTTPVTVTKEAAKTTEAPVVKPKKVEVKEIKTTPVTTSAKTVVKPVQSYQSAVTTAANNNYGTQWISTNTAPKAASTVLIKVTKTVDVLSAPDGQKLDQQVEAGSEFVVVASKYYNGNLYYEISNGKWIMAKYTTQEAQITAKSGVLTINSKPDYGVPVWRVPGQDQIAGKFLKDGSSWRYFRVANVQGQTWYDLGGNQWVSAKSVLVR

SEQ ID NO: 90 - protein, 208 aa, Lactobacillus gasseri CCOS 960
MPRRRRQKNIQYVIARAFAICFTLVVILSGFLYWRHEVAVNEQLRQAQLEKERALQSKERFIKVVAPIAQRADKPYGLFPSVTIAQACLESNFGQSELSKKYYNLFGVKGTDPNTSRELTTSEFVNDHWETVTGRFQIYNSYEESIQAHTRLFVNGTSWNKDQYQHVLAAKDYASQAQALETDGYATDPGYAKKLIDLIKEFNLTQYD

SEQ ID NO: 91 - protein, 513 aa, Lactobacillus gasseri CCOS 960
MVITLLTLDLEKYPSYTESFEDNGSLLRNQMGNYYSGTWVENSKNYAQATQNGLQGKYATAPNYAQTLNSVIAANGFDKYDPVTQVVNENRTVAQTTPIMSAPVDASVGTQVGTARTGQNVNVTKYITYNNGVKRAYIGTGWINALAFSPITTNTTTKQNTAANTNNQASQAVKTPVAQTQQVKSQAPAAPVKAATVKVKSAAEVKTPVQTTTLNVKTENKAAQPVKQLAVSLAVAPKKVEVKKNVVKAEPAKTTPVKTETTKTENKEVKTATPVVKTTDTVKKVETPAVKPVESVKKESTPVVKTTPVTVTKEAAKTTEAPVVKPKKVEVKEIKTTPVTTSAKTVVKPVQSYQSAVTTAANNNYGTQWISTNTAPKAASTVLIKVTKTVDVLSAPDGQKLDQQVEAGSEFVVVASKYYNGNLYYEISNGKWIMAKYTTQEAQITAKSGVLTINSKPDYGVPVWRVPGQDQIAGKFLKDGSSWRYFRVANVQGQTWYDLGGNQWVSAKSVLVR

SEQ ID NO: 92 - protein, 104 aa, Lactobacillus gasseri CCOS 960
MKKRTFTGIATAALITTAGISVTNNLKPENPLKTGEGTVQAATYQQEFLNKAIPAATTASSKYGTYTSVMLAQAAVESAWVNQVWHNRLIITYSVLRALTMGNQ

SEQ ID NO: 93 - protein, 772 aa, Lactobacillus plantarum CCOS 893
MLSTALLPMLSGKADTASTNQKPAAATKGNSAASAASQQVTLSAGSQTETTAAGATDQSVASDGAKTDDQAESTSTTTATTSATSRVTVRAASQVAKADSTELQSQSSASEAAKDNAAASATADSTTSAVDQLDKTAKASAATSQASHSTTNETAKASAAASQDSHVTTDQSSVTVTSEVAKSAASSAAPKQATEQAVAAKISPKIETAVAADAVQSSAMMARSTRAMTSQEIFLSQIKAGAISGWNKYQVLPSVTAAQAILESGWGQSQLATQGNNLFGIKGSYHGQSIYFPTQEWNGSQYITIQDAFRKYPNWSASVEDHGAFLVVNPRYSNLIGVTDYRRVASLLQQDGYATAPTYASSLISIIEYNKLHEWDQEALSGQASGGNDNNQVQPDQDVTPTSGTHKFTKTTTIHNAPDATSAVVGTYNAGETVNYNGKLTVGNATWLRYQSYSGVSRYVMISQTTTNDNNNQATVTPASGSYKFTAKTNIRSAASKTAQVVGTYNAGETVYYNGKITTGGTTWLRYLSYSGAQHYVAMSGDEVGSVAKPDVVATSGSYRFTKTTAIKSSPATSATTVGSYNAGDTVYYNGKVTTNGQTWLRYMSYSGAQHYVQISGESTSTNVDKPQVTPQSGSYRFTQTTAIKNTPAGNAPSVGTYSAGDTVYYNAKVTANGQTWLRYLSYSGAQHYVAISGNAATGNTTSKPVTNSQGAFRFVTTTNIRTAPSTRASVVGEYNPGETVYYNGTVQAEGYTWLRYLSRSGATHYVAKLEG

SEQ ID NO: 94 - protein, 212 aa, Lactobacillus plantarum CCOS 893
MAGKRRKSRRKQRTKTQLFVKKGRLQWVNILLVLAAMVGMVWYIQHNWAVKSRVTATAPTTTHAAFIKKLVPAAQQLDQQYHVLASITLSQAILESDWGQSTNATENNNLFGVKSTSGRLMTTQEYYDGAYHTVKRRFAVYDSWHASLVDHAKKLAYGTTWDSQHYAAVIKATDYQTAAQALQTAGYATDPSYAQKLINIIQKYDLQRYDRK

SEQ ID NO: 95 - protein, 421 aa, Lactobacillus plantarum CCOS 893
MSSVLGITLAKPVQGKADQTSSPSTTKVKAATSGATSEVSSISTITANSATNVSSATHQFSTATTTSQQASSATSNISTTTASKQISKSTTGKLNSNETATTSNSAATSVDSTAPYIPAKSNVSFTDNIKSTIANTPTTVAAPAIPSHSTQFIDDSAPITSPTPVTTNSIHVRPFTVHSSFSFKPGQFLRFTLPNVALLRDDVEQGVPNYVKNFFIAIKPGAMIGWSQYHILPSISGAQALLESGWGKSTLSVQGHNLFGIKGSYHGHSIEMPTTEYLNGEDVTIEATFRKYPDWATSIVDHGAFLNQNSRYRNLLGVKNYSTVAWDLQNDGYATAPNYATSLINAIQDYDLQEWDQEAFTGNTGSTTTTTGNHRSGTYTFIQNSNIRTEPSLSAPIIGVYYPGDVVNYTGQIKAEGYTWL

SEQ ID NO: 96 - protein, 258 aa, Lactobacillus plantarum CCOS 893
MVVPVDIWNQRGDASDQVTLKWPDNRKPKAAFTVNRTLAAPGNTIKFTNASSKNATSYKWEFDGATKTTSTAKNPTVTYRKAGTYNVTLTAKNKDGQRHVTMKKLITITPKAQGALTLLSKNAKTSASGYTNSSEAPKMAVDGKLDTKWCATGKAPHTLRLDLGRQTTVSAVKLAHAKAGGEGADMNTRAWTIQVSTDGKRYTDVARTYNNTQATSLNTFAATSARYVRLVVDKPTQVADTAVRIYEMDVLGLTQTLK

SEQ ID NO: 97 - protein, 94 aa, Lactobacillus plantarum CCOS 893
MRKDTASTIKLYTTDLDVTADTQVSLTAKASGKSTAKLVVTLKDGRTKTIAGDRTLSKHWTTVSYDVSQLTKKQSKALASKSVPPRLMLATAFN

SEQ ID NO: 98 - protein, 408 aa, Lactobacillus crispatus CCOS 961
MKKRLLTSFAAAAMLTSVAVPAVNTTMMNQASSQRVSAATADQTAFLNKAAKQAVKAAKKYGTLPSVMIAQAITESGWGKSGLAVNANNLFGMKADDSWTGETYTAKTREEDKNGKSYYITAKFRKYPSFEQSFEDNGSKLRNGVSWDPLRYKGTWIENASTYAAATKALTGTYATDSKYDKALNSHITSSNLTKYDPVTVNTTRTYTAGKDSSTYNWPTAPSVASVIGSVKAGEKVVVTKTITFHDGSSRMYIDGRGWVNGSVLDKSSSATKEPVTQAPKNVPAVSKNLMHNAYVYDQNGKKLKGKMYKTSDENGGKWINTYGTKTIKGKTYYRVGENEYIAAGNIDGSLRFLKKNAYVYNQYGNRDNNLKHKKNSQIATYGSAITINGKKYYKVGIRQYVKKSNFM

SEQ ID NO: 99 - protein, 215 aa, Lactobacillus crispatus CCOS 961
MARKRKSRVPKSVKTVVRVFVILFILMVAFVGFRYYRRYAIQSEQIQQAQLQKEQEAAKLLKQKKDFIKKIGPIAREVDKSYDLLPSITIAQACLESNYGQSDLSQKYNNLFGVKGSNPNTSAVMTTKEYVKNKWVTVKARFQIYDSYEASIRAHARLFQNGTTWNHDQYKHVLASKDYKTQAKALVTDGYATDPDYADKLINLIEQFDLEKYDK

SEQ ID NO: 100 - protein, 430 aa, Bifidobacterium bifidum CCOS 571
MRMQQIKHGGRRPRPSSAPTIIAAMLCVVALVAAGTAWWMLRPQQKDTLEHLAQPQSSSSTLNRDKAPTPKPQKSQERQKAAGDSPAAKASRAIATMSLDERAGQLIMAPMFAGGNPADLSALISTRHVGSVVLIGNWNNGTAAAKTAADALQSYAPSGNQLIVSTDQEGGQVQHLKGSGFDTMPSAVAQGQMSADTLRSSAKTWGGQLKQAGINVDLAPVLGTVQVKRSSNAPIGALNRDFGLDSNGNAQHGIAFVEGMRDAGVGATVKHYPGLGAVTGNTDFTTEGILDTTTTLDGEEIGAFNTTIKQAKPAMVMMSLATYQRIDSSAPAAFSSKIIDGTLRGSVGYDGVVISDSLSAAAVSGIATKDLGVRLVDAGGDLACIGDTSYVTPILDGIIARAQSDPAFAKKVTASATRVMTLKYQMGLAK

SEQ ID NO: 101 - protein, 1935 aa, Bifidobacterium bifidum CCOS 571
MAVRRLGGRIVAFAATVALSIPLGLLTNSAWAVEDATRSDSTTQMSSTPEVVYSSAVDSKQNRTSDFDANWKFMLSDSVQAQDPAFDDSAWQQVDLPHDYSITQKYSQSNEAESAYLPGGTGWYRKSFTIDRDLAGKRIAINFDGVYMNATVWFNGVKLGTHPYGYSPFSFDLTGNAKFGGENTIVVKVENRLPSSRWYSGSGIYRDVTLTVTDGVHVGNNGVAIKTPSLATQNGGNVTMNLTTKVANDTKAAANITLKQTVFPKGGKTDAAIGTVTTASKSIAAGASADVTSTITAASPKLWSIKNPNLYTVRTEVLNGGKVLDTYDTEYGFRWTGFDATSGFSLNGEKVKLKGVSMHHDQGSLGAVANRRAIERQVEILQKMGVNSIRTTHNPAAKALIDVCNEKGVLVVEEVFDMWNRSKNGNTEDYGKWFGQAIAGDNAVLGGDKDETWAKFDLTSTINRDRNAPSVIMWSLGNEMMEGISGSVSGFPATSAKLVAWTKAADSTRPMTYGDNKIKANWNESNTMGDNLTANGGVVGTNYSDGANYDKIRTTHPSWAIYGSETASAINSRGIYNRTTGGAQSSDKQLTSYDNSAVGWGAVASSAWYDVVQRDFVAGTYVWTGFDYLGEPTPWNGTGSGAVGSWPSPKNSYFGIVDTAGFPKDTYYFYQSQWNDDVHTLHILPAWNENVVAKGSGNNVPVVVYTDAAKVKLYFTPKGSTEKRLIGEKSFTKKTTAAGYTYQVYEGADKDSTAHKNMYLTWNVPWAEGTISAEAYDENNRLIPEGSTEGNASVTTTGKAAKLKADADRKTITADGKDLSYIEVDVTDANGHIVPDAANRVTFDVKGAGKLVGVDNGSSPDHDSYQADNRKAFSGKVLAIVQSTKEAGEITVTAKADGLQSSTVKIATTAVPGTSTEKTVRSFYYSRNYYVKTGNKPILPSDVEVRYSDGTSDRQNVTWDAVSDDQIAKAGSFSVAGTVAGQKISVRVTMIDEIGALLNYSASTPVGTPAVLPGSRPAVLPDGTVTSANFAVDWTKPADTVYNTAGTVKVPGTATVFGKEFKVTATIRVQRSQVTIGSSVSGNALRLTQNIPADKQSDTLDAIKDGSTTVDANTGGGANPSAWTNWAYSKAGHNTAEITFEYATEQQLGQIVMYFFRDSNAVRFPDAGKTKIQISADGKNWTDLAATETIAAQESSDRVKPYTYDFAPVGATFVKVTVTNADTTTPSGVVCAGLTEIELKTATSKFVTNTSAALSSLTVNGTKVSDSVLAAGSYNTPAIIADVKAEGEGNASVTVLPAHDNVIRVITESEDHVTRKTFTINLGTEQEFPADSDERDYPAADMTVTAGSEQTSGTATEGPKKFAVDGNTSTYWHSNWTPTTVNDLWIAFELQKPTKLDALRYLPRPAGSKNGSVTEYKVQVSDDGTNWTDAGSGTWTTDYGWKLAEFNQPVTTKHVRLKAVHTYADSGNDKFMSASEIRLRKAVDTTDISGATVTVPAKLTVDRVDADHPATFATKDVTVTLGDATLRYGVDYLLDYAGNTAVGKATVTVRGIDKYSGTVAKTFTIELKNAPAPEPTLTSVSVKTKPSKLTYVVGDAFDPAGLVLQLNYDDDSTGTVTWNTQTAGDFTFKPALDAKLKVTDKTVTVTYQGKSAVIDITVSQPAPTVSKTDLDKAIKAIEAKNPDSSKYTADSWKTFADAMAHAKAVIADDSATQQDIDNALKALTDAYAGLTEKTPEPAPVSKSELDKKIKAIEAEKLDGSKYTAESWKAFETALAHAKAVIASDSATQQDVDAALGALTSARDGLTEKGEVKPDPKPEPGTVDKAALDKAVKKVEAEKLDGSKYTADSWKAFETALAHAKAVIGNANSTQFDIDNALSMLNDARAALKEKPGRIIAIIDGSALSKTGASVAVIASVAAAMLAVGAGVMALRRKRS

SEQ ID NO: 102 - protein, 154 aa, Bifidobacterium bifidum CCOS 571
MHSRPMFPIPETQVGDGWVGDVDYTKQATKQDSNFLVDWVRVYQSEGQPVTRFDDLDGAESGAYRSAPASRTEGLTAVSNGDAAWRNKNNFYYGGQPRYETSRSHAVPLMQGRFALRLRGPQTLCRIRTNAFTRSERPVAGKVVPPNRRNRAAP

SEQ ID NO: 103 - protein, 185 aa, Bifidobacterium bifidum CCOS 571
MISASREIHSINLYRNGYENALNTFKRIKVEVSSNEDFSDANVLFGTADVEETAATKLAAQTINLTTPVTARYVRIWQKGHCIQNTNSSWKGYGNGVGLREIEVIAKLKDGETLPDAQETRNIALGKLPYVYGLDPTNIAAISDGKQDDNYAVHNSTGERWLQFEYKNRYRIHEGSSRAPIRWSA

SEQ ID NO: 104 - protein, 108 aa, Bifidobacterium bifidum CCOS 571
MRQLFRRITTISATCALAVSVAAAVAVAAEPTTGNILTGKLPTTNSTHLIGDGDTGFGPTDSNITKIIAGEENGSAENNGYASWDDVYLQYDFGEPRDTLHQPVPQWV

SEQ ID NO: 105 - protein, 1931 aa, Bifidobacterium bifidum CCOS 571
MRKRVVSVALAVALAVAPLGVVSTASAAPLSASDLQTLALRSAASSNDANANDVATVADDAAVNGWTIDRNTAKGGEILAAGTGDYAGWTHFKSTSANGNATSSSGYPAVAISGKTIDLTRAGEFSIKVKSPQAGSANRFGFYLGYKDPGNALFLGYDKGGWFWQKYVGGNGDWYNGTRVAAPAANAEITVNVSWTAAKVATLTIDGQKAFDVDYSSMTALTDKLAMKAGSYSGTSEVTDVYFKNFTVGEVAKHNVTGKVVDASGAAIAGAEVVTGKNSATTAADGTFTLTGLAAGDYTLTVSAEGYDDATKTVTVADGNASVGNITLNKSAEVATETLSTAAMDVRVKKNFPSVYDYTMKKLDGKIMYGQPKDVRVITINGTDVTLKDSDVTFKKVSATEAQYTLNVKSGDKINAVVTVQIKVVDNTLKLNVTKIVNKADDAKTEAEENPVQTIAFPNQSLISVRSGQDGAQFTGARMSSDTARPGDTNFDITADTTVSNANDYTYGFVSGNGLSAGLWSNSEHDGTTVGNTVAGGARNTRVLTSTQKVGKATSFGLGTAPWYYHRVVTDTKKNTYTVEETDMPKMAVAIAGDENEDGTVNWEDGAIAYRDIMNNPYKSEEVPELVAWRIAMNFGSQAQNPFLTTLDNVKKVALNTDGLGQSVLLKGYGNEGHDSGHPDYGDINTRAGGAADMNTLMEKGTKYGARFGVHVNASEMYPEAKAFSEDMVRRNSSGGLSYGWNWLDQGIGIDGIYDLASGMRKSRFADLKSKVGDNMDFIYLDVWGNNTSGAEDSWETRKMSQMINQNGWRMTTEWGAGNEYDATFQHWAADLTYGGSAMKGENSQVMRFLRNHQKDSWVGDYPSYGQAANAPLLGGYSMKDFEGWQGRNDYAAYIRNLYTHDVSTKFIQHFKVVRWVNSPLDATSVKDASVNNGNEQITLKDDHGNVVVLSRGSNDTNNTAYRNRTITLNGITVASGAVSPGNSNTVKGTESYLLPWLWDVNTGKLVKSSDEKLYHWNTQGGTTEWTLPKDWQNLASVKVYQLTDQGKTNEKTVAVSGGKISLTAEAETPYVVTKGSEKQISVKWSEGMHVVDAGFNGGQNTLKDNWAVSGTGKAEVEGTNNAMLRLTGDVKVSQKLTDLTAGKRYAIYVGVDNRTNSPAKITVTNGTKVLATNETGKSIAKNYIKAYGHNTYSNTEGGSSYFQNMYVWFVAPESGDVKVTLSHSGACDNTDHVYFDDVRVLENGYKGLTLNADGTLKTLTNDFEDNAQGIWPFVVSGSEGVEDNRIHLSELHDPFTQAGWDVKKMDDVLDGKWSVKANGLIQKGTLIYQTIPQNVKLEPGETYKVSFKYQSGSDDIYAIATGDGEYNASTVKLTNLKKALGEDGTAEFEITGSITGDSWFGIYSTSTAPDLQNTSDSAANFGGYKDFVLDDLKVEHVASAEHTKADAEAKLKEVKDTYDGKSGDYSAEVWTTYVNTVAEIEALIAKDKPDYTTAYNKAVALAEYMKNAPGDDSNDAYDVATDAYTVEAGSQQALSGGNEGPASLAQDGNAGTHWHTSWSANAVSAGTAWYQFNLNEPTTIDGLRYMARSGGANANGKIKKYKITLTLSDGTTKDVVTNGTFTTTSGVWQKVKFDAVKNVTKVRITALETAGQSAGEVNTYASAAELRVTTVRDVPSTEVKVNKCDLQNLYDDASALTEATYTADTWKVLVAKRDAAKKVLDDENATAHDVALAYQNLKDAIAALEERVDTSKLAGLVADAEKLKESAYTKDSWAAFKKALDAAKAVLNNANATKADVDAAYNALNAAMKALKPASSKPTPNPETTDKSKLQATIDQAKALDLSGYTKKSAQAVRDALAKAQSVLADDNATQADIDAAQKALADAIAALEKADANGNAISKTGANVAVIGMAGMMLVAAAGAVFIARKRAE

SEQ ID NO: 106 - protein, 867 aa, Bifidobacterium bifidum CCOS 571
MVSPHHLLKIATALSAVALTASVAVTPAYALQDIAIEDAVAQSGPVTADNGVVVQSDDQSDDQTGDQQSQDGMPDNPNAKLPDTVSDEISDDATVVSEDLAVTPEGEVKNIETGETVTDATLVGTQDQQPDPLAKTNGESFIPVSAEDVKNAVADANVQLSKFEGNEYGAHWGTYNNTKAFFDYQNNLFVQQAKGVIDVSEWQGDIDWAKAKADGVEGVIIRLGYGWGNNADRKAQRNISECKRLGIPFGIYWYSYADTPSIAKEEGAGVVAKLKRFGVRASDLAYPVYYDLEKWTWKGHQPPTDPNVYSDIVNNWYGALQSAGYKNLGVYSYTSYLQGPLKHADIYAKTTWVAQYGARMGFDSFPTNSRGWQYTSSGKVGGIRGNVDMNAFGNKEYVNGGSSNDLQAAIDVRKMTAVTIPNGNYYINVRSKVASSVDVPGGSAADSTAIQLYSGNSSKAQQFTFTRQSDGSYEIVNVNSGKALDVRNGVAENNAVVQQYSRNNSQAQRWFIRDSGAGSYLQSALGNWVLDLSGGNTANGAAIRLYAPNGTASQLFVVSSSDASIATGVSMIITSVANKKLVTDVTGASTANGARVQLDSSNNTNAQKYRFESIGNGTYKIINANSGKVLDVAGGSTADGAALQQYTSNNTVAQQWTVRNYGSGRIALVSVNANKAVDIPGGNAVQQAQLQLYSPNGTVAQQWLVAKAPLTLRERLNETAAKHRQDLPDGTYTFGSKLNTSMKMDVSGASRSNYGNVQIWAGNGTNAQKWKVTHDSNGYVTLTSVNSGKVLDVNGGVSANGTNVQQYDSNGTYAQKWIAVKNSDGSYTFQSALAENKVLDVSGASTSNGANVQLYTANGTNAQKWVK

SEQ ID NO: 107 - protein, 778 aa, Bifidobacterium bifidum CCOS 571
MSFDLIPEPQSVTLKGDAADSDDAGAPVPVALPLVGRISEDRDIDDIAGVFPTQLADDIEAATGLRWDIASDVMVAGLPAPNAAIAHPVPPHASCWKSFITLRLDPPSLEPQEYRLTIARSGIDVVGGDTEGVRNGVQTLRQIIRQCAPALPRLVIADKPAYKVRGYYLDATRGRVPTLDWLKTWADRLCLYKYNQLQLYIEHTFMFDDLSETWRGTSPLKPADIIAFDEYCARLGIELVPSVSTFGHQYMAMRTRELRHLGEFPEDADRRYGFVERQRHHTLNITEPESLAFSFKLIDAYMQLFRTRKFNICGDETFDLGRGRSKPEAERRGVAAMYADFVSQLCRHLSERGRDPMFWGDIAVEMPQILGLLPDNVTLLNWLYAPGIGEDKVRLVAQAGAPQYVCSAVWCWNALLPRLDDSWNNISRLARYGVKYGAVGYLVTDWGDYGHVNDPRMAVSGMIFGAQCAWNPMAHIQGEAGCGDGEEGSAAGYADAAADVVRENKAAADGDSPAPLPSSSESDDYTGGAADAIAGAPAGGDGSCAEMCRRVAEVEYGDRSGGIVEALRDAACRVAFGWDDMVWYCELDEGDGRMNRDAASAMHLGVHGFSGEYGREWEARLLGSADLDEARRTMLQGLSPHIVRAAEANEALLCDAMRLGAAAGRASRLGAARRDVPAMLAAIEGQRWFNLVGLCLARRHDVITVDAGDIARASAGLIEPDAGSSAGPEAVQDVSIRVARGLERWFETYCDLWRSVSAESELARIASIVWRCADALRS

SEQ ID NO: 108 - protein, 304 aa, Bifidobacterium bifidum CCOS 571
MADRFGAFLPHDTSGDVAQLHGIGLQKFGDTWYAYGENKVNGNLFQGVCCYTTTDFIAWRSHGIVLDVQEDGSALAADRIGERPKVLHCPATGKYVMYIHAETPDYGYAHIGVAVADAPTGPFAFQTTITWRGYLSRDIGVFQDEDGSGYIMSEDRDHGTHIYRLADDYLTIVEDVACERATDYPYGLESPTIIKKDGLYYWFGSQLTSWDTNDNKYSTATDLHGPWSEWKLFAPEGAKTYDSQVDIVVPLDDDPYNSEHFLFIGDRWQEHDLGNSPIVQMPISIADGVASLTWSDTYEGTTHR

SEQ ID NO: 109 - protein, 634 aa, Bifidobacterium bifidum CCOS 571
MMQFTMSGTMLRFDETTLRFSFSRDGATWSGCDGIEPQLTREDRSFSFAGAATVTHERIETGTGVGVRSVFAGFAGADYAFETYIWIERSSGDVLCEWVPLRECGAEPRIDRVLWPAPLSFDHADAHDVTLITHEQGVMIPNNWPTEVGTDAVSFGGRFETAGGYMPWFAQLRSDGHAYIAICETPWNAGYDIDHPAGGPYTHVGMWFEPSLGRMDYRRVVRYRLLDHADHTAVCKTYRAYVNERGRLRTLAEKAARNPSVRDLLGRSWVHVGIKTKVQPDSSFYDPAQPGKNDSLVTFAQRERQMRTLHEMGAGRLYLHLDGWAQPGYDNGHPDYLPACREAGGWKGMKSLVDACHEQGDLFGTHDQYRDYYFAARTFDPRNAIRLADGTMPEHAMWAGGRQTYLCAELAPDYVRRNFSEIATHGIALDCAYLDVFTCNEGDECSHPEHRMTRRGCYERRAECFEYLLAHGILTSSEEVSDWAVPSLVFCHYAPYDFQMRSPDAPRHGIPVPLYNLVYHDCVIQPWMMDRVAGGDDYMLYALLNGGAPYLIRDAAYAGMDGDMNAALRARTENDIERCAVVAGLHRRVGMQELVRHDLVGGDPLVQRSVFADGTAVTCDFHAQTYEVAANGSH

SEQ ID NO: 110 - protein, 1138 aa, Bifidobacterium bifidum CCOS 571
MRANGNSTHEILGKIVTAIASIAMTAAFAVPAMAASDSDTAADSGTTQQSGQYKIYPQPQNTEYGDGSLILRDKANTVVEPGIDSATKARLNEALKLKGIETTAADAVPETAYQLNVLVGINGSNGVVDKYAKQLIADGTLKVDDSTFSKNDSYVLAVRQGNAKTPDTILVLGRDTDSAFYGLTTLYQIFQQLPGRAVSNLTFSDWADVKSRGFIEGYYGSPWSTKDRVNLMTWGGYYKMNTYVYAPKDDPLHRNNWRGLYTEDQIENEIKPQAEAGNKSKVRFVYALAPFHNDGEARGKHFRFDTEEHYQKDLKELKAKYMQTIDAGVRQIALLADDSTDWGAQYGNDNTYVRVLKDLTDWIHELQQEKNDDGTAKYEGLKDTILYCPALYSYTGAGDAWYKDIPSNVQIVMTGGRTFGVASKDFADTFTKNTGRAPFMWINWPCSDMNRNTAYQYLVMGGQNNFLKPGATYGTYDGIMLNPMQQSEPSKQGIFMAADYSWNLWQSEKDGQQSWEDSFSYIDHNSPIASKGSRGLRDLAMNMRILNDGGIDGAHKDAEYDAVNKWWINNESVDYTGKLDVKGVLTELKGKLDGGTATAADFSQALTVYTTLQRAAKNYRANPGDKNMFDQIEPWISYWDDLTASAIDYITAAKQALAGDTETAKATYATAKAAFAKSDTHTIADYYQRNKPARGGLVIVRPTVQALDSFVKAKTSGSVTPTPSDATVSTNGVGAAAWHENVDPKAVIDGDDSTFFWMQSAGCDCVKANAALTVTYAEARKAKEFRFIQAEKGGDTIVNGKIEYQDADGNWTKIGDVNGNQKQIFTLDSAATVKAVRITNLAQTSKWWKVYDLSATKIDEPGTVTKDALNAKVAEAEKVDSADWTKSSREALADAIAAAKAVAADQDATQAKVDAAVAALESAMKGVERYTAKTADQLKAEHVSNDDATYTEASYNKYQSAYDDFAAALANADDLAKADGEALEAAYTAAKSALRYDQSARDYAQLALNDAEPYVGKASEYTKDSYAKFTVAYEALSKQLKADPNGEGDPATYTALRAALDKAIKGLVKSDGTELERPGEKPGEKPGENKPGEKPGVNKPGADGKLSNTGADVFGLIAAMTMLAAVGVTMAGLRKRIG

SEQ ID NO: 111 - protein, 1755 aa, Bifidobacterium bifidum CCOS 571
MNRRISMWLRGRGSPWRPAAAVIATVSMMLATVMGPHFAGMRAQAVEPVQTTTISHTKIAGDGNYFTFADNAWDPGNDVHTWSKAPSDSLPAEDIWYTVRFFGSAIDVYAGKNRPMGKVKYYIDGAEKGTYSLYNASNINETKIASFTGLDEGEHVFKAVATGERDTNSTNALIDCAKVVVTHQPYVVTGVTLDTTSMTLGVGDSKRISYTVAPDYATIDDMTYTSGDTSVATVGADGTVTAVAPGATAITVASTAAGISKIVDVTVARMAPNLTGGIVDPDTQYTQKRFDEVKALTTNNRALKAWKNDKVNSEISLAAVGTTVSNLTVTANDLTSQGGDVIAKSNVTATFIKSTKAYNGSYLGYGDPNREVPAATETNRSESNDILYQSGPITVKANQVQNIWVSFAIPKDAKAGTYTTTLTATADGMETPLTFTYTIEVKAATLPDPAEYEKNFDVELWQYPYSSAEYYGVTPFSDEHLQILRSSMELYKSIGGHAITTTINEDAWSGQTYSANAIHYPSMVKWTKSGGGFTYDFTDFDKWVTFNKGLGIGDKIVIYSIAPWHGNFTYWENGTMKSEKYTVGSERWRSVWTDFLRKLIEHLMDKGWFDESYIGIDERGFSADAFDLIDSIRNIHDVPLKTAGAMDGFVNKFDLALRVTDLNVGDTAAAAHPTDFTRLIEAREAKGLRTTLYSCTEHEPGNFSLSAPVESYWSVVNAGEQTSGFLRWAYDAWVADPLNDATHNAFEPGDPFLIYPSEKSGDKVSKSSVRLERIAEGVRDVNKIRLMVTEIPSLQADADAMYAKIRTTVTTSHSYLTAAQVTQLANEMSGFKGDLDTLTDKYISLKAQGTSTVESVAIDGGDQEIMLGTAKQLTATLKPANLLNASVTWRSSKTGVATVSAKGVVTAAGVGSTTITATSKADPTKSASITLTVTPQVVAQGLHYYSFDDSNANDSWGTRNGTADATAQYVDGKSGKALKVTDGKGVTLAGGNDIAKTDPWTIGYWVRSDAELTGRSAVMTSADGKYSADLKMDADRESGFRVGTASGDVLTFRYDFQPGTWYYIAWTQDKAAGLTMYVNGTKIGVTNTWTKMHDVVAPIDVIGGPGFTGLIDEVKIYKRVLSDTEIAAGMLLPGLNLAEHETDMYIGGTYTIVANLQGGDGDGTVTFESSDPTIAKVDASGTVTGVSRGTAVITVRGGGFTDMVTVNVSRELTIKNTLPQYKLDQTKVTDVHKSLDTSNQYFGQPDMIRTKSGRLITSFPQGHGKGPLIMKISDDDGATWTRKTDIPASWAGSQETPTLYVLNLADGTERIMMITACPGWGTDSAGNRYGWNTSYSDDNGETWTEYRHWQSNRTYDNANNDAIVAMASLVQLKDSDGNDIQKWMGVYHNYAYVNFRTYLTFDENGDEQWSESEPYLAQWRSIESAYQMCEIGMFRSPDGKRIIGLARSQSHNNPATLIYSDDEGETWSKPMDLPGSLAGERHKIAYDPISGRLLVTFREINYDLNGNNRFDGGNDWNAGDWVAWVGTYDQLINQEDGEYRILLAEDWTSNAKSGDTGYAGVAVLDDGTFIMDTYGHWDKEFSQNWPGGVTTDRCYIKQAKFKLGEVEYANGLIDRSGLKAAIKRAEALNAADYTADSWAKMDAAVKAAKAGDADDSLQQAQVDALAAAIDAAIDGLKAKDDGDKPGPGDGGKPGAGDGKPDDGGKPDPGKPGKGDETKPDTGKKGGLSATGAGIVPIAAAALTLMAGAALALAKR

SEQ ID NO: 112 - protein, 1627 aa, Bifidobacterium bifidum CCOS 571
MRLRRVKAAIGSVLAAVTLLSMSLTGVTAAQASDDNLALNQTVTASSYEVATTAPEKAVDGDLGTRWGTAQNKAANEWIEVGLGGTKTVKQINIDFERKDADQNITSFKVELKQGDTYTKVYQKDTRAKQQEIILLDQAQQASAVKVTVLSADGGTMNWVNVGINEISVYSAPKETVLDTADTNHMLGATMTASSNETATLTPDKAIDQNRTGRNNRWASGYETPSNIWLKAEFPRLTAVKDIRIYFFERDVNPKPTNVQSFDLSYTDSEGTEHTLKSGYAMTASGTGYVADVVIQLDQAVNARSLKLSNFAIKSSEYNNVSVAEWEAYSNDQAEPGATLDSVVSDLESNHLTIETDTDTLALPTVPDGYTVKFNGADYEQLIAADGTVNHPLVDKTVQVAYVVTDTATGNTKTTSDIPYVVKGTNQQQEGNNAKPTIIPEIAEWHSTSAAKLAASAVTKVVYDDDSLKAVVDEFVADYKDFTGIKLTAKKGAAEAGAFNFVKTDSTAAIAQLGDEGYTMDIRADRVVAKSSSVTGNMYAMQTILQMTKQDASGFVIGSMRDYPRFTTRGLLLDVARKPVSLEMMREITRTMRYYKMNDFQAHLSDNYIFLENYGKGDNEDEAFKAYDAFRLESSLTNDKGESPTAEDYSISKKTFKQFIQDERALGMNVVPEIDVPAHANSFTKIWPELMVKGRVSPINSNRPLIDHLDVSKPETIAKIKEIFDDYTKGDDPTFDSDTTVHIGADEFLYNYTAYRKFINEIVPYIKDTNTVRMWGGLTWINDHKTEITKDAIENVEMNLWSKDWADGLQMYNMGYKLINTIDDYGYMVPNGSYGRANAYGDLLNISRVFDSFEPNKIRSSGGYQAVPSGDDQMLGAAFAIWSDNIDKSASGLTESDLYWRFFDAMPFYAEKTWAATGKEKGTAAKLTALAAKQGTGPRTNPYYQATSKNSVYESYDFNDGLADASGNGRDLTIGDGSKAAVKDQSLKLAGGSSYATSKLDKLGNGNELTFDVTLQQAAKPGDILFEADAPYGTHDIRVMENGKLGFTRELYNYYFDYELPVGKTVTVTIKVDQQTTKLYVDGEFVSDATGKYIDKGIEKKTGITAATFALPLQRIGSKTSAINGVIDNVIVKKSEAETDQYNKSCWTGTTNSETQYNDTEGLLRYAFDNNPSTIWHSNWKGATDKLTGSNSFYAEIDMCQKYTINQFSFTPRTSQDSGQVTKADLYVKANANDEWKQVATDQVFEASRAKKTFMFDEQEVRYVKFVAKSSNDGWVAVSEFGVANKPSSTVRVFVAADPAEGGTVSVAAEGETGTDTAVDVASGASVTAKAVTADGYRFSGWFTTASETAVSTDATYTFAADGNTALTAKFTKDSTPDPGPKPTISSIAVTKPTVTDYKVGDTFDATGLAVTATMSDGSTKTLTAGEYTLSATQDGAAVALDKAFAKAGKVTVTVTANGKTATFDVTVTAKDPDPEPATLKSIKVTSKPDKATYTVDETFAKTGLAVTGTWSDGKTALLKDGEYKLSAVDADGKTVDLTKPFTAAGDVTVTVTSGKLTDSFTITVKAKTVTPTPGDNKPGENKPGADKPKPNTPDEVAKTGASVTAVVFSALLLLSAGYLLVRKRRI

SEQ ID NO: 113 - protein, 1960 aa, Bifidobacterium bifidum CCOS 571
MRSKALGGLLAAALSLSPAVAIGVQTAYAAGGDTAATEYTLYPKPHSIRYDSGQYILRDINVIYDDDIDEATQDRLDEVAALKNLNVTESDAAVSGKTNVYVGVNGSDGKAETAIESKYSPDSAIFDKTDSYFLKSDNGTISVLGKDTDASFYGLTTLYQVLGQIDSLTIRNFTVTDYADVVSRGFIEGYYGNPWSTQDRINLMKWGGYYKLNSYFYAPKDDPKHNSQWRTLYTQDELDTKIKPLADAGNASKTRFVFALHPFMNNAIRFNSEANYQADLKVLQDKFAQTIGVGVRQIAILADDAANVGGNNYTKLLTDMVAWLKEMKKTYPDLKTTLPFVTQEYMGNGMSYFANFPKEVQIVMTGGRVWGEVSQNFTDTFTSNVGRGPYMWINWPCSDNSKSHLIMGGYDTFLHPGVDPSKIQGIVLNPMQQSEPSKVGIFGNATYSWNIWRSKSEADQAWQDSFSFVDHNSAVPTAASNALRELSKHTINQNMDSRVTALQESVDLAPALTAAKAKLADGTITAHDLTDIKAAFVTLQKAAKTYRAKGDAKMLGDIGKDYTGQDANEQIAPWIDCWDDTTKAALAYIAGIEAALNGDTSSTLKEYSDAQSAFAASKKHGFYYVNHTEYAEVGVQHIVPFIKAMDSYLSNKVQQEADPNVVTKTYISDVFTTPTSGSIEDIFDGKDSTVTVFQNPNYLHKGNYVGVKFSKATTLKSIRFAFNGGKNHFYHSKLQTTTDGENWTDVPDATFERPKGSEEPIKVTGLNITGVTGVRLIATADNGDDLWLGIKGIDVNKVEKETLAPYTATGVQLENLNATYSSTKEQMIDGNPSTITYLKDPNGDKIAAGAAVIVDLGSSKPIGEVTITGHASSPDDRPSQGVVEVSDDKATWTKLGDLRDDVTSTVSGNVTGRYVRIRNTAAKNVWWRVAEITVTPPETADPLKSVYTNKTQHGYTATLGANTAELFDKSHTMLDGGQYAGLDLLAIRDLTDVELNTGNANPSLQISDNGLVWTTVEPGNLTGKTARYVRVINGTDGAAFSVNKLKVGFSTVGKFGKLVSSDIQKRNDWGTDTRESGNAFDGDMTTVIKFAGQPRQGNTAVFDLGQPIDITSLRIYTQDTQYDYIRDTKVQMSVDGKTWVDAFEIGDGVSDTDTTTAFGDISDTNKKTDSNYPNVFYYGKDDIANGTGMRYLRLLTTADYPQRALAFNEFMVNQGAYVSTEANAAFSATKVEERGHAPSNMIDGDLTTTYKPSAANGSLTYKIDDPSDIKSFRIVQSGAASGATVTGTVYDAATGTTAGVTARAAARSASEVTFGTLEQAINEFKVPDGKQLLSVKIAWGNAIPEISEFITLDSADTDADITTAKAALKEKIDATVDTSAWTANAKTAYDEAKATAQAVYGSPLVGKASIDAAASAVQSAIDAAQTKADAAAVAALRKLVDAAVTNDGHFYTTVTFTAYTDALDEVKEALKDTNNLSTADAASLKKAVDDALAALKDSTYQRELATIAVDSFATIDEADYTTNSYAAFKAAKEALDTLIAADGTKPATFKTKTAEYTTAKTALVNVAALKAQIAHESNYVEANYTADSWKAYSDALKAAKAELVNGTTDSVAAALTALTTAENALVRTTTPPDTTVLDETIADMEKVNGSEYTTDSYKALTDAIAKAKSDKAKGDAGLNQQNIDAMKAAKEALVSTVELKAKVAEAGKVDSSKYTTASYEALSKLLAAKDDTTSDPVVKGLDTLYKSGTVKELAERVAAIDAAVAKLDARATGVKDYVDGIKLKDNDKGYYTDASYKAYSDAYKALKKLAAAGEGEVGIAEFTEAKEAFEAAEAKLAYKSADYGKIDDLLAKVPSDLSGYTADSVAKFEAAKKAVKRGLTIDQQSKVDAMADALEAAIKGLTLKSQAPGGNKGDGTQSGTHKGDDISKTGADVQVFAIIIALATCAGLGAVAYARRRREA

SEQ ID NO: 114 - protein, 1923 aa, Bifidobacterium bifidum CCOS 571
MATLMCGLITSGRLARAVEPAIAGVTASGAAADGHAAAAAVDGDPATYWQSPADSSMQDYRRFLDFDLHGTYSISQIDITNLAGSYYHYEVYLSKDGADYGKVAYKSDDAPATGAADTHPIDATEAAYARISVSYNSAAQQVNLAEVAFHGTKVSDEQASPKAISVTDFDSSSWGREWARVETDADYAAEKTVTEVRNLVGRVIGERWVDKFDFQLRGKADGKDVFEISDAGDDRISIRGNNGVSLASGLNYYLRHWCKVDYNPLFGSQLSMPESLPAVGRKILKYTNYEYRYALNFCTYSYTMAFWNWDDYEPFLDWAAMNGVNLMLDIVGQEEVLRETLTQYGYSDDEVREYLSGPGYYAWFYMQNLYSVGGPLPAAWFEQRVELGRRIHDRMQAYGITPVIQGFGGQVPVDFQEKNPTSVAASSGTWSGFDRPYMIKTYLTDADKAAGKEDYFQKVGDTFYKAQENVFGKVSNYYAVDPFHEGGTIPDGFDIVDIYRTVQRKMLDHDPAAVWVMQQWQWGIDETKLSGLADKGQALVLDLQSDLRSQASPMENQGVPWVWNMLHNFGGRMGLDGVPEVISQDITKAYNSSGYMRGIGITPEAIDNSPIVYELLFDMTWEQDPVDYRSWTQEYAERRYGGTDGTIEKAWDILLDTAYKHTDGEYYQGAGESIINARPSDNTIGSASTWGHSDIDYDKRQFEKAAALFEQAYDSYKDSAGFRYDYVDVMRQVLANSFQEYQPLAGQAYKSGDLETFRTLSSRMLDIIKAQDKLLSSSDDFLVGAWIDDARTMLDGADDWTADLFELNARALVTTWGLNKNGSLIDYSNRQWAGLTGDYYYRRWKTYVDNRLNKLEHGTDFTDPDWFDYGWQWANRKSDEDGYGFATEAADDVDQKALGKIILDQYSVTAMDDVTDGGTAVERTNLALGHDVTDEDTGTVVPDVTDGNTDTGWTQTGKTDATLVVDLDGTYSITGAGITLQQIAADFPLRYEIDVWNGSGWVEIGRSEADAVSSKNEVAADILGSKVRWKLHSTNGRDLTGIYELSVWGAAQPQPEYTNLALGGAASAGPSERPASNGNDGDDGTLWVGNGSDPNWYRIDLASAQRVDRVRLVFETAGRLFQFRVVAGLADGTERTLIDETQNQGALDQVYAANLGEEVEHVTVEFTGSVGGTAWPALAELELLQEAGDTIEGVNIATSAAITSSPTKDAPENAGALVDGKATAWVSRDGATPAWFQLDYAKAREVDSIRLKFEEGQPDRSMQFTLKVIDANGDEHTVAERTEADLSKQQGIVMDVPVGMSITRIRMDIADARIPSSGSPAWPLVSEIEVYATPGNVARDAKTTASDGSTLTAADLAKLTDGDRDSAATLTATADKTLTFTLAKAADINMLGLLASGNSEPVRFKAEYRVVPQDGGGAGDGAADQWKTLTDYSGNAQMKPEIVARLARPVYTDAVRITVLNENPVAINELYLYQADAGASLESYLSSVETVLGKLTVGEYAGNVTRAAKTKLEVVLERARAALDAGLTSREAGRWTTTVEDAVSEFYRTGYVSLDRNALYVAIDDAAALIASLDAHGLPASSAALAEARASAKQVSDAYGTVTQQDLDDAAAALRRSADTALAQLDAQERYQVVLDAAVKTLEDAQTAGSVGEYEGQHPQSAADALRQAIDDAKAAHGAAAGDADKVDAAADALRQATTAFNESIVHIDAAALDAAKRAATGLVESQYDRAAWATMREALAAAGDTDMAHISQADVDTLAARLNDAIAALSDARLDRGPLSDAIASAQALKEGDYTAESWKAFAEALAAAQEECGRRSTTQGDLDKAVKALTQARDGLERKQPGGGEEPGGGEDPEQPGSGGQTERPGGVKPGAGGNADTSKPGTAGTETLSKTGAQTLLLAVTACIMLAAGFSITTARSRRR

SEQ ID NO: 115 - protein, 1112 aa, Bifidobacterium bifidum CCOS 571
MEKSSNRRFGVRTVAAIVAGLMVGGMCTAMTASAADDSAAGYSATAPVNLTRPATVPSMDGWTDGTGAWTLGEGTRVVSSDALAARAQSLASELTKFTDVDIKAATGSATGKDISLTLDASKKAELGDEGFKLSIGSKGLEVIGATDIGVFYGTRSVSQMLRQGQLTLPAGTVATKPKYKERGATLCACQINISTDWIDRFLSDMADLRLNYVLLEMKLKPEEDNTKKAATWSYYTRDDVKKFVKKANNYGIDVIPEINSPGHMNVWLENYPEYQLADNSGRKDPNKLDISNPEAVKFYKTLIDEYDGVFTTKYWHMGADEYMIGTSFDNYSKLKTFAEKQYGAGATPNDAFTGFINDIDKYVKAKGKQLRIWNDGIVNTKNVSLNKDIVIEYWYGAGRKPQELVQDGYTLMNATQALYWSRSAQVYKVNAARLYNNNWNVGTFDGGRQIDKNYDKLTGAKVSIWPDSSIYQTENEVEKEIFDGMRFISQMTWSDSRPWATWNDMKADIDKIGYPLDIREYDYTPVDAGIYDIPQLKSISKGPWELITTPDGYYQMKDTVSGKCLALFTGSKHLDVVTQVGATPELRNCADVSVGQDQRDTANERNTQKWQIRADKDGKYTISPALTQQRLAIATGNEQNIDLETHRPAAGTVAQFPADLVSDNALFTLTGHMGMSATVDSKTVNPASPSKITVKVRAASNANTGDVTVTPVVPEGWEIKPGSVSLKSIPAGKAAIAYFNVVNTTGTGDATVQFKLTNTKTGEELGTTSVALTGSLTKDVEASDYAASSQETTGEHAPVGNAFDKNANTFWHSKYSNPSANLPHWLAFKASPGEGNKIAAITHLYRQDKLNGPAKNVAVYVVAASDANSVADVTNWGEPVATAEFPYTKELQTIALPNTIPSGDVYVKFQINDAWGLTETSAGVTWAAVAELAATAKATPVELTEPEQPKDNPEVTETPEATGVTVSGDGVANGALSLKKGTTAQLTAKVAPDDADQAVTWASSDDKVVTVDKTGKVTAVAKGVAKVTATTANGKSASVTVTVTEDSEVPGPTGPTEPTKPGTEKPTTKPTTKPNDGKLSATGADTAVLATIAALFALAGGAVVAVRRRSVR

SEQ ID NO: 116 - protein, 673 aa, Bifidobacterium breve CCOS 586
MNGQTSLQGWTIIPMPQTMQHKANIALLPMCGRINEARAVGDDRHILAVQLIDDIRAATGLEWDIATGDRWPGFITLTTFDDPHAHPSGAYTLDVTPDGVTVAGADFEGVRNGVQTLRQLIRQCGAALPCLHIEDRPAFETRGYYLDVTRGRVPTLDWLKHWADKLCLYKYNQLQLYIEHTFAFDSMSETWRGSSPLTPRDILEFDDYCAERGIELVPSVSTFGHLYMALRTQSLRDLGEFPETADEPFGFIDRMHHHTLNISDDRAFDLSCRLIDDYLQLFRSDKFNICADETFDLGKGRSKPLADRIGVAAMYADYVTRLCRHLEARGRRPMMWGDIALEHPEILDRLPETVTLLNWQYDPQVTDEKIRTVAESGAKQIVCPAVWCWNALLPRIDDAWNNITRMARYGAQYHAQGMLITDWGDFGHVNDPRMAIPGMIIGAQESWNPGRIPDEADMLRRISRLEYHDASGELLDILARASHAASFEWNHLITWLELDDGQGGVNTGVLQTIPGLLPENERPDDVIRSLQNESKTPSLAESRRMLLRYLKHRITLGETADHLLQASTRRISAITATAGPRNAGNAAAFRIAVEGQRLLNRVGLRLASETGITDTLQPNTTSQHDDEANLAEALEIWMEAYATQWSTVSRDSELRRLQDTVWKLTDHLRFQSV

SEQ ID NO: 117 - protein, 174 aa, Bifidobacterium breve CCOS 586
MKYPDIPNVTKEYLDEVRPAINAGGSCSATAGATIGALSPPLVVDGTSIDIDASGVPVASINSYSVGQCTWWAAARRQQIGKPVDPYMGHGYMWAASAEKHGYPTGGTIQLGDVMSFERGVLGASGEYGHVAIVEEIHEDGSILISESGVDQRRAWTRLLTREQAENPGITYIH

SEQ ID NO: 118 - protein, 616 aa, Bifidobacterium breve CCOS 586
MRLSSGDHAGRASARTRHRKWLRSGLAAVLSMATLAALAAPASATDTMPWGGQYADTSHPEQSAGANQPYQHGYTGLDILNWNPDADKDSEYLRSRVPLQTRIAANAATQKDPNLPADTEMFNLAGDYGNAFFESFHDNSVFSQYLFNYWQYTDYYGTWHGQPTANVPKSLYDEKAQSDWTQKWFEFGTLNLPNAAYTNVAHKNGAKSIATIFYSGNDRGEQTYKDLLQGKRADGTYPVADKLVEIAKYYGFDGYFVNQESSVNSADVPAYQDFMKQIIDQGIYIQWYDSATYPNGGVSYQNMFNDANSPWVQDPNKGKISDSIFLNYWFSGNMLQDSADHAKSLGIDPKYAVFAGIEAGQKKFGSIASNANYMNVNLDADGKPYVSLAALGTDFVSHELGDDKKVYPKYQNQVFDRERRLWTGSSTGEKGTTDISDPYIDDGTSSDSWKGFASQIAERSVIDGPVFSTSFNTGHGLEWRDNGEQTSNQQWGNINLQDILPTWQWWIDADSDPLQADFDYGKKYEAAPRFNYTKVGGYEGGDSLVLSGKLSSDNTVRLYKTDLSVAAGSKVELTYNKLNSDDSKLQLGLIFADDTKTIVPVDMETVGQATAGRPQL

SEQ ID NO: 119 - protein, 627 aa, Bifidobacterium breve CCOS 586
MEFTVSGTTVRFDERTMQFAFTRDGAEWNTCADFKPTLQCTQGTFAFADATSITHEQRETGTGTGIRSIFTGFGHSAYSFETYVWVERASGDVLFEWIPLNEQGLTVTGVTWPAAIAFDRDDSHDVTLITHEQGVMIPNTWPTAVSTKDITFDGRFETAGGYMPWFAQLRADGHGYIAICETPWNAGYGIDHPSNGPYTHINTWFEPSLGTMNYRRVVRYQFLDHADHTAVCKAYRSYVNERGRLRTLAEKAARNPSVRDLIGRSWVHVGIKTKVQPDSFYYDKDHPEKNDSLVTFAQREKQMRTLHSMGAGRLYMHLDGWAQPGYDNAHPDYLPACQEAGGWEGMKSLVDACHEQGDIFGTHDQYRDYYFTAQTFDANNAIRLADGTMPEHARWAGGHQTYLCAELAPDYVRRNFTQIAAHGIKLDCAYLDVFTCNEGDECSNPEHRMTRRECFDRRTECFEYLLSHGILSSSEEVSDWAVPSLIFCHYAPYDFQMRSPNEPRQGVPVPLYNLVYHDCVIEPWMMERVVNGDDYMLYALLNGGAPYLIRDAAYIGVDGDMDDEQRARTENDIERCHTVAAFHERVGMQELVRHEFVDDDPLVQRSVFVDGTAVTCDFHTQTYRITD

SEQ ID NO: 120 - protein, 237 aa, Bifidobacterium breve CCOS 586
MSTDQLRQSASVWGSQLAAAGINVDLAPVLGTVVANRAANAPIGALYRDFGLDAAGNAAQGTAFVQGMADAGVQSAIKHYPGLGAVTGNTDFTADGILDTTTTLDGTEIKAFDTTIDQADPAMVMMALATYQAIDPNDPAVFSSIIIDGHLRGDLGYDGVVISDSMSAAAVSAYDTTQLGVKLVEAGGDLACIGYTNYVAPILDGLSTRAASDPAFANEVTQSAIRVMTLKIKMGLA

SEQ ID NO: 121 - protein, 133 aa, Bifidobacterium breve CCOS 586
MSIGEDTAGVRLCGEVRGGGLFLYPLGEGQIRKISDVPPTTDTALFDKGYEGSASYRIPSLVTTPSGVTIAGADQRVVISNDAPMRSISLSAAPWIADRRGCRCKPSSPFPVMGWMARASSTHASSVIVRQAV

SEQ ID NO: 122 - protein, 433 aa, Bifidobacterium breve CCOS 586
MSTFPQLATHPGMNPAAVIQGDRWRIGIITESLVRLEWQDNGKFEDHATQMIVNRDWLSDDANGADGANRADGTSNPPKFTKTERDGLLIIDTPALRLTYDMQPFSKEGLSIVVKGVANSQMNTWHYGEAQDGNLRGTARTLDAVDGEIELGLGVISRDGWAVLDDSASNVIVEGAEAATVKGEANPFGMWVIPREHPGKDLYVFGYGHRYIEAVQDFYKLTGPTPLLPRFALGNWWSRYHRYTEAEYLELVDRFEQEGLPFTTAVIDMDWHLVDNVDPKYGSGWTGYTWNREFFPDPERFQRILHEHGLRTTLNVHPRDGVRAFEDGYAKVAEHMGIDPAGGEPVEFDLTSPRFMEAYFDLHHGLETLGTDFWWLDWQQGGVTRQKGLDPLWMLNHMHYLDSAVTGAGRSRSRDMPARARTVIRSGSPATQS

SEQ ID NO: 123 - protein, 338 aa, Bifidobacterium breve CCOS 586
MIDVSAWQGNINWQAVKNSGVEGAIIRIGYGWDNGFDKQALRNISECRRLGIPFGIYLYSYAYDANTGAAEGSSLVNLLQKAGVSSSDLGYPVYYDLERWTWTGHEVPNDPGTYDGIVNAWYGRLQSAGYNNLAVYSYTSYLNTALNSGNIHSKTRWVAQYGSSMGYTAFPTNDRGWQYTSRGSVSGISGTVDLNAFGNQTATSSAPSVPVYRVYNPNSGLHHYTMNYNEVIMLVGKGWRYEKTAFRAGQSGIPVYRVYNPNDGNHLFTMNSYERDNLARLGWHDEGVSWYVPSGGSINVYRLYNPNNGEHVFTTEYGEYVLVGRAGWHQEGVAWTSL

SEQ ID NO: 124 - protein, 124 aa, Bifidobacterium longum CCOS 974
MGIPVRSGGYQLIGAKKTFIDEMNQWMKTESNKPFLFTEYGADTDAGVHKLPSVQWSEEYQCEYLAMQHEVFDMFEAVVGEQVWNLCDFQTGEGIMRVDGNKKRLHSRPSAQSRRLCTQGALGD

SEQ ID NO: 125 - protein, 400 aa, Bifidobacterium longum CCOS 974
MATICALAVVLAGVAAYGWHVGWFAKSTSNGNTTTPQTSQTSALPRADVPSPKKNEPAAQAQRAVSAMTLEERVGQLVMVPLLAGSDPSSLASTIADEHIGSAILIGNWNTGVDTVKTATAQLQGYAPAGNRLIIATDQEGGQVQHLTGTGFDTMPSAVEQGTMSADALRQSAGTWGSQLAAAGINVDLAPVLGTVVGDRASNTPIGALDRDFGLDAAGNAEHGIAVIEGLRDAQVGAAVKHYPGLGAVSGNTDFTTEGILDTTTTLDGAEAGAFDQAITKTDPAMAMMSLATYQSIDPNNPAVFSSTIIDGHIRNALKYTGVVISDSMSAEALSSYDVSQLGVKLVEAGGDMSCIGQTDYVKPIVDGLNERAKSDPAFASKVTAAATRVMALKIKMGLA

SEQ ID NO: 126 - protein, 631 aa, Bifidobacterium longum CCOS 974
MEFTVSGTTVRFDERTMQFAFTRDGAEWNTCADFKPTLQCAQGTFAFADATSITHEQRETGTGTGIRSIFTGFGHSAYSFETYVWVERASGDVLFEWIPLNEQGLNITNVTWPAAMDFDCADDHDTTLITHEQGVMIPNTWPTAVSTKDIAFDGRFETAGGYMPWFAQLRADGHGYIAICETPWNAGYGIDHPSNGPYTHINTWFEPSLGTMNYRRVVRYQFLDHADHTAVCKAYRSYVNERGRLRTLAEKAARNPSVRDLIGRSWVHIGIKTKVQPDSYYYDKDHPEKNESLVTFAQREKQMRTLHGMGAGRLYMHLDGWAQPGYDNAHPDYLPACQEAGGWEGMKSLVDACHEQGDIFGTHDQYRDYYFTAQTFDANNAIRLADGTMPEHARWAGGRQTYLCAELAPDYVRRNFTQIAAHGIKLDCAYLDVFTCNEGDECSNPEHRMTRRECFDRRAECFEYLLSHGILSSSEEVSDWAVPSLIFCHYAPYDFQMRSPNEPRQGVPVPLYNLVYHDCVIEPWMMERVVDGDDYMLYALLNGGAPYLIRDAAYIGVDGDMDDEQRARTENDIERCHTVAAFHERVGMQELVRHEFVDDDPLVQRSVFADGTAVTCDFHTQTYRITDCPHH

SEQ ID NO: 127 - protein, 315 aa, Bifidobacterium longum CCOS 974
MGILNKGKPKHGHLHRRVGMTLTALAVAVSMAFAPAAMADMQGVDMSNWQCGADVYNMQADFIVVGTTWGTGQVNNNCLVSGVNTDANRMIAQAQASGKKFGLYHYAMGGNPEAEAQFFYRNTSNYWRHGIVALDWEMDDNPAWGDWDWVRRFTAECERLSGGVKPLLYTGPVAGTIPGDIRANYGLWIAQYANMSPTGYQANPWMLGAYGEAMRQYSGTGVVNTWSPIDLNIFRGEGWQWICTPTPPAPQPRPRQRPRPCSRALPRPTPTRVASATSCNGEKPSGDSPSPMMLGPCPRGIRRAVTSTATTWATS

SEQ ID NO: 128 - protein, 711 aa, Bifidobacterium longum CCOS 974
MPTFEYKADAATPCLTLIPAPVTLEYTHGTAMIGSLVTIEKRIPEYAVTEDADETWETLPIEQLSSELERYCGVAVRTRRVLTATDEADAGANAAEKARDAGVGAGAGAGAPAAMNGTVILLCVDARLAHDEYTLDVFASDTIAVRGGSESGLRYGMQTLRQMIRQTSRTLPCLHIQDKPAFAVRAYSLDVTRGRVPTMAFLTWFIDQLALYKYNQFQLYVEHAFAFGELSEAWRGTDPLTADDIMFLDEYCAHHGIELVPSLATFGHMYMNLRTREHRGLGEFPEDADRPFSFIERMEHHTLNAANPKSHDFASRLIEEYAPLFRSRSFNIGGDETFDLGRGRSVQDSPGASRDELYADFVKDLCSTLAHRGLQPMLWADIALENPHTMDLLPGDITMLNWMYEPDIDESKIQTIASQGRRQFVCPAVRAWSRFFPDYDGAWLNTYRMAVAGLKYGAEGMVVTDWGDYGHVNDPRLSVPGLCYGAQNAWNPVAIDACEMNHRISNLAYGDESGWLMDSLARIDSDGVSFPWDLAVQVLELEYGSGTGMLNTDVASYVERSCGGELMFDRALGCADARRRLLLRNHARLERRRDCDRALIDCGSAVVAVLDGLARGGLNPELLWVMLDGQRLFNRLGEELLVLAGGEDACDTKDVTGRALDASRRARLAADLELWFERYRVQWLSIGRYAELARIAHVVWSFADILRRGAL

SEQ ID NO: 129 - protein, 634 aa, Bifidobacterium longum CCOS 974
MVEKKRLDGSDAKGATGAARATGMLRALRARAAASGAGRGVTAAVTSVAAVAMLGAVCVTPASALADVNADADASGVRSAASATASDGTSSDARSQARSATSATRPVANGVTVADETAADAMPDNPDAELPDKVSAEISDDAMVVSEQYAATPEGELKDIETGETVTDPKIVGTESKQPDPLAKTDGESFIPVSAADVKEKVAANGGDVNAVSSKTRAANASVKLAALQNNEYGAHWGTYNGTQAFFDARNNLFAQQAKGVIDVSAWQNTIDWQAVKNAGVEGAIIRLSYGWGNGFDVQAKRNISECKRLGIPFGVYVFSYAESAADGASEGADVVNLLRQAGVNPGDLSYPVFYDLENWTYTGHKSPTSPSVYDGMVNSWYGKLQAAGYNNLSVYSYTSYLNSALNSSNIHGKTRWVAQYGSTMQYTAFPTNDRGWQYTSGGSINGISGRVDMNAFGNYQFTPAVQITWVYRSEDIAVGASVDYPSSDIDYKWQSYNLSSKRWKTITDWTGANWAGWVDQLGDYWLHVEARDSRTRKIIGSQTIAFRYAPGTTRVAATYAGWQNNHVLLGESSNNAAAHYEIKIYDVRRSKWVQGFKGPWAIWKPKKGIYWTHYEVYTSDGRLADTKTYAFGV

SEQ ID NO: 130 - protein, 439 aa, Lactococcus lactis CCOS 949
MPVSRIKVKNRHLKKKAKKPLAFYKPATKFAGAVLIAGTLTTTHELLLQQTSPMVQAATNSTEAFIESIAASAKPVADSNGLYPSVMIAQAILESNWGSSQLSRAPYYNLFGIQGTYQGKSVVFKTQEYLNGKWVTKDMPFRVYPSFNQSFQDNAYVLKTTNFGNGPYYAKAWRANAATYQAATAALTGKYATDPNYGASLNRIISQYNLTRFDGASSAGTSNSGGSTATNTNNNSNTSSTTYTVKSGDTLWGISQKYGISVAQIQSANNLKSTVIYIGQKLVLTTSSSSSNTNSSTSSGNSAGTTTPTTSVTPAKPASQTTIKVKSGDTLWGLSVKYKTTIAQLKSWNHLNSDTIFIGQNLIVSQSAGSSSSSTGSSSASTSSTSNSSAASNTSIHKVVKGDTLWGLSQKSGSPIASIKAWNHLSSDTILIGQYLRIK

SEQ ID NO: 131 - protein, 347 aa, Lactococcus lactis CCOS 949
MKKVIKRKVILFSLPFLLLLLPILAFFALFVGSSDLSSDTDINTNTPQQQTAKVIWDRVLKEGGTKEGAAALLGNNQAESELQPSIIQSNATYNEAKAMDTTLGGYAFGLAQWDSGRRVNLLNYAKSQKKSWTDTNLQVEFMFEQDGTDSTLLKQLIKGTNVKQTTEDIMRKWERAGAVDSLPKRQGFAEYWYTFMTTGGDSGTGGGSGITPDIPSGWTLDKPINTSGYLATSYEYKQCTWFTWNRAQDFGITFGMYMGNGADWQHQAGYTVTTTPTLHSAVSFSGGQTVGGQWTADPQYGHVAFVEGIHSDGSVLISQSGTGFSTVYTFQVLTKAQASQLHYVIGK

SEQ ID NO: 132 - protein, 297 aa, Lactococcus lactis CCOS 949
MQYKKKENKVLVIFVLVVIFILCGCIYVLLVRYTHTDKITTISYKQPTKTSASNGYVEQKGEEAAVGSITLVDDAGVPEWVKVPSKVNLDKFTDLSTNNITIYRINNPEVLKTVTNRTDQRMKMSEVIAKYPNALIMNASAFDMQTGQVAGFQINNGKLIQDWSPGTTTQYAFVINKDGSCKIYDSSTPALTIIKNGGQQAYDFGTAIIRDGKIQPSDGSVDWKIHIFIANDKDNNLYAILSDTNAGYDNIMKSVSNLKLQNMLLLDSGGSSQLSVNGKTIVASQDDRAVPDYIVMK

SEQ ID NO: 133 - protein, 499 aa, Lactococcus lactis CCOS 949
MTNNDKTKRLKKEKFIAGTALILGMTTFGVAGHADGVTVGSSSDASSSTGSSSSSSGTGGSSSSSSTGSSSSSSNSNASSSSSSTGNSSSSSKPSTSGSTSKPSNPSSSTNNNSTSNSSTTTQAPSTSVSTIAPSASTSTVAPSNYSQDNAYYQTSTAAQIPNSSADSAPSIYAGPVLKTIEAAKSIDKIDTSSTEAFIKSIADRVRILAGKNNLYASIILAQAILESGSGQSNMSQQYFNIFNITGAYLGKSISFKTEEFSGNNPYYIEQSFRVYSNYDQALDDYINLMIKGTTWNSEIYAGAWKSHAKTYQEAAQALQGIFATDPAYAQKLIEIIQEYKLDAYDNVDSTTQVVDSKIPESPLAASKLDNSAYPEYNGVEYPGADSYAFGNCTQYVYNRIIQLGGLVGTHMGNGGEWGINAQAQGYFTTTVPTEGYAVSFPPGVAGSSSEYGHVAFVEKVYSDNSILVSEMNVKGNNIVSERHISAGVAALATYIQPK

SEQ ID NO: 134 - protein, 259 aa, Lactococcus lactis CCOS 949
MSSIENMIAWMQARKGKVTYSMTLRMGPRSYDCSSSVFFAMIAGGFLSEGSMGNTETLFGMSGTKLKEISRGEVHRGDIFISGTPGGSAGSDGHTGIFLSNGSFIHCSYTHNGIAVDTNDAYMSTRLPHHFYRIVGSGSANTDSKPQMVTLNVDGQFGNATAKRLQEYFDTAGKDGVISHQYKQTFNQNIYAAQFDSSLTGSNVVKALQRFLGIGQDGLFGQGTIKALQKHLGTTQDGTISPVSDSVRELQRRLNANKL

SEQ ID NO: 135 - protein, 271 aa, Lactococcus lactis CCOS 949
MKPKMRRKLKKMGAFIFTASMIAMIALLGLVRIRPVEPPKKAATEKIVVNHILDEKVLDLNKPVVDLSGWQRPEDIDYNTLSQHVIGAVIRVNGSYGHADNSASKDGEDTAYKQHIKAFQERGIPTAVYAFVTGENTSEMRKQARDFYRRASPYKPTYYWLDVEVTNMKNMNQGIEAFRSELEKQGAKNIGIYAQDWFLRDNQIKVDKFKAIWIAAYGRNTGYWDASPETTLSYKMQQFTDQGTLPGYSGNVDLNMVNNQTNYNELFKNQK

SEQ ID NO: 136 - protein, 870 aa, Lactococcus lactis CCOS 949
MDKRSKENFKASLNVQKRVSDGIDANAFRKPRQATQLSKQAFKEGKKTLKIRRKNYRKLKAGSGLQVVAAKKKVLEAKADKTVSKAVFKNAKKSDPTRAANQAKGYAKNQAKQTAVNHLVLSPLEKDDTLREGSDLYRKTQRTKSGLKLSKDVVTSSAKASVNLSNHTYGLANRSVNIVRGRGFVRTPSELGFRRQAAKRMRNFQNKLSAARKAKKAEQGFSLIRSILKGQQTLSRAFTLIVTSKGLLVVLAVMFILCLLGILNMASSVPTKQDDFQLTKSWTYFTKLDADNSENGNSFYTPLDDVMFYMNDQFEDYNLQDQVPVGSNGAALPNQNYEQYLTGLWSALNGSSPDYKLTTMEALETDKRSKYYLSPDDYSDFKERVNEVGYDSLDGQLQFPYQTESLVINRRYGYERNGDKTELHASIDVSSAPGQDLTSPMHGIVNSVTDPNTLVISEAENARLTIVGINSGRFIGGETVDAGTLLGKATKSSLNMTYEKYNEDDKKWEKVNPAFYFPKVTYTQFTSLASDSFDPGKSVSERAEAVYNFLTKLGYKKEGICAILGSFTEESQINPKRAEGDYLSPPVGASGNSWDDPAWLAMGGLDIYGKYPNILHRGLGLGQWTDTSDGSERHTLLLNYAKAKNKKWYDLDLQLDFMLNGDTPGNQTMFKNTASNAVSSSIPELTNYFLTYWEGNPGDKIQARVQAAQNWFTYFSNNGGSDADMSASSKELFEKYKDKIKPLPSNKETQQGQGWPGNGYEPGNCTWYVFNRQAQIGHNINGYMGNGGQWGYNYTKTPGATIDSKPQVGDAVSFSPGVAGSSSEYGHVAQVEVVNPDGTFLVSEMNTLGLYSMGYRMFKPGAGMTFVHFK

SEQ ID NO: 137 - protein, 325 aa, Lactococcus lactis CCOS 949
MEKGLLVDIGRKYWSIAELKRLVLLLQEHKLTHLQLHLNENEGFALNFTDSPVSKKYSENMLKELKEFAKTHEITLIPDFDSPGHMGSLLEQNPEFALPDSNQQAVDVTNPAVIDWIMGIIDKIVDIFPDSDTFHIGADEFIDFRQIEKYPYLVEKTREKYGNKASGLEFYYDYVNQLTEHLQKKGKQVRIWNDGFLRKDLQSLVPLNKNVEVCYWTNWDKGMAEVKEWLTKGYTLINFCDNDLYYVLGEEAGYSYPTAEKLEREGKIQKFSGQQYLNQEEMKAVRGTYFSIWADNAAAKSVSEILDDLSKVLPVFMKIYGGNDE

SEQ ID NO: 138 - protein, 546 aa, Lactococcus lactis CCOS 949
MKKSKKFFIRICLSTGILASATLLTACFGTPAKHVKANYKVTAEAIPDYQSKNAPISSYWMPDKFLEWSAENDKDLVYNQSRVPLTKRISPDKLSPSNQNQNKKTKIVALSMMNSQTSGNPSRGTTKFESYTFDYWQYIDTLVYWGGSSGEGIIVTPSADVIDEAHSNGVPVLGTIFLPPKEYGGKVDWVKTMLKKDEQGQYPFASQMVKVAKTYGFEGWFINEETQGLNADDAANMKALIQQVKKEDSSLQIMWYDAMTKDGKVDWQNQLNDQNATFVQDKAADAMFLNFWWTQNNLADQKLLEKSNLYAKNHNIDPYNIYAGIDVQAKDVQTPVKWNLLEKGNQATQTSIGLYAASATYTNASNWDDFQNRESAFWVNQKADPRQVDHSVNESWTGLSKYVLEKSAISGNEFNTNFNLGNGYNYFKAGQKISEMDWNDRSLAGILPSYRWIIDNEGKNKISPSFDFANAYNGGNSLKFMAEHLDAGKSSNITLFASDLKIAMGAKFSVSMRSDQALKVSAILELANGQKVSIAGDKSLTENWSK

SEQ ID NO: 139 - protein, 209 aa, Lactococcus lactis CCOS 949
MKYKTRRRKPNRRQSLLKQLIFIFLVILGILVYNKIFNNQAQKPSEAQLQEINEHKFIKEIAPLAQKSQKESQVLASITIAQACLESNFGKSELASKYHNLFGVKASDDVPKVSLATQEYENGQWVTVQGVFRVYPNFADSVSAHTQLFLYGTTWNSKQYASVLSATDYKTAAKAVQNSGYATDPTYADKLINMIETYHLNQYDKSSSI

SEQ ID NO: 140 - protein, 259 aa, Lactococcus lactis CCOS 949
MSSIENMIAWMQARKGKVTYSMTLRMGPRSYDCSSSVFFAMIAGGFLSEGSMGNTETLFGMSGTKLKEISRGEVQRGDIFISGTPGGSAGSDGHTGIFLSNGSFIHCSYTHNGIAVDTNDAYMSTRLPHHFYRIVGSGSGNTDNKPQMVTLNVDGQFGNATAKRLQEYFDTAGKDGVISHQYKQTFNQNIYAAQFDSSLTGSKVVKALQRFLGIGQDGLFGQATIKALQKHLGTTQDGTISPVSDSVRELQRRLNANKL

SEQ ID NO: 141 - protein, 259 aa, Lactococcus lactis CCOS 949
MSSIENMIAWMQARKGKVTYSMTSRMGPKSYDCSSSVFFAMIAGGFLSEGSMGNTETLFGMSGTKLKEISRGEVQRGDIFISGTPGGSAGSDGHTGIFLSNGSFIHCSYTHNGIAVDTNDAYMSTRLPHHFYRIVGSGSGKTDSKPQMITLNVDGQFGNATAKRLQEYFDTAGKDGVISHQYKQTFNQNIYAAQFDSSLTGSNVVKALQRFLGIGQDGLFGQGTIKALQKHLGTTQDGTISPVSDSVRELQRRLNANKL

SEQ ID NO: 142 - protein, 403 aa, Lactococcus lactis CCOS 949
MTKRLKKKAKPVVFLALVLGCALILSGVLGLAGHLNEQESSKTKKKSQLSETKRSSTSPKNMDKNIEQMTLEQKVGQLFMTGMPANNYNQATFDAIEKYQVGSIILTGRSNLSVPEMKDITDKLQGLEPANRKLLISCDQEGGNVQVLQGQGFSQIPDGLTQGSWTADKLQKESQTWGSELYAAGVNFDLAPVADQVLSADFAPQNAPIGYWSRQYAYDKASIISHAQAFTEGMKAAKVLTTAKHFPGLGAVTGNTDISAGVRDDQTNSNSESVQIFKDLISSGTPSIMTATAIYDKIDPNLPGAFSSKMVDGLLRKQLGFDGLVITDDLSNAVQVQSWTPGQRAVLALSAGNDLVLANEPTQIPEMISEVLQKVKADPDFAKKISQSATRVIKVKEEMKLVE

SEQ ID NO: 143 - protein, 312 aa, Lactococcus lactis CCOS 949
MIAQGILESSGGQSALASNYNNIFGVKYTSGTPVYLPTQEYLNGTMTNVVEPFQAYSSVYDACVAQAKMLRASSYYSGAWRENTSSYLDATAWLEGRYATDPTYASKLNSVISELGLSVYDQGGEISGGTAVTTSSSASTNSAGTYKVQEGDSLSAIAAQYGTTVDALVSANSLENANDIHVGEVLQVAGASTTTTSTNTTSNVSSSSTYTVKSGDSLYSIAEQYGMTVSSLMSANGIYDVNSMLQVGQVLQVTVSTSATTSNTTTSNSYTIQNGDSIYSIATANGMTADQLAALNGFGINDMIHPGQTIRI

SEQ ID NO: 144 - protein, 346 aa, Lactococcus lactis CCOS 949
MEKAIKRKVILVSLPFLLLLLPILAFFSLFVGSNSSSDTDINTNTPQQQTAKVIWDRVLKEGGTKEGAAALLGNNQAESELQPSIIQSNATYNEAKAMDTTLGGYAFGLAQWDSGRRVNLLNYAKSQKKSWTDTNLQVEFMFEQDGTDSTLLKQLVKGTNVKQTTEDIMRKWERAGAVDSLPKRQGFAEYWYTFMTTGGDSGTGGGSGITPDIPSGWTLDKPINTSGYLATSYEYKQCTWFTWNRAKDFGITFGMYMGNGADWQHQAGYTVTTTPTLHSAVSFSGGQTVGGQWNADPVYGHVAFVEGIHSDGSVLISQSGTGFSAVYTFQVLTKAQASQLHYVIGK

SEQ ID NO: 145 - protein, 717 aa, Lactococcus lactis CCOS 949
MKINKIDTRHGTANQSTFSHGNCLPYTGFPWGMNYFSPSTGAARGAWWFHPEDRTFEGYRITHQPSPWMGDFSHLTMTPVAGPLPETSLWHTVSSYRPEESTFNPTQLKITQLRYQITSQLIPSMYGGILSMNYQNLSLKDNGLMLHLPGSYELQQLDDYSLELSIINFAGCEDENFTFYLKFTADQPFVLSGNLSDEDSSVRLDFKAAKQVQIHFATSFISKEQAALNLEREQDNSAETYLENAESAWNNLFSRIEIEHHNQQEVSTFYHNLYRSFLFPQTFYEFDQEHQKIHYDTSSKTVKKGPLYTNNGFWDTFRTVYPLYSLIAVDEYGDMLEGFLNSYRATGFLPKWLSPDERGLMPGTLIDAVIADAASKNIRPDLMPEFLEAMKKGATSQSENSNYGRRGTKDYLKLGYVPLTHHESVNHTLDYAFSDYCISQVAKQTGDKEISDFYAHQAKDYQNIFDSETGFMRAKDADGNFRADFLDIRWGRDYAEGSAWQTSWSVLHDFAGLIKLHGSRENFENKLIELCNQRPNFNVEGYGFEIHEMSEMAAIEFGQVAISNQPSFHYPYLFSYIGKPWMATPLIKNLLTETFNDSPKGYPGDEDNGTMAAWYIFSSLGFYPVTAASNQYVLGIPLWDKARINLSSGQQLTILAEPNAPQQVFVNQITFTDKKVNDTFIKHEELIKGGTLKFDLGIVPNPLKYTNEQLPYSLTEN

SEQ ID NO: 146 - protein, 384 aa, Lactococcus lactis CCOS 949
MVKISFDVKKFEGQTIKKIGLSIKSDQAMDFKAINLGEMTLTNGQKVAPIALSDAKVTDEAFEEEGTVGGFRLSWKSDANKNNFSTYEIYQLNDDGSKEFLGASNINAFFVNALKRGKNINSTKFEIVPINKAGESGHSVTTSVKWPDNSLAKAAFVADKTLVTIGEKVTLMNQSNLASVKYKWDIDGASPATSTEKNPQVSFDKAGSYSVKLTVINEKGQEDSVTQTELITVIDQPVELTNFALNQSVQVDSFTNESESGPKAVDGKLNTKWCAVGPGKHNITIDIGKSEKINQVLIDHAQKGGESPDMNTSDYTIEISKDNQNWTEVVNVKKNKLGETKDSFKQTEARYVRITATKPTQGADTAVRLYEIQVLGQKKADKGL

SEQ ID NO: 147 - protein, 569 aa, Lactobacillus jensenii CCOS 962
MTKQTLQAEANGRNGKIKFDINIDNNEIKDIKVTKSSETPAIFNQVFDKLKNSIIEEQSFDVDAVSGATIMTSALLDSGKKALNQAGVTPVAKESDKTHREVNLDVDVAVIGSGAAGLIAACRALSMGKNVVVLEKNGYLGGATILNGSNVVATGSNLAQQLFGTEAQEDSSKRLFADITRECRGTNYPELSKVLVENIGKAVDFIKEFAGLTYQKAETQTIEHSVNRQVEMPSESSYELIKKIAAAFEEKGGKILLDARVEKINSENGVPISLVAEGKHQTTNVKFKSLILAAGGWGAKDFKEKRTSIPYYGPMTSTGDYFFFNKGLNLASRNLDWYKVYPHGLEVEPGIAKLTTYSTKEASDMGAIFINRAGNRIVNESDPYTHFRDAIAAQKDQIAFVLMDQRIWNRFYELMLKYGFTADEISHYFALDGKQSPILVKGTLETVANKAGINFENLQHTLSNYQNYAKNGKDPEFGREAKFMHEYSGDTYYVIEQKLRFCTTLGGYETNSQMQLLNNDMKPVANYYAAGEVIGGANGHDSMPSMMNSWSYASGFLAGTNASDNCNNR

SEQ ID NO: 148 - protein, 717 aa, Lactobacillus jensenii CCOS 962
MKTKKITGVATAALLASVAVPVTNNLANIQTSYTAKAVTGQQQAFLNTAIPNAEAASARYGTYTSVMLAQSILESGWGASLLATQANNLFGMKGSYNGQTYYTNTSEWASGTGYYNINAGFRKYPSWAASFEDNGYKLRTGTTDNPSRYRMAWIENAANYQVATQGLKDGGYATSPTYPQSLNRVISSYGLNQYDPSVDTTTKTMRVLSNGTVYSGPADSSVVSATGNITAGQVVTVDKTVTYKNGLSYMHISNGWINGSLLTGSSTQATTTEKAGTTTDAGNAAIKVVYTSAIAEWKNPGSGVVGYLQKGTTQTVVGKIQVNGAWWYKLSSGNWVPGEYVYVTGASRIPTIDNNVVNQNTKVKIKYISGYSIAVWSNPAIGTTGQYLKDGTEVQTIGYTTANGKKWYKLANNTWIPAEYTEVVSSSTVVTNITNESNTVAINYPHYSIAVWSEPGRNSTGKYLSDGTKVQTVGYTTVNGKKWYKLADNTWIPAEYTKVVSSSTVVTNITNESNTVAINYPHYSIAVWGEPGKNSTGKYLSDGTKVQTVGYTTVNGKKWYKLADNTWIPAEYTKAVSSTDTTSGNNTVTVNYPGYSIVVWSEPGRNSTGKYISDGTSVKYYATANYNGQTWYKIGENQWVPGQYVKVNASNNSGSVTVKYISGYGIAIWSNPGRNSTGKYLENGTTVKYFETQNYNGQTWYKIGENQWVPAQYVSVN

SEQ ID NO: 149 - protein, 775 aa, Lactobacillus jensenii CCOS 962
MAENNHRSASNTAPKNSRMANLHHDSGQPKRRLWLQILKWFSIGILLILVSGVGLFAYYAKDAPSISQDQLQSGGSSSFYTSDGKFLLSLGSEKRTYVKNSDIPQTLKDAVVSVEDKRFYQENLGIDPIRIVGSIVSNAKSSGIAAGGSSITQQLVKLTVFSTAASQRTLKRKAQEAWLAIRVEHDYTKNQILEYYINKVYMNYGVYGMGTAADYYYGKSLKDLDLAQTALIAGMPNAPVAYDPYTYPKAAKYRRDIVLNAMYANGKISKAQLKAAKAESITQGLKTQQNSSESSIRRIDDPYIKEAISEVKSKGYDPYNDNLKITLNIDQDAQNKLYELANGSSIPFSSSKMQVGATIINPSNGHVVAIIGGRNLPSVQLGLDRAVQTGRSTGSSIKPVLDYAPAIEYLNWSTAHYLEDTKYVYPGTSIQLYDWDNKYMGKMTMRYALEQSRNVPAVKTLAKVGMKKASLFAKKMNISVGSNQGLSVAIGANASSLQMAGAYAAFANEGVYYKPQFVSQIETADGVVHSYSATGTRVMKKSTAYMITDMLKGVLTEGSGTNARTGLYEAGKTGTVKYSDDELVKYPSYANTPKDAWFVGYTKKYSIGIWTGYDNLSDGTISGQGQYASQYLYKYMMKYLMSDKENSNWTKPSNVVRKRIVKGSDPLEVTSSKKNSTSELFLRGHTPDGSNEDSDESSSSSNSSSSSKDNEVVTNKSSSSSSSSSSEGHEDGSTSNSSSSQSSSGGSPNNNQGTTTNNQTNNNNNTGQNNGGGNN

SEQ ID NO: 150 - protein, 2089 aa, Lactobacillus jensenii CCOS 962
MFSKNNMKMRMQKVADKEQQHFALRKLNVGLVSVLMGTTLFFVGQTSIAKADTLESTKTSVTEISSSSNSNQEKLEQAKAVSSQEQTTSTEENVDSASSSQSKSENNSSSSAKSEVSTQDRTDSNDNATTNQVDTTQVSTTSLKAVQSSNQAANLLAESKVEDSTTANVSDFDSFNSALMNQNITTININSDFTSGNYGTNVEHRRVVPRTLVINGNGHTVDLGSIGYFMNPGGNQAADWTVENGTFYSKSAVGPFALTGDHGTDKAWQATNGAVHRMTYKDMTVYAGGGAYAANAEIDLEGTNNLNATASYQSKFSNGTVYTETGGNRSGVEGQWIIIKDNANVTVNTDHGQAISTEYSDGNHRIEVGENATLNGNYLYTTYGTPYGGGKIAVLSNGANGGTVIFHKGSKSHFTMPNQNVTGFGGNGFSNYGTGSVLYLGAANTTIEKGAEVTIDNPKEANNDNSIFIRSDGTQLNIFGNLIINDGARDYTIRADNRVSINVGQSIADDDYSNDNGKLIINRNGDFYLNNDGGALSMWGPITINVNSGAALEVYSTGINNVSGSGANPALMRVGGSSKLNVYKRGTFILSDSSNGKVSLVDDYNANGNFNFDNTAKVIFDISNNNNQNSRIFALNGTVYATHDKVRAMLTPSSNIADMGTFKTVQFNTSGQGGVTGDALHSEYQNQAYNNIVAIRDAIRTGQLRYLEFSTRSVNNASITGEGHGFTDNGAQIKGSVVDESTNTGAVAVAYDKDNNKVGSGNVDDQGNFTINLDKPLLNKEEVKVRIETPRGASGFVSTTAPLGPTAKSPITVAKDDNLAGQDASQYITNKDEIANIKPGTTDYEPTFKSAAWKSVDTNTKKGIITVTYADNTTTDLDVDLNVVDKITDADKFTPEGGTIKVDNGHKLDGNDAYEAIKNHDDLPADKAGYNWVVDENHPAVDTTKPGDQTGYVQVTYNDGSKSDLVPVTVHVIADNEKYTAIGKTQNLQKGQSANPQDFIANKDGEVSQDGKTYTKLPDGTKYEWVDGGIDTSTIGPKQAQVKVTYPDGTTQIVPVKANVYSDANLSTVVGKDINAGYKEDLTNRAIDAIDKDKSTNLPTDPSAYTWVNGAPDTSKTGDIPATVKVTYPDGSYNTVDVTVHVTSDAEKYSPVPETISVPKGTDLSGRAKDGIANADKDANGKEKLPDGTKYEWDGGVPNTSVTNNKYGHVKVTYPDGSSTVVEVPLNITDNNKSDAEKHNPQANILHATLNQDLSSNDWAKKGILNADEQDGATFRWRKGYVPDTSKEGQVWGIVVVSYPDSSINEVRVPVIVQSDASKYGIETQEINVHEGTDISSDEWARKGILNADQAGKQNEQLPDGTSYTWANGNVPDTTKPNKKTGYVTVTFPDNSSRTVPVIVNVIGDGRSDAEKYQLKAHDIWTYINDTPVAEKAVSNLDELKDVSSITWATTPDVSKVGNVPAIVVVTYKDGTSNAAPINIEVKGLANDYKPEGTTIYAGLNEDITNRAADGIANKDQMPVANKPEGTVHTTYSWKDNIIPDTTKPGTKYGIVEVNFPDGSTKDVPVEVKVTSLASDYQNKIDTKQIIAKYKGNIPQASDGIANKDQATKEGDKDFPSLADVLAPNGIQWKKNFEPDLSKPGLTSGEAILTFKDGSTAEVTIPVLVQTDADRNTPETQTIKTLPGQTVNPEDGVINLHKPGENNPQLPDGTKVTFDNQSDVDDFTKHGMPGSDKSFDATVTYPDGTTDKIKLPVHITADNEVNTPITQGIITPKDSVPDANKGIANLKKATTKEGKTYPALPENTTVEWVNPGQMKTELENAKGGTTKNYDAVVIYPDKSTEIVSIPVTVATDADTYKVVTQPIDLKDRNLPDNADDGITNLHKPADFKTPQLPDGTHAEWQDKDAAQEVVKNLKPGETVKLPATVVFPDGSKKGEGIDVSVHLHGQSDDYNIETQPVNTDKDGNLPENADSGIKNLGKLPEGTHASWGDGAQDIAKNLKLGETKDVPATVVFPDGSKKEITIPVHREGQSDGYDVEPQLVNTDKNGQLPNAKEGIKNLADLPEGTNQPGQIELKIKLIRLSLVQIQLLK

SEQ ID NO: 151 - protein, 214 aa, Lactobacillus jensenii CCOS 962
MARSGSRVKKTTLTLVKVFGVLLILVVAFVCFRYYRRQAINNELIRQEQLAREQAAAKELKIKTDFIKKIGPIAQKADQGFALLPSITIAQACLESNYGQSELSQKYNNLFGVKSNDPNTSKILSTKEYVNGKWITVKASFQIYDSYESSIQAHARLFQNGTTWNKDQYQHVLAAKDYKTQAKALVTDGYATDPDYASKLINLIEQFNLNKYDN

SEQ ID NO: 152 - DNA, 1323 bp, Lactobacillus rhamnosus CCOS 965
atgaaacatatcggacaacttaagaaatggccgctggtgatcttattggcgctattgtttggcgttggtgccgcaacaaccagtgtgatggccaacacccaatacatgacagtcaaagccgagagcgtcaatgtacggctaggtcccggcttggcatatggcatcatgggtcaggtaaaatccggcaatgaattgaccattatcggttccaaaaattcctggtatcaagtgcgccttgccggcaataaaatcggttgggttgcttcatggttagtcgatcaaagcgaagccgcaaccacgagtgcgaaagttgccacggtgaatcaaccggttaacgttcgcgaatatgccagccaggatgccaagcagttaggaacgcttaatgccggcgatagtgtcaaagttgtgtatcaagaaggcgattggacccagattgcctataacaatacggcggcatggatcactagcagcagtgtccagctcactggtcagacaactaatctggcacaacctgcccaagccaatctgacgcaagccaaaagcggggccgcattgaaagtcaccaccaataccatgactaacctgcgcaatgcggcgggtatcaatgccccatccgtcgagaaactcgataaaggcactgaactgaccgttaccaaacaacaagacgattggtatcaagtcactgcccctgatggcaaatcgggttatgttgccagctggaccgtcaccgccccgaataatggtcaaacccaaaaagcggcaacgaaactatccgaagccacgattgttctggatcccggacatggtggtacagacacgggtgcgccagctaacaataatcatgattacgaaaaaacctataccttgaaaacggccgaactcgttgccaatgctttgcgggctgctggtgctaacgttatcatgacgcgaacgactgacacctttgtcgacctcgcgccacgtccgacaactgctaacaacgcccatgccgatgcatttatctccttccattttgactccagcccgtccaaaaactctgcctccgggttcaccacctattactacagcagcaaaaaggatctcgccttggctaaggcagttaacaacgcttttgatgacttaccactagaaaatcgtggggttgcatttggtaactatgaagttctacgcgataataaacagccggccatcctgaatgaaatgggttatatcaataacgacaaagactttaagtatattaaaaacccaacgtatcaatctaaaattgcgaccaatattgttaacggtttaaatgcttactttaaagccggtcatcatcaataa

SEQ ID NO: 153 - DNA, 636 bp, Lactobacillus rhamnosus CCOS 965
ttggcgaaaaagcgccgacgttttaccttaaagaaggttccattggcggcttggctggtcatcgctttttttgcggttggttcaatgttggttgtcagctcgtattggtcgcaacggcaagccgaagtttcacagcgccaagcaattgtcgataagaaggcggctgaaaaagcgaagaaagaggcttttatcaagcgattggtgccgacagcccaggccatgcagaaacagtatggtgtcttaacgagcattacgctgtcccaagcgattcttgagtctgattggggaacgagcacgttagccaaggattaccataacttatttggcattaaagggacggatcctgccaccacgaaagtattacggacgaaggaatatgttaacgataaatggattaccgttaatggtcggtttcgggtttatagcgatgatgctgcttcgattcgtgatcatgccttgttattcgttaacggtaccgactggaatccgcaacagtatgcaacggtaagagccgcaaaagattataagactgctgcctcggctttgcagacggacggctatgccactgatccggattatccccagaagctgattcatttgatcgaagcatggaatctgacccagtatgacaattga

SEQ ID NO: 154 - DNA, 765 bp, Lactobacillus rhamnosus CCOS 965
atggcgatgttaatggcagatgtaagcagttggcagccggattcggatagctggtttcgcaagttggctgatctgggtgtcaaggcggtggtcgtcaaactgacagaaggaacgacttaccagaatcctaaggcggcggcacagttggcggctgggcgcaggatggggatgcaggtgcacgcttatcactatgcccattttcataacagtgccgaagccgttgcagaaggacgtttcttcggcgtcacggcccgcgcgctgggcgtgtcgacgcaaagtgtgatggcagcggatgttgaagcacctgatttgaatggggagctgacggggctgacgaatgttttcattcagacggtcaaagcgctagggtatccacacacagacctgtatacaatggcgaattggatgaaaaccagacgctttgatcgcgtggcattgattcctaagaacctgtggattgcgagttatggcgttgatcagccgggcatcaataatgtcgggacctggcagtttaccaataactttcacggcttaggggtggatatgagttatgactttttcggtcactacaccacgcgcttgaccggtaacctcaatggcggcgtggcgcgcgttcccacgattcgctatcacacggttttggcaggcgaaagctggtgggcgattgcagatcgatatggcttgaatatgtacaagctcgcggccctcaatggtaagacgatctacagtgtgattcatccgggcgatcagctgcggttgaattaa

SEQ ID NO: 155 - DNA, 1323 bp, Lactobacillus paracasei CCCOS 1201
atgaagaaaattggacaattaaaaaaatggccgctggtcgttctggtggcgctacttttcggcgttggtgttgcaacaaccagtgtaatggccaacacacaatacatgactgtcaaggcagataccgtcaacgtgcggttaggtcctggtttggcatattcaattatgggacaagtgaaatccggtaatgaactgtcgattatcggtgcgaaaaactcctggtatcaagtccgactagctggtaataaaatcggctgggttgcctcttggttggtggatcaaagtgaagcagcaacttcacaggccaaagtggcaacggttaatcaaccggttaacgtccgtgaatatgccagtcaaaatgcaaaacaactaggttcgctaaatgccggcgacagcgtcaaggtcgtctatcaagaaggcgcttggactcagattgcgtacaacaccacggctgcatggatcaccagcagcagcgttcagttaaccggccaaaccaccaatttagcccagcctgcgcaaacggcgttggcaaccgagaaaagtgcgccggcgctgaaggtaacaaccaatacgatgaccaaccttcgcaatgccgccggtatcaatgcgccttcggttgaaaagctagacaaaggcaccgaactgacggtctctaagcaacaagatgattggtatgcggtcacggcaccagatggcaaaactggctacgttgcgagctggaccgtcagcgcaccaaatgacgggcaaacgcaaaaagccgctacaaaactgtcagaggctacgattgtccttgatccaggtcacggcggctccgacactggtgcgattgccaatgatggcaccgactatgaaaaaacatacacgcttaagacggccaatttagttgctaacgttttacgcgcggctggtgccaatgtcattatgacccgtacaacggatactttcgttgatttggcacctcgaccaaatactgccaacaatgctcacgcggatgctttcatctctttccattttgactccagtccatccaagaattcagcatctgggatcaccacctattactacgacagcaaaaaagaccttgccttggccaagtccgtcaacagtgctttcagcggccttccgctggaaaaccgcggtgtcgcctttggtaatttcgaagtcctgcgtgataataaacaacctgctattctgaacgagatgggttacatcaacaacgataaagatttccgtcaaatcaaagatccgagctatcagtccaagattgctaccgatattgtaaatggcctaaacgcctactttaaggcaggcaatcatcagtga

SEQ ID NO: 156 - DNA, 765 bp, Lactobacillus paracasei CCCOS 1201
atggtgatattaatggcagatgtgagtagctggcagccggaattggacagctggtttcgcaagctggcggatgttggggtgaaggcggtggtggtaaagctgacggaaggcaccacctaccgcaatcctaaggccgcagcgcaattggcggcaggtcggcgaatggggatgcaggtgcatggttatcattacgcgcattatcacaacagcgctgatgccgtggcggaaggacggttcttcggaaccacagccaaggctttaggtttgtcaaccgagtcggtaatggcagcagatgtggaggatccgggtttatctggtgagttgacgggggtgacgaatgtttttctccaaactgtcaaagcgatcggatatcctcacacggatctatataccatggccagttggctgaccgcgcggcgctttgatcgggttgccttgattccgaaaaatctgtggcttgccagttacggcgtgaatcaaccgggcgttgataatgtcggcacatggcagttcacgaataactttcaggggctaggtgttgatatgagttacgacttttttggtcactatacgacgcgtctcactggcacactcaacggtggtgtcgcgcgcgtgccaacgattcggtttcataccgtgcagccaggggagagctggtgggcgattgcgcaccagtacggacatgacatggacaagctggctgcattgaatggcaagacgattttgagtgtgattcaccctggggatcagctgcgggtggaataa

SEQ ID NO: 157 - DNA, 738 bp, Lactobacillus paracasei CCCOS 1201
gtgcgcagtcgggtcatttatgctgatacctatcgcaaacgtcatcaaagacgcttatttttgctggccgttttaatcatcgctttgggcgcactgtttgtttggtggcatcagcgcaacccccgccctgatccgcagacctatcccgtgttgggcgtgcgtcttgaccaaaccgatggggtgcaggattttgacagtttgcgcagcagcaaagtcagttttgtctatctcaaagcgactgaaggcagcagctattttgatgataattttaatacgaattttaatcaggcagctggcagtcgactgagcatcggcatttaccatgtgttcagctttgaaacgacaccccaagcccaagctgaccaattcacgcgccaagtcggccaaaatatcggtgatttaccgattggcatttacttaagctattacactgaaaagaagccaagcacacaatggctgacaactcatttacaaacttttgtcacattggtgcagcaacattatcatcgccaagtgttgctgatgggtagcccaagtattttaaaagctgtccaaaaagtcgacccgcaagcaccacgctgggttgtaagcgacaagaagccgacaacgagcagtggtttctggcaatatacgtctggcgcccggttgccgaatgggccacacgcagattaccgtgctgccgtatttatgggggatcgggcggcctttttaaaactgtctcagcagatagtcaattaa

SEQ ID NO: 158 - protein, 440 aa, Lactobacillus rhamnosus CCOS 965
MKHIGQLKKWPLVILLALLFGVGAATTSVMANTQYMTVKAESVNVRLGPGLAYGIMGQVKSGNELTIIGSKNSWYQVRLAGNKIGWVASWLVDQSEAATTSAKVATVNQPVNVREYASQDAKQLGTLNAGDSVKVVYQEGDWTQIAYNNTAAWITSSSVQLTGQTTNLAQPAQANLTQAKSGAALKVTTNTMTNLRNAAGINAPSVEKLDKGTELTVTKQQDDWYQVTAPDGKSGYVASWTVTAPNNGQTQKAATKLSEATIVLDPGHGGTDTGAPANNNHDYEKTYTLKTAELVANALRAAGANVIMTRTTDTFVDLAPRPTTANNAHADAFISFHFDSSPSKNSASGFTTYYYSSKKDLALAKAVNNAFDDLPLENRGVAFGNYEVLRDNKQPAILNEMGYINNDKDFKYIKNPTYQSKIATNIVNGLNAYFKAGHHQ

SEQ ID NO: 159 - protein, 211 aa, Lactobacillus rhamnosus CCOS 965
MAKKRRRFTLKKVPLAAWLVIAFFAVGSMLVVSSYWSQRQAEVSQRQAIVDKKAAEKAKKEAFIKRLVPTAQAMQKQYGVLTSITLSQAILESDWGTSTLAKDYHNLFGIKGTDPATTKVLRTKEYVNDKWITVNGRFRVYSDDAASIRDHALLFVNGTDWNPQQYATVRAAKDYKTAASALQTDGYATDPDYPQKLIHLIEAWNLTQYDN

SEQ ID NO: 160 - protein, 254 aa, Lactobacillus rhamnosus CCOS 965
MAMLMADVSSWQPDSDSWFRKLADLGVKAVVVKLTEGTTYQNPKAAAQLAAGRRMGMQVHAYHYAHFHNSAEAVAEGRFFGVTARALGVSTQSVMAADVEAPDLNGELTGLTNVFIQTVKALGYPHTDLYTMANWMKTRRFDRVALIPKNLWIASYGVDQPGINNVGTWQFTNNFHGLGVDMSYDFFGHYTTRLTGNLNGGVARVPTIRYHTVLAGESWWAIADRYGLNMYKLAALNGKTIYSVIHPGDQLRLN

SEQ ID NO: 161 - protein, 440 aa, Lactobacillus paracasei CCCOS 1201
MKKIGQLKKWPLVVLVALLFGVGVATTSVMANTQYMTVKADTVNVRLGPGLAYSIMGQVKSGNELSIIGAKNSWYQVRLAGNKIGWVASWLVDQSEAATSQAKVATVNQPVNVREYASQNAKQLGSLNAGDSVKVVYQEGAWTQIAYNTTAAWITSSSVQLTGQTTNLAQPAQTALATEKSAPALKVTTNTMTNLRNAAGINAPSVEKLDKGTELTVSKQQDDWYAVTAPDGKTGYVASWTVSAPNDGQTQKAATKLSEATIVLDPGHGGSDTGAIANDGTDYEKTYTLKTANLVANVLRAAGANVIMTRTTDTFVDLAPRPNTANNAHADAFISFHFDSSPSKNSASGITTYYYDSKKDLALAKSVNSAFSGLPLENRGVAFGNFEVLRDNKQPAILNEMGYINNDKDFRQIKDPSYQSKIATDIVNGLNAYFKAGNHQ

SEQ ID NO: 162 - protein, 254 aa, Lactobacillus paracasei CCCOS 1201
MVILMADVSSWQPELDSWFRKLADVGVKAVVVKLTEGTTYRNPKAAAQLAAGRRMGMQVHGYHYAHYHNSADAVAEGRFFGTTAKALGLSTESVMAADVEDPGLSGELTGVTNVFLQTVKAIGYPHTDLYTMASWLTARRFDRVALIPKNLWLASYGVNQPGVDNVGTWQFTNNFQGLGVDMSYDFFGHYTTRLTGTLNGGVARVPTIRFHTVQPGESWWAIAHQYGHDMDKLAALNGKTILSVIHPGDQLRVE

SEQ ID NO: 163 - protein, 245 aa, Lactobacillus paracasei CCCOS 1201
MRSRVIYADTYRKRHQRRLFLLAVLIIALGALFVWWHQRNPRPDPQTYPVLGVRLDQTDGVQDFDSLRSSKVSFVYLKATEGSSYFDDNFNTNFNQAAGSRLSIGIYHVFSFETTPQAQADQFTRQVGQNIGDLPIGIYLSYYTEKKPSTQWLTTHLQTFVTLVQQHYHRQVLLMGSPSILKAVQKVDPQAPRWVVSDKKPTTSSGFWQYTSGARLPNGPHADYRAAVFMGDRAAFLKLSQQIVN